European Patent Specification EP 3 921 423 B1, published January 4, 2023. Title: METHOD FOR DETECTING A SPECIFIC SPLICE EVENT OF A GENE OF INTEREST. Applicant: Helmholtz Zentrum Muenchen GmbH Klinikum rechts der Isar der Technischen Universitaet Muenchen. The sequence listing filed with the application follows.

SEQUENCE LISTING (65 sequences)

SEQ ID NO: 1 - protein, 105 aa, Artificial
  N-terminal splicing region of NrdJ-1
CLVGSSEIITRNYGKTTIKEVVEIFDNDKNIQVLAFNTHTDNIEWAPIKAAQLTRPNAELVELEIDTLHGVKTIRCTPDHPVYTKNRGYVRADELTDDDELVVAI

SEQ ID NO: 2 - protein, 88 aa, Artificial
  N-terminial splicing region of gp41-1
CLDLKTQVQTPQGMKEISNIQVGDLVLSNTGYNEVLNVFPKSKKKSYKITLEDGKEIICSEEHLFPTQTGEMNISGGLKEGMCLYVKE

SEQ ID NO: 3 - protein, 40 aa, Artificial
  C-terminal splicing region of NrdJ-1
MEAKTYIGKLKSRKIVSNEDTYDIQTSTHNFFANDILVHN

SEQ ID NO: 4 - protein, 37 aa, Artificial
  C-terminal splicing region of gp41-1
MMLKKILKIEELDERELIDIEVSGNHLFYANDILTHN

SEQ ID NO: 5 - protein, 808 aa, Artificial
  split intein - heterologous polynucleotide construct
CLVGSSEIITRNYGKTTIKEVVEIFDNDKNIQVLAFNTHTDNIEWAPIKAAQLTRPNAELVELEIDTLHGVKTIRCTPDHPVYTKNRGYVRADELTDDDELVVAIGGGGPEDELAANEEELQQNEQKLAQIKQKLQAIKYGGSGGGGSGTGMEDAKNIKKGPAPRYPLEDGTAGEQLHKAMKRYAQVPGTIAFTDAHIEVNITYAEYFEMSVRLAEAMKRYGLNTNHRIVVCSENSLQFFMPVLGALFIGVAVAPANDIYNERELLNSMNISQPTVVFVSKKGLQKILNVQKKLPIIQKIIIMDSKTDYQGFQSMYTFVTSHLPPGFNEYDFKPESFDRDKTIALIMNSSGSTGLPKGVALPHRTACVRFSHARDPIFGNQIKPDTAILSVVPFHHGFGMFTTLGYLICGFRVVLMYRFEEELFLRSLQDYKIQSALLVPTLFSFFAKSTLIDKYDLSNLHEIASGGAPLSKEVGEAVAKRFHLPGIRQGYGLTETTSAILITPEGDDKPGAVGKVVPFFEAKVVDLDTGKTLGVNQRGELCVRGPMIMSGYVNNPEATNALIDKDGWLHSGDIAYWDEDEHFFIVDRLKSLIKYKGYQVAPAELESILLQHPNIRDAGVAGLPDDDAGELPAAVVVLEHGKTMTEKEIVDYVASQVTTAKKLRGGVVFVDEVPKGLTGKLDARKIREILIKAKKGGKIAVGGSGGDYKDDDDKGSPGITSYSTHYTKLSGGSPEDEIQQLEEEIAQLEQKNAALKEKNQALKYGGGGMEAKTYIGKLKSRKIVSNEDTYDIQTSTHNFFANDILVHN

SEQ ID NO: 6 - protein, 755 aa, Artificial
  split intein - heterologous polynucleotide construct
CLVGSSEIITRNYGKTTIKEVVEIFDNDKNIQVLAFNTHTDNIEWAPIKAAQLTRPNAELVELEIDTLHGVKTIRCTPDHPVYTKNRGYVRADELTDDDELVVAIGGGGPEDELAANEEELQQNEQKLAQIKQKLQAIKYGGSGGGGSGTGMEDAKNIKKGPAPRYPLEDGTAGEQLHKAMKRYAQVPGTIAFTDAHIEVNITYAEYFEMSVRLAEAMKRYGLNTNHRIVVCSENSLQFFMPVLGALFIGVAVAPANDIYNERELLNSMNISQPTVVFVSKKGLQKILNVQKKLPIIQKIIIMDSKTDYQGFQSMYTFVTSHLPPGFNEYDFKPESFDRDKTIALIMNSSGSTGLPKGVALPHRTACVRFSHARDPIFGNQIKPDTAILSVVPFHHGFGMFTTLGYLICGFRVVLMYRFEEELFLRSLQDYKIQSALLVPTLFSFFAKSTLIDKYDLSNLHEIASGGAPLSKEVGEAVAKRFHLPGIRQGYGLTETTSAILITPEGDDKPGAVGKVVPFFEAKVVDLDTGKTLGVNQRGELCVRGPMIMSGYVNNPEATNALIDKDGWLHSGDIAYWDEDEHFFIVDRLKSLIKYKGYQVAPAELESILLQHPNIRDAGVAGLPDDDAGELPAAVVVLEHGKTMTEKEIVDYVASQVTTAKKLRGGVVFVDEVPKGLTGKLDARKIREILIKAKKGGKIAVGGSGGDYKDDDDKGSPGITSYSTHYTKLSGQVSILFTAQLNETDRNWSCRNRVG

SEQ ID NO: 7 - protein, 414 aa, Artificial
  split intein - heterologous polynucleotide construct
CLDLKTQVQTPQGMKEISNIQVGDLVLSNTGYNEVLNVFPKSKKKSYKITLEDGKEIICSEEHLFPTQTGEMNISGGLKEGMCLYVKEGGGGPEDKLQAIKYELAQNEEELAQIEEKLAANKEGGSGGGGSGTGFANELGPRLMGKGSGGGGSGVFTLEDFVGDWRQTAGYNLDQVLEQGGVSSLFQNLGVSVTPIQRIVLSGENGLKIDIHVIIPYEGLSGDQMGQIEKIFKVVYPVDDHHFKVILHYGTLVIDGVTPNMIDYFGRPYEGIAVFDGKKITVTGTLWNGNKIIDERLINPDGSLLFRVTINGVTGWRLCERILAGSGGSSYTSNRIGTSGGSPEDENAALEEKIAQLKQKNAALKEEIQALEYGGGGMMLKKILKIEELDERELIDIEVSGNHLFYANDILTHN

SEQ ID NO: 8 - protein, 380 aa, Artificial
  split intein - heterologous polynucleotide construct
CLDLKTQVQTPQGMKEISNIQVGDLVLSNTGYNEVLNVFPKSKKKSYKITLEDGKEIICSEEHLFPTQTGEMNISGGLKEGMCLYVKEGGGGPEDKLQAIKYELAQNEEELAQIEEKLAANKEGGSGGGGSGTGFANELGPRLMGKGSGGGGSGVFTLEDFVGDWRQTAGYNLDQVLEQGGVSSLFQNLGVSVTPIQRIVLSGENGLKIDIHVIIPYEGLSGDQMGQIEKIFKVVYPVDDHHFKVILHYGTLVIDGVTPNMIDYFGRPYEGIAVFDGKKITVTGTLWNGNKIIDERLINPDGSLLFRVTINGVTGWRLCERILAGSGGSSYTSNRIGTSNWLRCPSVGRAHIAHSPREVGGRGRQLNRCLEKVARGKLGK

SEQ ID NO: 9 - protein, 363 aa, Artificial
  split intein - heterologous polynucleotide construct
CLDLKTQVQTPQGMKEISNIQVGDLVLSNTGYNEVLNVFPKSKKKSYKITLEDGKEIICSEEHLFPTQTGEMNISGGLKEGMCLYVKEGGGGPEDKLQAIKYELAQNEEELAQIEEKLAANKEGGSGGGGSGTGFANELGPRLMGKGSGGGGSGVFTLEDFVGDWRQTAGYNLDQVLEQGGVSSLFQNLGVSVTPIQRIVLSGENGLKIDIHVIIPYEGLSGDQMGQIEKIFKVVYPVDDHHFKVILHYGTLVIDGVTPNMIDYFGRPYEGIAVFDGKKITVTGTLWNGNKIIDERLINPDGSLLFRVTINGVTGWRLCERILAGSGGSSYTSNRIGTSQVSILFTAQLNETDRNWSCRNRVG

SEQ ID NO: 10 - protein, 331 aa, Artificial
  split intein - heterologous polynucleotide construct
CLDLKTQVQTPQGMKEISNIQVGDLVLSNTGYNEVLNVFPKSKKKSYKITLEDGKEIICSEEHLFPTQTGEMNISGGLKEGMCLYVKEGGGGPEDKLQAIKYELAQNEEELAQIEEKLAANKEGGSGGGGSGGGGSGGGGSAKPLSQEESTLIERATATINSIPISEDYSVASAALSSDGRIFTGVNVYHFTGGPCAELVVLGTAAAAAAGNLTCIVAIGNENRGILSPCGRCRQVLLDLHPGIKAIVKDSDGQPTAVGIRELLPSGYVWEGGGGGSGTGFANELGPRLMGKGSGGSSYTSNRIGTSQVSILFTAQLNETDRNWSCRNRVG

SEQ ID NO: 11 - protein, 652 aa, Artificial
  split intein - heterologous polynucleotide construct
CLDLKTQVQTPQGMKEISNIQVGDLVLSNTGYNEVLNVFPKSKKKSYKITLEDGKEIICSEEHLFPTQTGEMNISGGLKEGMCLYVKEGGGGPEDKLQAIKYELAQNEEELAQIEEKLAANKEGGSGGGGSGTGFANELGPRLMGKGSGGGGSGPPRKRCCCARRGTQLMLVGLLSTAMWAGLLALLLLWHWETEGGGGSGGGGSEIGTGFPFDPHYVEVLGERMHYVDVGPRDGTPVLFLHGNPTSSYVWRNIIPHVAPTHRVIAPDLIGMGKSDKPDLGYFFDDHVRFMDAFIEALGLEEVVLVIHDWGSALGFHWAKRNPERVKGIAFMEFIRPIPTWDEWPEFARETFQAFRTTDVGRKLIIDQNVFIEGTLPMGVVRPLTEVEMDHYREPFLNPVDREPLWRFPNELPIAGEPANIVALVEEYMDWLHQSPVPKLLFWGTPGVLIPPAEAARLAKSLPNAKAVDIGPGLNLLQEDNPDLIGSEIARWLSTLEISGGGGGSGGGGSAHHFSEPEITLIIFGVMALVIGTILLISYGIRRLIKKSPSGGGGSTGSGGSGFCYENEVGSGRSRFVKKDGHCNVQFINVGSGKSRITSEGEYIPLDQIDINVGSGGSSYTSNRIGTSQVSILFTAQLNETDRNWSCRNRVG

SEQ ID NO: 12 - protein, 933 aa, Artificial
  split intein - heterologous polynucleotide construct
CLDLKTQVQTPQGMKEISNIQVGDLVLSNTGYNEVLNVFPKSKKKSYKITLEDGKEIICSEEHLFPTQTGEMNISGGLKEGMCLYVKEGGGGPEDKLQAIKYELAQNEEELAQIEEKLAANKEGGSGGGGSGTGFANELGPRLMGKGSGGGGSGPPRKRCCCARRGTQLMLVGLLSTAMWAGLLALLLLWHWETEGGGGSGGGGSGGGGSGGGGSRKRTQPTFGFTVNWKFSESTTVFTGQCFIDRNGKEVLKTMWLLRSSVNDIGDDWKATRVGINIFTRLRTQKEGGSGGSARKCSLTGKWTNDLGSNMTIGAVNSRGEFTGTYITAVTATSNEIKESPLHGTQNTINKSGGSTTVFTGQCFIDRNGKEVLKTMWLLRSSVNDIGDDWKATRVGINIFTRLRTQKEGGSGGSARKCSLTGKWTNDLGSNMTIGAVNSRGEFTGTYITAVTATSNEIKESPLHGTQNTINKRTQPTFGFTVNWKFSEGGSGSGSGSGSGRTQPTFGFTVNWKFSESTTVFTGQCFIDRNGKEVLKTMWLLRSSVNDIGDDWKATRVGINIFTRLRTQKEGGSGGSARKCSLTGKWTNDLGSNMTIGAVNSRGEFTGTYITAVTATSNEIKESPLHGTQNTINKSGGSTTVFTGQCFIDRNGKEVLKTMWLLRSSVNDIGDDWKATRVGINIFTRLRTQKEGGSGGSARKCSLTGKWTNDLGSNMTIGAVNSRGEFTGTYITAVTATSNEIKESPLHGTQNTINKRTQPTFGFTVNWKFSEGGGGSGGGGSGGGGSGGGGSAHHFSEPEITLIIFGVMALVIGTILLISYGIRRLIKKSPSGGGGSTGSGGSGFCYENEVGSGRSRFVKKDGHCNVQFINVGSGKSRITSEGEYIPLDQIDINVGSGGSSYTSNRIGTSQVSILFTAQLNETDRNWSCRNRVG

SEQ ID NO: 13 - protein, 415 aa, Artificial
  split intein - heterologous polynucleotide construct
CLDLKTQVQTPQGMKEISNIQVGDLVLSNTGYNEVLNVFPKSKKKSYKITLEDGKEIICSEEHLFPTQTGEMNISGGLKEGMCLYVKEGGGGPEDKLQAIKYELAQNEEELAQIEEKLAANKEGGSVSKGEEDNMASLPATHELHIFGSINGVDFDMVGQGTGNPNDGYEELNLKSTKGDLQFSPWILVPHIGYGFHQYLPYPDGMSPFQAAMVDGSGYQVHRTMQFEDGASLTVNYRYTYEGSHIKGEAQVKGTGFPADGPVMTNSLTAADWCRSKKTYPNDKTIISTFKWSYTTGNGKRYRSTARTTYTFAKPMAANYLKNQPMYVFRKTELKHSKTELNFKEWQKAFTDVMGMDELYKGTGFANELGPRLMGKGSGGSSYTSNRIGTSQVSILFTAQLNETDRNWSCRNRVG

SEQ ID NO: 14 - protein, 391 aa, Artificial
  split intein - heterologous polynucleotide construct
CLDLKTQVQTPQGMKEISNIQVGDLVLSNTGYNEVLNVFPKSKKKSYKITLEDGKEIICSEEHLFPTQTGEMNISGGLKEGMCLYVKEGGGGSGGGGSGGGGSGGGGSGLVPELNEKDDDQVQKALASRENTQLMNRDNIEITVRDFKTLAPRRWLNSGIISFFMKYIEKSTPNTVAFNSFFYTNLSERGYQGVRRWMKRKKTQIDKLDKIFTPINLNQSHWALGIIDLKKKTIGYVDSLSNGPNAMSFAILTDLQKYVMEESKHTIGEDFDLIHLDCPQQPNGYDCGIYVCMNTLYGSADAPLDFDYKDAIRMRRFIAHLILTDALKGGGGSGTGFANELGPRLMGKGSGGGGMMLKKILKIEELDERELIDIEVSGNHLFYANDILTHN

SEQ ID NO: 15 - protein, 436 aa, Artificial
  split intein - heterologous polynucleotide construct
CLDLKTQVQTPQGMKEISNIQVGDLVLSNTGYNEVLNVFPKSKKKSYKITLEDGKEIICSEEHLFPTQTGEMNISGGLKEGMCLYVKEGGGGPEDKLQAIKYELAQNEEELAQIEEKLAANKEGGSGGGGSGGGGSGGGGSGESLFKGPRDYNPISSTICHLTNESDGHTTSLYGIGFGPFIITNKHLFRRNNGTLVVQSLHGVFKVKNTTTLQQHLIDGRDMIIIRMPKDFPPFPQKLKFREPQREERICLVTTNFQTKSMSSMVSDTSCTFPSGDGIFWKHWIQTKDGQCGSPLVSTRDGFIVGIHSASNFTNTNNYFTSVPKNFMELLTNQEAQQWVSGWRLNADSVLWGGHKVFMVKPEEPFQPVKEATQLMNGGGGSGTGFANELGPRLMGKGSGGSSYTSNRIGTSQVSILFTAQLNETDRNWSCRNRVG

SEQ ID NO: 16 - protein, 139 aa, Artificial
  split intein - heterologous polynucleotide construct
LQRGAERVPQEQEEVLQDHPGRWQRDHLLRGTPVPNPDRRDEHLWRPERGHVPVRERRRRRIRVQGRRGQHGQPACHPRAAHLRQHQRRGLRHGGTGHRQPQRRIRGTEPEVHQGGPPVQPLDSGAPHRLRLPPVPALP

SEQ ID NO: 17 - protein, 984 aa, Artificial
  split intein - heterologous polynucleotide construct
CLDLKTQVQTPQGMKEISNIQVGDLVLSNTGYNEVLNVFPKSKKKSYKITLEDGKEIICSEEHLFPTQTGEMNISGGLKEGMCLYVKEGGGGPEDKLQAIKYELAQNEEELAQIEEKLAANKEGGSGGGGSGTGFANELGPRLMGKGSGGGGSGPPRKRCCCARRGTQLMLVGLLSTAMWAGLLALLLLWHWETEGGGGSGGGGSGGGGSGGGGSRKRTQPTFGFTVNWKFSESTTVFTGQCFIDRNGKEVLKTMWLLRSSVNDIGDDWKATRVGINIFTRLRTQKEGGSGGSARKCSLTGKWTNDLGSNMTIGAVNSRGEFTGTYITAVTATSNEIKESPLHGTQNTINKSGGSTTVFTGQCFIDRNGKEVLKTMWLLRSSVNDIGDDWKATRVGINIFTRLRTQKEGGSGGSARKCSLTGKWTNDLGSNMTIGAVNSRGEFTGTYITAVTATSNEIKESPLHGTQNTINKRTQPTFGFTVNWKFSEGGSGSGSGSGSGRTQPTFGFTVNWKFSESTTVFTGQCFIDRNGKEVLKTMWLLRSSVNDIGDDWKATRVGINIFTRLRTQKEGGSGGSARKCSLTGKWTNDLGSNMTIGAVNSRGEFTGTYITAVTATSNEIKESPLHGTQNTINKSGGSTTVFTGQCFIDRNGKEVLKTMWLLRSSVNDIGDDWKATRVGINIFTRLRTQKEGGSGGSARKCSLTGKWTNDLGSNMTIGAVNSRGEFTGTYITAVTATSNEIKESPLHGTQNTINKRTQPTFGFTVNWKFSEGGGGSGGGGSGGGGSGGGGSAHHFSEPEITLIIFGVMALVIGTILLISYGIRRLIKKSPSGGGGSTGSGGSGFCYENEVGSGRSRFVKKDGHCNVQFINVGSGKSRITSEGEYIPLDQIDINVGSGGSSYTSNRIGTSGGSPEDENAALEEKIAQLKQKNAALKEEIQALEYGGGGMMLKKILKIEELDERELIDIEVSGNHLFYANDILTHN

SEQ ID NO: 18 - protein, 703 aa, Artificial
  split intein - heterologous polynucleotide construct
CLDLKTQVQTPQGMKEISNIQVGDLVLSNTGYNEVLNVFPKSKKKSYKITLEDGKEIICSEEHLFPTQTGEMNISGGLKEGMCLYVKEGGGGPEDKLQAIKYELAQNEEELAQIEEKLAANKEGGSGGGGSGTGFANELGPRLMGKGSGGGGSGPPRKRCCCARRGTQLMLVGLLSTAMWAGLLALLLLWHWETEGGGGSGGGGSEIGTGFPFDPHYVEVLGERMHYVDVGPRDGTPVLFLHGNPTSSYVWRNIIPHVAPTHRVIAPDLIGMGKSDKPDLGYFFDDHVRFMDAFIEALGLEEVVLVIHDWGSALGFHWAKRNPERVKGIAFMEFIRPIPTWDEWPEFARETFQAFRTTDVGRKLIIDQNVFIEGTLPMGVVRPLTEVEMDHYREPFLNPVDREPLWRFPNELPIAGEPANIVALVEEYMDWLHQSPVPKLLFWGTPGVLIPPAEAARLAKSLPNAKAVDIGPGLNLLQEDNPDLIGSEIARWLSTLEISGGGGGSGGGGSAHHFSEPEITLIIFGVMALVIGTILLISYGIRRLIKKSPSGGGGSTGSGGSGFCYENEVGSGRSRFVKKDGHCNVQFINVGSGKSRITSEGEYIPLDQIDINVGSGGSSYTSNRIGTSGGSPEDENAALEEKIAQLKQKNAALKEEIQALEYGGGGMMLKKILKIEELDERELIDIEVSGNHLFYANDILTHN

SEQ ID NO: 19 - protein, 584 aa, Artificial
  split intein - heterologous polynucleotide construct
CLDLKTQVQTPQGMKEISNIQVGDLVLSNTGYNEVLNVFPKSKKKSYKITLEDGKEIICSEEHLFPTQTGEMNISGGLKEGMCLYVKEGGGGPEDKLQAIKYELAQNEEELAQIEEKLAANKEGGSGGGGSGTGFANELGPRLMGKGSGGGGSGPPRKRCCCARRGTQLMLVGLLSTAMWAGLLALLLLWHWETEGGGGSGTGSGVFTLEDFVGDWRQTAGYNLDQVLEQGGVSSLFQNLGVSVTPIQRIVLSGENGLKIDIHVIIPYEGLSGDQMGQIEKIFKVVYPVDDHHFKVILHYGTLVIDGVTPNMIDYFGRPYEGIAVFDGKKITVTGTLWNGNKIIDERLINPDGSLLFRVTINGVTGWRLCERILAGTDYKDDDDKGGGGGSAHHFSEPEITLIIFGVMALVIGTILLISYGIRRLIKKSPSGGGGSTGSGGSGFCYENEVGSGRSRFVKKDGHCNVQFINVGSGKSRITSEGEYIPLDQIDINVGSGGSSYTSNRIGTSGGSPEDENAALEEKIAQLKQKNAALKEEIQALEYGGGGMMLKKILKIEELDERELIDIEVSGNHLFYANDILTHN

SEQ ID NO: 20 - protein, 604 aa, Artificial
  split intein - heterologous polynucleotide construct
CLDLKTQVQTPQGMKEISNIQVGDLVLSNTGYNEVLNVFPKSKKKSYKITLEDGKEIICSEEHLFPTQTGEMNISGGLKEGMCLYVKEGGGGPEDKLQAIKYELAQNEEELAQIEEKLAANKEGGSGGGGSGTGFANELGPRLMGKGSGGGGSGPPRKRCCCARRGTQLMLVGLLSTAMWAGLLALLLLWHWETEGGGGSRRRRRKRSARGTGSGVFTLEDFVGDWRQTAGYNLDQVLEQGGVSSLFQNLGVSVTPIQRIVLSGENGLKIDIHVIIPYEGLSGDQMGQIEKIFKVVYPVDDHHFKVILHYGTLVIDGVTPNMIDYFGRPYEGIAVFDGKKITVTGTLWNGNKIIDERLINPDGSLLFRVTINGVTGWRLCERILAGTDYKDDDDKGRRRRRKRSARGGGGSAHHFSEPEITLIIFGVMALVIGTILLISYGIRRLIKKSPSGGGGSTGSGGSGFCYENEVGSGRSRFVKKDGHCNVQFINVGSGKSRITSEGEYIPLDQIDINVGSGGSSYTSNRIGTSGGSPEDENAALEEKIAQLKQKNAALKEEIQALEYGGGGMMLKKILKIEELDERELIDIEVSGNHLFYANDILTHN

SEQ ID NO: 21 - protein, 352 aa, Artificial
  split intein - heterologous polynucleotide construct
CLDLKTQVQTPQGMKEISNIQVGDLVLSNTGYNEVLNVFPKSKKKSYKITLEDGKEIICSEEHLFPTQTGEMNISGGLKEGMCLYVKEGGGGGGSGGGGSGTGFANELGPRLMGKGSGGGGSGVFTLEDFVGDWRQTAGYNLDQVLEQGGVSSLFQNLGVSVTPIQRIVLSGENGLKIDIHVIIPYEGLSGDQMGQIEKIFKVVYPVDDHHFKVILHYGTLVIDGVTPNMIDYFGRPYEGIAVFDGKKITVTGTLWNGNKIIDERLINPDGSLLFRVTINGVTGWRLCERILAGSGGSSYTSNRIGTSGGSGGGGMMLKKILKIEELDERELIDIEVSGNHLFYANDILTHN

SEQ ID NO: 22 - protein, 414 aa, Artificial; identical to SEQ ID NO: 7
  split intein - heterologous polynucleotide construct

SEQ ID NO: 23 - DNA, 8642 bp, Artificial
  Expression vector for Cas9
cccgcctggctgaccgcccaacgacccccgcccattgacgtcaatagtaacgccaatagggactttccattgacgtcaatgggtggagtatttacggtaaactgcccacttggcagtacatcaagtgtatcatatgccaagtacgccccctattgacgtcaatgacggtaaatggcccgcctggcattgtgcccagtacatgaccttatgggactttcctacttggcagtacatctacgtattagtcatcgctattaccatggtcgaggtgagccccacgttctgcttcactctccccatctcccccccctccccacccccaattttgtatttatttattttttaattattttgtgcagcgatgggggcggggggggggggggggcgcgcgccaggcggggcggggcggggcgaggggcggggcggggcgaggcggagaggtgcggcggcagccaatcagagcggcgcgctccgaaagtttccttttatggcgaggcggcggcggcggcggccctataaaaagcgaagcgcgcggcgggcgggagtcgctgcgacgctgccttcgccccgtgccccgctccgccgccgcctcgcgccgcccgccccggctctgactgaccgcgttactcccacaggtgagcgggcgggacggcccttctcctccgggctgtaattagctgagcaagaggtaagggtttaagggatggttggttggtggggtattaatgtttaattacctggagcacctgcctgaaatcactttttttcaggttggatccttaattaataatacgactcactataggggccgccaccatggacaagaagtacagcatcggcctggacatcggcaccaactctgtgggctgggccgtgatcaccgacgagtacaaggtgcccagcaagaaattcaaggtgctgggcaacaccgaccggcacagcatcaagaagaacctgatcggagccctgctgttcgacagcggcgaaacagccgaggccacccggctgaagagaaccgccagaagaagatacaccagacggaagaaccggatctgctatctgcaagagatcttcagcaacgagatggccaaggtggacgacagcttcttccacagactggaagagtccttcctggtggaagaggataagaagcacgagcggcaccccatcttcggcaacatcgtggacgaggtggcctaccacgagaagtaccccaccatctaccacctgagaaagaaactggtggacagcaccgacaaggccgacctgcggctgatctatctggccctggcccacatgatcaagttccggggccacttcctgatcgagggcgacctgaaccccgacaacagcgacgtggacaagctgttcatccagctggtgcagacctacaaccagctgttcgaggaaaaccccatcaacgccagcggcgtggacgccaaggccatcctgtctgccagactgagcaagagcagacggctggaaaatctgatcgcccagctgcccggcgagaagaagaatggcctgttcggcaacctgattgccctgagcctgggcctgacccccaacttcaagagcaacttcgacctggccgaggatgccaaactgcagctgagcaaggacacctacgacgacgacctggacaacctgctggcccagatcggcgaccagtacgccgacctgtttctggccgccaagaacctgtccgacgccatcctgctgagcgacatcctgagagtgaacaccgagatcaccaaggcccccctgagcgcctctatgatcaagagatacgacgagcaccaccaggacctgaccctgctgaaagctctcgtgcggcagcagctgcctgagaagtacaaagagattttcttcgaccagagcaagaacggctacgccggctacattgacggcggagccagccaggaagagttctacaagttcatcaagcccatcctggaaaagatggacggcaccgaggaactgctcgtgaagctgaacagagaggacctgctgcggaagcagcggaccttcgacaacggcagcatcccccaccagatccacctgggagagctgcacgccattctgcggcggcaggaagatttttacccattcctgaaggacaaccgggaaaagatcgagaagatcctgaccttccgcatcccctactacgtgggccctctggccaggggaaacagcagattcgcctggatgaccagaaagagcgaggaaaccatcaccccctggaacttcgaggaagtggtggacaagggcgcttccgcccagagcttcatcgagcggatgaccaacttcgataagaacctgcccaacgagaaggtgctgcccaagcacagcctgctgtacgagtacttcaccgtgtataacgagctgaccaaagtgaaatacgtgaccgagggaatgagaaagcccgccttcctgagcggcgagcagaaaaaggccatcgtggacctgctgttcaagaccaaccggaaagtgaccgtgaagcagctgaaagaggactacttcaagaaaatcgagtgcttcgactccgtggaaatctccggcgtggaagatcggttcaacgcctccctgggcacataccacgatctgctgaaaattatcaaggacaaggacttcctggacaatgaggaaaacgaggacattctggaagatatcgtgctgaccctgacactgtttgaggacagagagatgatcgaggaacggctgaaaacctatgcccacctgttcgacgacaaagtgatgaagcagctgaagcggcggagatacaccggctggggcaggctgagccggaagctgatcaacggcatccgggacaagcagtccggcaagacaatcctggatttcctgaagtccgacggcttcgccaacagaaacttcatgcagctgatccacgacgacagcctgacctttaaagaggacatccagaaagcccaggtgtccggccagggcgatagcctgcacgagcacattgccaatctggccggcagccccgccattaagaagggcatcctgcagacagtgaaggtggtggacgagctcgtgaaagtgatgggccggcacaagcccgagaacatcgtgatcgaaatggccagagagaaccagaccacccagaagggacagaagaacagccgcgagagaatgaagcggatcgaagagggcatcaaagagctgggcagccagatcctgaaagaacaccccgtggaaaacacccagctgcagaacgagaagctgtacctgtactacctgcagaatgggcgggatatgtacgtggaccaggaactggacatcaaccggctgtccgactacgatgtggaccatatcgtgcctcagagctttctgaaggacgactccatcgacaacaaggtgctgaccagaagcgacaagaaccggggcaagagcgacaacgtgccctccgaagaggtcgtgaagaagatgaagaactactggcggcagctgctgaacgccaagctgattacccagagaaagttcgacaatctgaccaaggccgagagaggcggcctgagcgaactggataaggccggcttcatcaagagacagctggtggaaacccggcagatcacaaagcacgtggcacagatcctggactcccggatgaacactaagtacgacgagaatgacaagctgatccgggaagtgaaagtgatcaccctgaagtccaagctggtgtccgatttccggaaggatttccagttttacaaagtgcgcgagatcaacaactaccaccacgcccacgacgcctacctgaacgccgtcgtgggaaccgccctgatcaaaaagtaccctaagctggaaagcgagttcgtgtacggcgactacaaggtgtacgacgtgcggaagatgatcgccaagagcgagcaggaaatcggcaaggctaccgccaagtacttcttctacagcaacatcatgaactttttcaagaccgagattaccctggccaacggcgagatccggaagcggcctctgatcgagacaaacggcgaaaccggggagatcgtgtgggataagggccgggattttgccaccgtgcggaaagtgctgagcatgccccaagtgaatatcgtgaaaaagaccgaggtgcagacaggcggcttcagcaaagagtctatcctgcccaagaggaacagcgataagctgatcgccagaaagaaggactgggaccctaagaagtacggcggcttcgacagccccaccgtggcctattctgtgctggtggtggccaaagtggaaaagggcaagtccaagaaactgaagagtgtgaaagagctgctggggatcaccatcatggaaagaagcagcttcgagaagaatcccatcgactttctggaagccaagggctacaaagaagtgaaaaaggacctgatcatcaagctgcctaagtactccctgttcgagctggaaaacggccggaagagaatgctggcctctgccggcgaactgcagaagggaaacgaactggccctgccctccaaatatgtgaacttcctgtacctggccagccactatgagaagctgaagggctcccccgaggataatgagcagaaacagctgtttgtggaacagcacaagcactacctggacgagatcatcgagcagatcagcgagttctccaagagagtgatcctggccgacgctaatctggacaaagtgctgtccgcctacaacaagcaccgggataagcccatcagagagcaggccgagaatatcatccacctgtttaccctgaccaatctgggagcccctgccgccttcaagtactttgacaccaccatcgaccggaagaggtacaccagcaccaaagaggtgctggacgccaccctgatccaccagagcatcaccggcctgtacgagacacggatcgacctgtctcagctgggaggcgacgcctatccctatgacgtgcccgattatgccagcctgggcagcggctcccccaagaaaaaacgcaaggtggaagatcctaagaaaaagcggaaagtggactgaacgcgtaaatgattgcagatccactagttctagagctcgctgatcagcctcgactgtgccttctagttgccagccatctgttgtttgcccctcccccgtgccttccttgaccctggaaggtgccactcccactgtcctttcctaataaaatgaggaaattgcatcgcattgtctgagtaggtgtcattctattctggggggtggggtggggcaggacagcaagggggaggattgggaagagaatagcaggcatgctggggatgcggtgggctctatggcttctgaggcggaaagaaccagctgggggcggccgcaggaacccctagtgatggagttggccactccctctctgcgcgctcgctcgctcactgaggccgggcgaccaaaggtcgcccgacgcccgggctttgcccgggcggcctcagtgagcgagcgagcgcgcagctgcctgcaggggcgcctgatgcggtattttctccttacgcatctgtgcggtatttcacaccgcatacgtcaaagcaaccatagtacgcgccctgtagcggcgcattaagcgcggcgggtgtggtggttacgcgcagcgtgaccgctacacttgccagcgccctagcgcccgctcctttcgctttcttcccttcctttctcgccacgttcgccggctttccccgtcaagctctaaatcgggggctccctttagggttccgatttagtgctttacggcacctcgaccccaaaaaacttgatttgggtgatggttcacgtagtgggccatcgccctgatagacggtttttcgccctttgacgttggagtccacgttctttaatagtggactcttgttccaaactggaacaacactcaaccctatctcgggctattcttttgatttataagggattttgccgatttcggcctattggttaaaaaatgagctgatttaacaaaaatttaacgcgaattttaacaaaatattaacgtttacaattttatggtgcactctcagtacaatctgctctgatgccgcatagttaagccagccccgacacccgccaacacccgctgacgcgccctgacgggcttgtctgctcccggcatccgcttacagacaagctgtgaccgtctccgggagctgcatgtgtcagaggttttcaccgtcatcaccgaaacgcgcgagacgaaagggcctcgtgatacgcctatttttataggttaatgtcatgataataatggtttcttagacgtcaggtggcacttttcggggaaatgtgcgcggaacccctatttgtttatttttctaaatacattcaaatatgtatccgctcatgagacaataaccctgataaatgcttcaataatattgaaaaaggaagagtatgagtattcaacatttccgtgtcgcccttattcccttttttgcggcattttgccttcctgtttttgctcacccagaaacgctggtgaaagtaaaagatgctgaagatcagttgggtgcacgagtgggttacatcgaactggatctcaacagcggtaagatccttgagagttttcgccccgaagaacgttttccaatgatgagcacttttaaagttctgctatgtggcgcggtattatcccgtattgacgccgggcaagagcaactcggtcgccgcatacactattctcagaatgacttggttgagtactcaccagtcacagaaaagcatcttacggatggcatgacagtaagagaattatgcagtgctgccataaccatgagtgataacactgcggccaacttacttctgacaacgatcggaggaccgaaggagctaaccgcttttttgcacaacatgggggatcatgtaactcgccttgatcgttgggaaccggagctgaatgaagccataccaaacgacgagcgtgacaccacgatgcctgtagcaatggcaacaacgttgcgcaaactattaactggcgaactacttactctagcttcccggcaacaattaatagactggatggaggcggataaagttgcaggaccacttctgcgctcggcccttccggctggctggtttattgctgataaatctggagccggtgagcgtgggtctcgcggtatcattgcagcactggggccagatggtaagccctcccgtatcgtagttatctacacgacggggagtcaggcaactatggatgaacgaaatagacagatcgctgagataggtgcctcactgattaagcattggtaactgtcagaccaagtttactcatatatactttagattgatttaaaacttcatttttaatttaaaaggatctaggtgaagatcctttttgataatctcatgaccaaaatcccttaacgtgagttttcgttccactgagcgtcagaccccgtagaaaagatcaaaggatcttcttgagatcctttttttctgcgcgtaatctgctgcttgcaaacaaaaaaaccaccgctaccagcggtggtttgtttgccggatcaagagctaccaactctttttccgaaggtaactggcttcagcagagcgcagataccaaatactgtccttctagtgtagccgtagttaggccaccacttcaagaactctgtagcaccgcctacatacctcgctctgctaatcctgttaccagtggctgctgccagtggcgataagtcgtgtcttaccgggttggactcaagacgatagttaccggataaggcgcagcggtcgggctgaacggggggttcgtgcacacagcccagcttggagcgaacgacctacaccgaactgagatacctacagcgtgagctatgagaaagcgccacgcttcccgaagggagaaaggcggacaggtatccggtaagcggcagggtcggaacaggagagcgcacgagggagcttccagggggaaacgcctggtatctttatagtcctgtcgggtttcgccacctctgacttgagcgtcgatttttgtgatgctcgtcaggggggcggagcctatggaaaaacgccagcaacgcggcctttttacggttcctggccttttgctggccttttgctcacatgtcctgcaggcagctgcgcgctcgctcgctcactgaggccgcccgggcaaagcccgggcgtcgggcgacctttggtcgcccggcctcagtgagcgagcgagcgcgcagagagggagtggccaactccatcactaggggttcctgcggccgcaaggtcgggcaggaagagggcctatttcccatgattccttcatatttgcatatacgatacaaggctgttagagagataattggaattaatttgactgtaaacacaaagatattagtacaaaatacgtgacgtagaaagtaataatttcttgggtagtttgcagttttaaaattatgttttaaaatggactatcatatgcttaccgtaacttgaaagtatttcgatttcttggctttatatatcttgtggaaaggacgaaacaccgggtcttcgagaagacctgtttaagagctatgctggaaacagcatagcaagtttaaataaggctagtccgttatcaacttgaaaaagtggcaccgagtcggtgctttttttgaattcgtttaaacggtacccgttacataacttacggtaaatgg

SEQ ID NO: 24 - DNA, 8927 bp, Artificial
  Expression vector for Cas9
cccgcctggctgaccgcccaacgacccccgcccattgacgtcaatagtaacgccaatagggactttccattgacgtcaatgggtggagtatttacggtaaactgcccacttggcagtacatcaagtgtatcatatgccaagtacgccccctattgacgtcaatgacggtaaatggcccgcctggcattgtgcccagtacatgaccttatgggactttcctacttggcagtacatctacgtattagtcatcgctattaccatggtcgaggtgagccccacgttctgcttcactctccccatctcccccccctccccacccccaattttgtatttatttattttttaattattttgtgcagcgatgggggcggggggggggggggggcgcgcgccaggcggggcggggcggggcgaggggcggggcggggcgaggcggagaggtgcggcggcagccaatcagagcggcgcgctccgaaagtttccttttatggcgaggcggcggcggcggcggccctataaaaagcgaagcgcgcggcgggcgggagtcgctgcgacgctgccttcgccccgtgccccgctccgccgccgcctcgcgccgcccgccccggctctgactgaccgcgttactcccacaggtgagcgggcgggacggcccttctcctccgggctgtaattagctgagcaagaggtaagggtttaagggatggttggttggtggggtattaatgtttaattacctggagcacctgcctgaaatcactttttttcaggttggatccttaattaataatacgactcactataggggccgccaccatggacaagaagtacagcatcggcctggacatcggcaccaactctgtgggctgggccgtgatcaccgacgagtacaaggtgcccagcaagaaattcaaggtgctgggcaacaccgaccggcacagcatcaagaagaacctgatcggagccctgctgttcgacagcggcgaaacagccgaggccacccggctgaagagaaccgccagaagaagatacaccagacggaagaaccggatctgctatctgcaagagatcttcagcaacgagatggccaaggtggacgacagcttcttccacagactggaagagtccttcctggtggaagaggataagaagcacgagcggcaccccatcttcggcaacatcgtggacgaggtggcctaccacgagaagtaccccaccatctaccacctgagaaagaaactggtggacagcaccgacaaggccgacctgcggctgatctatctggccctggcccacatgatcaagttccggggccacttcctgatcgagggcgacctgaaccccgacaacagcgacgtggacaagctgttcatccagctggtgcagacctacaaccagctgttcgaggaaaaccccatcaacgccagcggcgtggacgccaaggccatcctgtctgccagactgagcaagagcagacggctggaaaatctgatcgcccagctgcccggcgagaagaagaatggcctgttcggcaacctgattgccctgagcctgggcctgacccccaacttcaagagcaacttcgacctggccgaggatgccaaactgcagctgagcaaggacacctacgacgacgacctggacaacctgctggcccagatcggcgaccagtacgccgacctgtttctggccgccaagaacctgtccgacgccatcctgctgagcgacatcctgagagtgaacaccgagatcaccaaggcccccctgagcgcctctatgatcaagagatacgacgagcaccaccaggacctgaccctgctgaaagctctcgtgcggcagcagctgcctgagaagtacaaagagattttcttcgaccagagcaagaacggctacgccggctacattgacggcggagccagccaggaagagttctacaagttcatcaagcccatcctggaaaagatggacggcaccgaggaactgctcgtgaagctgaacagagaggacctgctgcggaagcagcggaccttcgacaacggcagcatcccccaccagatccacctgggagagctgcacgccattctgcggcggcaggaagatttttacccattcctgaaggacaaccgggaaaagatcgagaagatcctgaccttccgcatcccctactacgtgggccctctggccaggggaaacagcagattcgcctggatgaccagaaagagcgaggaaaccatcaccccctggaacttcgaggaagtggtggacaagggcgcttccgcccagagcttcatcgagcggatgaccaacttcgataagaacctgcccaacgagaaggtgctgcccaagcacagcctgctgtacgagtacttcaccgtgtataacgagctgaccaaagtgaaatacgtgaccgagggaatgagaaagcccgccttcctgagcggcgagcagaaaaaggccatcgtggacctgctgttcaagaccaaccggaaagtgaccgtgaagcagctgaaagaggactacttcaagaaaatcgagtgcttcgactccgtggaaatctccggcgtggaagatcggttcaacgcctccctgggcacataccacgatctgctgaaaattatcaaggacaaggacttcctggacaatgaggaaaacgaggacattctggaagatatcgtgctgaccctgacactgtttgaggacagagagatgatcgaggaacggctgaaaacctatgcccacctgttcgacgacaaagtgatgaagcagctgaagcggcggagatacaccggctggggcaggctgagccggaagctgatcaacggcatccgggacaagcagtccggcaagacaatcctggatttcctgaagtccgacggcttcgccaacagaaacttcatgcagctgatccacgacgacagcctgacctttaaagaggacatccagaaagcccaggtgtccggccagggcgatagcctgcacgagcacattgccaatctggccggcagccccgccattaagaagggcatcctgcagacagtgaaggtggtggacgagctcgtgaaagtgatgggccggcacaagcccgagaacatcgtgatcgaaatggccagagagaaccagaccacccagaagggacagaagaacagccgcgagagaatgaagcggatcgaagagggcatcaaagagctgggcagccagatcctgaaagaacaccccgtggaaaacacccagctgcagaacgagaagctgtacctgtactacctgcagaatgggcgggatatgtacgtggaccaggaactggacatcaaccggctgtccgactacgatgtggaccatatcgtgcctcagagctttctgaaggacgactccatcgacaacaaggtgctgaccagaagcgacaagaaccggggcaagagcgacaacgtgccctccgaagaggtcgtgaagaagatgaagaactactggcggcagctgctgaacgccaagctgattacccagagaaagttcgacaatctgaccaaggccgagagaggcggcctgagcgaactggataaggccggcttcatcaagagacagctggtggaaacccggcagatcacaaagcacgtggcacagatcctggactcccggatgaacactaagtacgacgagaatgacaagctgatccgggaagtgaaagtgatcaccctgaagtccaagctggtgtccgatttccggaaggatttccagttttacaaagtgcgcgagatcaacaactaccaccacgcccacgacgcctacctgaacgccgtcgtgggaaccgccctgatcaaaaagtaccctaagctggaaagcgagttcgtgtacggcgactacaaggtgtacgacgtgcggaagatgatcgccaagagcgagcaggaaatcggcaaggctaccgccaagtacttcttctacagcaacatcatgaactttttcaagaccgagattaccctggccaacggcgagatccggaagcggcctctgatcgagacaaacggcgaaaccggggagatcgtgtgggataagggccgggattttgccaccgtgcggaaagtgctgagcatgccccaagtgaatatcgtgaaaaagaccgaggtgcagacaggcggcttcagcaaagagtctatcctgcccaagaggaacagcgataagctgatcgccagaaagaaggactgggaccctaagaagtacggcggcttcgacagccccaccgtggcctattctgtgctggtggtggccaaagtggaaaagggcaagtccaagaaactgaagagtgtgaaagagctgctggggatcaccatcatggaaagaagcagcttcgagaagaatcccatcgactttctggaagccaagggctacaaagaagtgaaaaaggacctgatcatcaagctgcctaagtactccctgttcgagctggaaaacggccggaagagaatgctggcctctgccggcgaactgcagaagggaaacgaactggccctgccctccaaatatgtgaacttcctgtacctggccagccactatgagaagctgaagggctcccccgaggataatgagcagaaacagctgtttgtggaacagcacaagcactacctggacgagatcatcgagcagatcagcgagttctccaagagagtgatcctggccgacgctaatctggacaaagtgctgtccgcctacaacaagcaccgggataagcccatcagagagcaggccgagaatatcatccacctgtttaccctgaccaatctgggagcccctgccgccttcaagtactttgacaccaccatcgaccggaagaggtacaccagcaccaaagaggtgctggacgccaccctgatccaccagagcatcaccggcctgtacgagacacggatcgacctgtctcagctgggaggcgacgcctatccctatgacgtgcccgattatgccagcctgggcagcggctcccccaagaaaaaacgcaaggtggaagatcctaagaaaaagcggaaagtggacggcagcggcgccaccaactttagcttgctgaaacaggctggcgacgttgaagagaatcccgggcctttgattttcgtgaaaacccttaccgggaaaaccatcaccctcgaggttgaaccctcggatacgatagaaaatgtaaaggccaagatccaggataaggaaggaattcctcctgatcagcagagactggcctttgctggcaaatcgctggaagatggacgtactttgtctgactacaatattctaaaggactctaaacttcatcctctgttgagacttcgttgaacgcgtaaatgattgcagatccactagttctagagctcgctgatcagcctcgactgtgccttctagttgccagccatctgttgtttgcccctcccccgtgccttccttgaccctggaaggtgccactcccactgtcctttcctaataaaatgaggaaattgcatcgcattgtctgagtaggtgtcattctattctggggggtggggtggggcaggacagcaagggggaggattgggaagagaatagcaggcatgctggggatgcggtgggctctatggcttctgaggcggaaagaaccagctgggggcggccgcaggaacccctagtgatggagttggccactccctctctgcgcgctcgctcgctcactgaggccgggcgaccaaaggtcgcccgacgcccgggctttgcccgggcggcctcagtgagcgagcgagcgcgcagctgcctgcaggggcgcctgatgcggtattttctccttacgcatctgtgcggtatttcacaccgcatacgtcaaagcaaccatagtacgcgccctgtagcggcgcattaagcgcggcgggtgtggtggttacgcgcagcgtgaccgctacacttgccagcgccctagcgcccgctcctttcgctttcttcccttcctttctcgccacgttcgccggctttccccgtcaagctctaaatcgggggctccctttagggttccgatttagtgctttacggcacctcgaccccaaaaaacttgatttgggtgatggttcacgtagtgggccatcgccctgatagacggtttttcgccctttgacgttggagtccacgttctttaatagtggactcttgttccaaactggaacaacactcaaccctatctcgggctattcttttgatttataagggattttgccgatttcggcctattggttaaaaaatgagctgatttaacaaaaatttaacgcgaattttaacaaaatattaacgtttacaattttatggtgcactctcagtacaatctgctctgatgccgcatagttaagccagccccgacacccgccaacacccgctgacgcgccctgacgggcttgtctgctcccggcatccgcttacagacaagctgtgaccgtctccgggagctgcatgtgtcagaggttttcaccgtcatcaccgaaacgcgcgagacgaaagggcctcgtgatacgcctatttttataggttaatgtcatgataataatggtttcttagacgtcaggtggcacttttcggggaaatgtgcgcggaacccctatttgtttatttttctaaatacattcaaatatgtatccgctcatgagacaataaccctgataaatgcttcaataatattgaaaaaggaagagtatgagtattcaacatttccgtgtcgcccttattcccttttttgcggcattttgccttcctgtttttgctcacccagaaacgctggtgaaagtaaaagatgctgaagatcagttgggtgcacgagtgggttacatcgaactggatctcaacagcggtaagatccttgagagttttcgccccgaagaacgttttccaatgatgagcacttttaaagttctgctatgtggcgcggtattatcccgtattgacgccgggcaagagcaactcggtcgccgcatacactattctcagaatgacttggttgagtactcaccagtcacagaaaagcatcttacggatggcatgacagtaagagaattatgcagtgctgccataaccatgagtgataacactgcggccaacttacttctgacaacgatcggaggaccgaaggagctaaccgcttttttgcacaacatgggggatcatgtaactcgccttgatcgttgggaaccggagctgaatgaagccataccaaacgacgagcgtgacaccacgatgcctgtagcaatggcaacaacgttgcgcaaactattaactggcgaactacttactctagcttcccggcaacaattaatagactggatggaggcggataaagttgcaggaccacttctgcgctcggcccttccggctggctggtttattgctgataaatctggagccggtgagcgtgggtctcgcggtatcattgcagcactggggccagatggtaagccctcccgtatcgtagttatctacacgacggggagtcaggcaactatggatgaacgaaatagacagatcgctgagataggtgcctcactgattaagcattggtaactgtcagaccaagtttactcatatatactttagattgatttaaaacttcatttttaatttaaaaggatctaggtgaagatcctttttgataatctcatgaccaaaatcccttaacgtgagttttcgttccactgagcgtcagaccccgtagaaaagatcaaaggatcttcttgagatcctttttttctgcgcgtaatctgctgcttgcaaacaaaaaaaccaccgctaccagcggtggtttgtttgccggatcaagagctaccaactctttttccgaaggtaactggcttcagcagagcgcagataccaaatactgtccttctagtgtagccgtagttaggccaccacttcaagaactctgtagcaccgcctacatacctcgctctgctaatcctgttaccagtggctgctgccagtggcgataagtcgtgtcttaccgggttggactcaagacgatagttaccggataaggcgcagcggtcgggctgaacggggggttcgtgcacacagcccagcttggagcgaacgacctacaccgaactgagatacctacagcgtgagctatgagaaagcgccacgcttcccgaagggagaaaggcggacaggtatccggtaagcggcagggtcggaacaggagagcgcacgagggagcttccagggggaaacgcctggtatctttatagtcctgtcgggtttcgccacctctgacttgagcgtcgatttttgtgatgctcgtcaggggggcggagcctatggaaaaacgccagcaacgcggcctttttacggttcctggccttttgctggccttttgctcacatgtcctgcaggcagctgcgcgctcgctcgctcactgaggccgcccgggcaaagcccgggcgtcgggcgacctttggtcgcccggcctcagtgagcgagcgagcgcgcagagagggagtggccaactccatcactaggggttcctgcggccgcaaggtcgggcaggaagagggcctatttcccatgattccttcatatttgcatatacgatacaaggctgttagagagataattggaattaatttgactgtaaacacaaagatattagtacaaaatacgtgacgtagaaagtaataatttcttgggtagtttgcagttttaaaattatgttttaaaatggactatcatatgcttaccgtaacttgaaagtatttcgatttcttggctttatatatcttgtggaaaggacgaaacaccgggtcttcgagaagacctgtttaagagctatgctggaaacagcatagcaagtttaaataaggctagtccgttatcaacttgaaaaagtggcaccgagtcggtgctttttttgaattcgtttaaacggtacccgttacataacttacggtaaatgg

SEQ ID NO: 25 - DNA, 7723 bp, Artificial
  Expression vector for Cas9
cccgcctggctgaccgcccaacgacccccgcccattgacgtcaatagtaacgccaatagggactttccattgacgtcaatgggtggagtatttacggtaaactgcccacttggcagtacatcaagtgtatcatatgccaagtacgccccctattgacgtcaatgacggtaaatggcccgcctggcattgtgcccagtacatgaccttatgggactttcctacttggcagtacatctacgtattagtcatcgctattaccatggtcgaggtgagccccacgttctgcttcactctccccatctcccccccctccccacccccaattttgtatttatttattttttaattattttgtgcagcgatgggggcggggggggggggggggcgcgcgccaggcggggcggggcggggcgaggggcggggcggggcgaggcggagaggtgcggcggcagccaatcagagcggcgcgctccgaaagtttccttttatggcgaggcggcggcggcggcggccctataaaaagcgaagcgcgcggcgggcgggagtcgctgcgacgctgccttcgccccgtgccccgctccgccgccgcctcgcgccgcccgccccggctctgactgaccgcgttactcccacaggtgagcgggcgggacggcccttctcctccgggctgtaattagctgagcaagaggtaagggtttaagggatggttggttggtggggtattaatgtttaattacctggagcacctgcctgaaatcactttttttcaggttggatccttaattaataatacgactcactataggggccgccaccatgaagaggaactacatcctcggcctggacatcggcatcacatctgtcggctacggcatcatcgactacgagacaagggacgtgatcgacgctggcgtgcggctgttcaaagaggccaacgtcgagaacaacgagggcagaagatccaagagaggcgccagaaggctgaagagaagaaggcggcacagaatccagagagtgaagaagctgctgttcgactacaacctgctgaccgaccacagcgagctgagcggcatcaatccttacgaggccagagtgaagggcctgagccagaagctgagcgaggaagagttctctgccgctctgctgcacctggctaaaagacggggagtgcacaacgtgaacgaggtggaagaggacaccggcaacgagctgtccaccaaagagcagatcagcagaaacagcaaggccctggaagagaaatacgtggccgagctgcaactggaaaggctgaaaaaggacggcgaagtgcggggcagcatcaacagattcaagaccagcgactacgtgaaagaggctaagcagctcctgaaggtgcagaaggcttaccaccagctggaccagagcttcatcgacacctacatcgacctgctggaaaccagaaggacctactacgaaggacctggcgagggcagcccttttggctggaaggacatcaaagaatggtacgagatgctgatgggccactgcacatacttccccgaggaactgagaagcgtgaagtacgcctacaacgccgacctgtacaacgccctgaacgacctgaacaacctcgtgatcaccagggacgagaacgagaagctggaatattacgagaagttccagatcatcgagaacgtgttcaagcagaagaagaagcccacactgaagcagatcgccaaagagatcctcgtcaacgaggaagatattaagggctacagagtgaccagcaccggcaagcccgagttcaccaatctgaaggtgtaccacgacatcaaggacattaccgctcggaaagaaatcatcgaaaacgctgagctgctggaccaaatcgccaagatcctgaccatctaccagagcagcgaggacattcaagaagaactgaccaacctgaactccgagctgacccaagaggaaatcgagcagattagcaacctgaagggatacaccggcacacacaacctgagcctgaaggccatcaacctgatcctggacgagctgtggcacaccaacgacaaccagatcgctatcttcaacaggctgaagctggtgcctaagaaggtggacctgtcacagcagaaagagattcctacaacactggtggacgacttcatcctgtctccagtggtcaagcgcagcttcatccagagcatcaaagtgatcaacgccatcatcaagaagtacggcctgcctaacgacatcatcatcgagctggctagagagaagaactccaaggacgcccagaaaatgatcaacgagatgcagaagagaaaccggcagaccaacgagaggatcgaggaaatcatcagaaccaccggcaaagagaacgccaagtacctgatcgagaagatcaagctgcacgacatgcaagagggcaagtgcctgtacagcctggaagctatccctcttgaggacctgctgaacaatcccttcaactatgaggtggaccacatcatccccagaagcgtgtccttcgacaacagcttcaacaacaaggtgctcgtgaagcaagaagagaactccaagaagggcaacagaaccccattccagtacctgagcagcagcgacagcaagatcagctacgagactttcaagaagcacatcctgaacctcgccaaaggcaagggccgcatcagcaagaccaagaaagagtatctgctggaagaacgggacatcaacaggttctccgtgcagaaagacttcatcaaccggaacctggtggacaccagatacgccacaaggggcctgatgaatctgctgagaagctacttccgcgtgaacaatctggacgtgaaagtcaagtccatcaacggcggcttcaccagctttctgagaagaaagtggaagtttaagaaagagcggaacaaggggtacaagcaccacgccgaggacgccctgatcattgccaacgccgatttcatcttcaaagagtggaagaaactggacaaggcaaagaaagtgatggaaaaccagatgttcgaggaaaagcaggccgagagcatgcccgagatcgagacagagcaagagtacaaagaaatcttcatcacgccccaccagatcaagcacattaaggacttcaaggactacaagtacagccaccgcgtggacaagaagcctaacagagagctgattaacgacaccctgtactccaccagaaaggacgacaagggaaacaccctgatcgtcaacaacctgaatggcctgtacgacaaggacaacgacaagctcaagaagctgatcaacaagagccccgaaaagctgctgatgtaccaccacgatcctcagacctaccagaaactgaagctcatcatggaacagtacggcgacgagaagaaccctctgtacaagtactacgaggaaaccgggaactacctgaccaagtactccaaaaaggataacggccccgtgatcaagaagattaagtattacggcaacaagctgaacgcccacctggacatcaccgacgactaccctaactccagaaacaaggtcgtgaagctgtccctgaagccttacagattcgacgtgtacctggacaacggcgtgtacaagttcgtgaccgtgaagaacctggatgtgatcaaaaaagaaaactactatgaagtgaacagcaagtgctatgaggaagccaaaaagctgaagaagatcagcaaccaggctgagtttatcgcctccttctacaacaacgatctgatcaagatcaacggggagctgtatagagtgatcggagtgaacaacgacctgctcaacaggatcgaagtgaatatgatcgacatcacctaccgcgagtacctggaaaacatgaacgacaagaggccacctcggatcattaagacaatcgccagcaagacgcagagcattaagaagtacagcacagacatcctgggcaacctgtacgaagtgaagtctaagaagcacccgcagattatcaagaaaggcggatccacaccgcctaagaaaaagagaaaggtcgaggacggcgagggcccagctgccaaaagagtgaaactggattccggagccgctcctgccgccaagaagaaaaagctggattacaaggacgacgatgacaagtgaacgcgtaaatgattgcagatccactagttctagagctcgctgatcagcctcgactgtgccttctagttgccagccatctgttgtttgcccctcccccgtgccttccttgaccctggaaggtgccactcccactgtcctttcctaataaaatgaggaaattgcatcgcattgtctgagtaggtgtcattctattctggggggtggggtggggcaggacagcaagggggaggattgggaagagaatagcaggcatgctggggatgcggtgggctctatggcttctgaggcggaaagaaccagctgggggcggccgcaggaacccctagtgatggagttggccactccctctctgcgcgctcgctcgctcactgaggccgggcgaccaaaggtcgcccgacgcccgggctttgcccgggcggcctcagtgagcgagcgagcgcgcagctgcctgcaggggcgcctgatgcggtattttctccttacgcatctgtgcggtatttcacaccgcatacgtcaaagcaaccatagtacgcgccctgtagcggcgcattaagcgcggcgggtgtggtggttacgcgcagcgtgaccgctacacttgccagcgccctagcgcccgctcctttcgctttcttcccttcctttctcgccacgttcgccggctttccccgtcaagctctaaatcgggggctccctttagggttccgatttagtgctttacggcacctcgaccccaaaaaacttgatttgggtgatggttcacgtagtgggccatcgccctgatagacggtttttcgccctttgacgttggagtccacgttctttaatagtggactcttgttccaaactggaacaacactcaaccctatctcgggctattcttttgatttataagggattttgccgatttcggcctattggttaaaaaatgagctgatttaacaaaaatttaacgcgaattttaacaaaatattaacgtttacaattttatggtgcactctcagtacaatctgctctgatgccgcatagttaagccagccccgacacccgccaacacccgctgacgcgccctgacgggcttgtctgctcccggcatccgcttacagacaagctgtgaccgtctccgggagctgcatgtgtcagaggttttcaccgtcatcaccgaaacgcgcgagacgaaagggcctcgtgatacgcctatttttataggttaatgtcatgataataatggtttcttagacgtcaggtggcacttttcggggaaatgtgcgcggaacccctatttgtttatttttctaaatacattcaaatatgtatccgctcatgagacaataaccctgataaatgcttcaataatattgaaaaaggaagagtatgagtattcaacatttccgtgtcgcccttattcccttttttgcggcattttgccttcctgtttttgctcacccagaaacgctggtgaaagtaaaagatgctgaagatcagttgggtgcacgagtgggttacatcgaactggatctcaacagcggtaagatccttgagagttttcgccccgaagaacgttttccaatgatgagcacttttaaagttctgctatgtggcgcggtattatcccgtattgacgccgggcaagagcaactcggtcgccgcatacactattctcagaatgacttggttgagtactcaccagtcacagaaaagcatcttacggatggcatgacagtaagagaattatgcagtgctgccataaccatgagtgataacactgcggccaacttacttctgacaacgatcggaggaccgaaggagctaaccgcttttttgcacaacatgggggatcatgtaactcgccttgatcgttgggaaccggagctgaatgaagccataccaaacgacgagcgtgacaccacgatgcctgtagcaatggcaacaacgttgcgcaaactattaactggcgaactacttactctagcttcccggcaacaattaatagactggatggaggcggataaagttgcaggaccacttctgcgctcggcccttccggctggctggtttattgctgataaatctggagccggtgagcgtgggtctcgcggtatcattgcagcactggggccagatggtaagccctcccgtatcgtagttatctacacgacggggagtcaggcaactatggatgaacgaaatagacagatcgctgagataggtgcctcactgattaagcattggtaactgtcagaccaagtttactcatatatactttagattgatttaaaacttcatttttaatttaaaaggatctaggtgaagatcctttttgataatctcatgaccaaaatcccttaacgtgagttttcgttccactgagcgtcagaccccgtagaaaagatcaaaggatcttcttgagatcctttttttctgcgcgtaatctgctgcttgcaaacaaaaaaaccaccgctaccagcggtggtttgtttgccggatcaagagctaccaactctttttccgaaggtaactggcttcagcagagcgcagataccaaatactgtccttctagtgtagccgtagttaggccaccacttcaagaactctgtagcaccgcctacatacctcgctctgctaatcctgttaccagtggctgctgccagtggcgataagtcgtgtcttaccgggttggactcaagacgatagttaccggataaggcgcagcggtcgggctgaacggggggttcgtgcacacagcccagcttggagcgaacgacctacaccgaactgagatacctacagcgtgagctatgagaaagcgccacgcttcccgaagggagaaaggcggacaggtatccggtaagcggcagggtcggaacaggagagcgcacgagggagcttccagggggaaacgcctggtatctttatagtcctgtcgggtttcgccacctctgacttgagcgtcgatttttgtgatgctcgtcaggggggcggagcctatggaaaaacgccagcaacgcggcctttttacggttcctggccttttgctggccttttgctcacatgtcctgcaggcagctgcgcgctcgctcgctcactgaggccgcccgggcaaagcccgggcgtcgggcgacctttggtcgcccggcctcagtgagcgagcgagcgcgcagagagggagtggccaactccatcactaggggttcctgcggccgcaaggtcgggcaggaagagggcctatttcccatgattccttcatatttgcatatacgatacaaggctgttagagagataattggaattaatttgactgtaaacacaaagatattagtacaaaatacgtgacgtagaaagtaataatttcttgggtagtttgcagttttaaaattatgttttaaaatggactatcatatgcttaccgtaacttgaaagtatttcgatttcttggctttatatatcttgtggaaaggacgaaacaccgggtcttcgagaagacctgttatagtactctggaaacagaatctactataacaaggcaaaatgccgtgtttatctcgtcaacttgttggcgagatttttttgaattcgtttaaacggtacccgttacataacttacggtaaatgg

SEQ ID NO: 26 - DNA, 8008 bp, Artificial
  Expression vector for Cas9
cccgcctggctgaccgcccaacgacccccgcccattgacgtcaatagtaacgccaatagggactttccattgacgtcaatgggtggagtatttacggtaaactgcccacttggcagtacatcaagtgtatcatatgccaagtacgccccctattgacgtcaatgacggtaaatggcccgcctggcattgtgcccagtacatgaccttatgggactttcctacttggcagtacatctacgtattagtcatcgctattaccatggtcgaggtgagccccacgttctgcttcactctccccatctcccccccctccccacccccaattttgtatttatttattttttaattattttgtgcagcgatgggggcggggggggggggggggcgcgcgccaggcggggcggggcggggcgaggggcggggcggggcgaggcggagaggtgcggcggcagccaatcagagcggcgcgctccgaaagtttccttttatggcgaggcggcggcggcggcggccctataaaaagcgaagcgcgcggcgggcgggagtcgctgcgacgctgccttcgccccgtgccccgctccgccgccgcctcgcgccgcccgccccggctctgactgaccgcgttactcccacaggtgagcgggcgggacggcccttctcctccgggctgtaattagctgagcaagaggtaagggtttaagggatggttggttggtggggtattaatgtttaattacctggagcacctgcctgaaatcactttttttcaggttggatccttaattaataatacgactcactataggggccgccaccatgaagaggaactacatcctcggcctggacatcggcatcacatctgtcggctacggcatcatcgactacgagacaagggacgtgatcgacgctggcgtgcggctgttcaaagaggccaacgtcgagaacaacgagggcagaagatccaagagaggcgccagaaggctgaagagaagaaggcggcacagaatccagagagtgaagaagctgctgttcgactacaacctgctgaccgaccacagcgagctgagcggcatcaatccttacgaggccagagtgaagggcctgagccagaagctgagcgaggaagagttctctgccgctctgctgcacctggctaaaagacggggagtgcacaacgtgaacgaggtggaagaggacaccggcaacgagctgtccaccaaagagcagatcagcagaaacagcaaggccctggaagagaaatacgtggccgagctgcaactggaaaggctgaaaaaggacggcgaagtgcggggcagcatcaacagattcaagaccagcgactacgtgaaagaggctaagcagctcctgaaggtgcagaaggcttaccaccagctggaccagagcttcatcgacacctacatcgacctgctggaaaccagaaggacctactacgaaggacctggcgagggcagcccttttggctggaaggacatcaaagaatggtacgagatgctgatgggccactgcacatacttccccgaggaactgagaagcgtgaagtacgcctacaacgccgacctgtacaacgccctgaacgacctgaacaacctcgtgatcaccagggacgagaacgagaagctggaatattacgagaagttccagatcatcgagaacgtgttcaagcagaagaagaagcccacactgaagcagatcgccaaagagatcctcgtcaacgaggaagatattaagggctacagagtgaccagcaccggcaagcccgagttcaccaatctgaaggtgtaccacgacatcaaggacattaccgctcggaaagaaatcatcgaaaacgctgagctgctggaccaaatcgccaagatcctgaccatctaccagagcagcgaggacattcaagaagaactgaccaacctgaactccgagctgacccaagaggaaatcgagcagattagcaacctgaagggatacaccggcacacacaacctgagcctgaaggccatcaacctgatcctggacgagctgtggcacaccaacgacaaccagatcgctatcttcaacaggctgaagctggtgcctaagaaggtggacctgtcacagcagaaagagattcctacaacactggtggacgacttcatcctgtctccagtggtcaagcgcagcttcatccagagcatcaaagtgatcaacgccatcatcaagaagtacggcctgcctaacgacatcatcatcgagctggctagagagaagaactccaaggacgcccagaaaatgatcaacgagatgcagaagagaaaccggcagaccaacgagaggatcgaggaaatcatcagaaccaccggcaaagagaacgccaagtacctgatcgagaagatcaagctgcacgacatgcaagagggcaagtgcctgtacagcctggaagctatccctcttgaggacctgctgaacaatcccttcaactatgaggtggaccacatcatccccagaagcgtgtccttcgacaacagcttcaacaacaaggtgctcgtgaagcaagaagagaactccaagaagggcaacagaaccccattccagtacctgagcagcagcgacagcaagatcagctacgagactttcaagaagcacatcctgaacctcgccaaaggcaagggccgcatcagcaagaccaagaaagagtatctgctggaagaacgggacatcaacaggttctccgtgcagaaagacttcatcaaccggaacctggtggacaccagatacgccacaaggggcctgatgaatctgctgagaagctacttccgcgtgaacaatctggacgtgaaagtcaagtccatcaacggcggcttcaccagctttctgagaagaaagtggaagtttaagaaagagcggaacaaggggtacaagcaccacgccgaggacgccctgatcattgccaacgccgatttcatcttcaaagagtggaagaaactggacaaggcaaagaaagtgatggaaaaccagatgttcgaggaaaagcaggccgagagcatgcccgagatcgagacagagcaagagtacaaagaaatcttcatcacgccccaccagatcaagcacattaaggacttcaaggactacaagtacagccaccgcgtggacaagaagcctaacagagagctgattaacgacaccctgtactccaccagaaaggacgacaagggaaacaccctgatcgtcaacaacctgaatggcctgtacgacaaggacaacgacaagctcaagaagctgatcaacaagagccccgaaaagctgctgatgtaccaccacgatcctcagacctaccagaaactgaagctcatcatggaacagtacggcgacgagaagaaccctctgtacaagtactacgaggaaaccgggaactacctgaccaagtactccaaaaaggataacggccccgtgatcaagaagattaagtattacggcaacaagctgaacgcccacctggacatcaccgacgactaccctaactccagaaacaaggtcgtgaagctgtccctgaagccttacagattcgacgtgtacctggacaacggcgtgtacaagttcgtgaccgtgaagaacctggatgtgatcaaaaaagaaaactactatgaagtgaacagcaagtgctatgaggaagccaaaaagctgaagaagatcagcaaccaggctgagtttatcgcctccttctacaacaacgatctgatcaagatcaacggggagctgtatagagtgatcggagtgaacaacgacctgctcaacaggatcgaagtgaatatgatcgacatcacctaccgcgagtacctggaaaacatgaacgacaagaggccacctcggatcattaagacaatcgccagcaagacgcagagcattaagaagtacagcacagacatcctgggcaacctgtacgaagtgaagtctaagaagcacccgcagattatcaagaaaggcggatccacaccgcctaagaaaaagagaaaggtcgaggacggcgagggcccagctgccaaaagagtgaaactggattccggagccgctcctgccgccaagaagaaaaagctggattacaaggacgacgatgacaagggcagcggcgccaccaactttagcttgctgaaacaggctggcgacgttgaagagaatcccgggcctttgattttcgtgaaaacccttaccgggaaaaccatcaccctcgaggttgaaccctcggatacgatagaaaatgtaaaggccaagatccaggataaggaaggaattcctcctgatcagcagagactggcctttgctggcaaatcgctggaagatggacgtactttgtctgactacaatattctaaaggactctaaacttcatcctctgttgagacttcgttgaacgcgtaaatgattgcagatccactagttctagagctcgctgatcagcctcgactgtgccttctagttgccagccatctgttgtttgcccctcccccgtgccttccttgaccctggaaggtgccactcccactgtcctttcctaataaaatgaggaaattgcatcgcattgtctgagtaggtgtcattctattctggggggtggggtggggcaggacagcaagggggaggattgggaagagaatagcaggcatgctggggatgcggtgggctctatggcttctgaggcggaaagaaccagctgggggcggccgcaggaacccctagtgatggagttggccactccctctctgcgcgctcgctcgctcactgaggccgggcgaccaaaggtcgcccgacgcccgggctttgcccgggcggcctcagtgagcgagcgagcgcgcagctgcctgcaggggcgcctgatgcggtattttctccttacgcatctgtgcggtatttcacaccgcatacgtcaaagcaaccatagtacgcgccctgtagcggcgcattaagcgcggcgggtgtggtggttacgcgcagcgtgaccgctacacttgccagcgccctagcgcccgctcctttcgctttcttcccttcctttctcgccacgttcgccggctttccccgtcaagctctaaatcgggggctccctttagggttccgatttagtgctttacggcacctcgaccccaaaaaacttgatttgggtgatggttcacgtagtgggccatcgccctgatagacggtttttcgccctttgacgttggagtccacgttctttaatagtggactcttgttccaaactggaacaacactcaaccctatctcgggctattcttttgatttataagggattttgccgatttcggcctattggttaaaaaatgagctgatttaacaaaaatttaacgcgaattttaacaaaatattaacgtttacaattttatggtgcactctcagtacaatctgctctgatgccgcatagttaagccagccccgacacccgccaacacccgctgacgcgccctgacgggcttgtctgctcccggcatccgcttacagacaagctgtgaccgtctccgggagctgcatgtgtcagaggttttcaccgtcatcaccgaaacgcgcgagacgaaagggcctcgtgatacgcctatttttataggttaatgtcatgataataatggtttcttagacgtcaggtggcacttttcggggaaatgtgcgcggaacccctatttgtttatttttctaaatacattcaaatatgtatccgctcatgagacaataaccctgataaatgcttcaataatattgaaaaaggaagagtatgagtattcaacatttccgtgtcgcccttattcccttttttgcggcattttgccttcctgtttttgctcacccagaaacgctggtgaaagtaaaagatgctgaagatcagttgggtgcacgagtgggttacatcgaactggatctcaacagcggtaagatccttgagagttttcgccccgaagaacgttttccaatgatgagcacttttaaagttctgctatgtggcgcggtattatcccgtattgacgccgggcaagagcaactcggtcgccgcatacactattctcagaatgacttggttgagtactcaccagtcacagaaaagcatcttacggatggcatgacagtaagagaattatgcagtgctgccataaccatgagtgataacactgcggccaacttacttctgacaacgatcggaggaccgaaggagctaaccgcttttttgcacaacatgggggatcatgtaactcgccttgatcgttgggaaccggagctgaatgaagccataccaaacgacgagcgtgacaccacgatgcctgtagcaatggcaacaacgttgcgcaaactattaactggcgaactacttactctagcttcccggcaacaattaatagactggatggaggcggataaagttgcaggaccacttctgcgctcggcccttccggctggctggtttattgctgataaatctggagccggtgagcgtgggtctcgcggtatcattgcagcactggggccagatggtaagccctcccgtatcgtagttatctacacgacggggagtcaggcaactatggatgaacgaaatagacagatcgctgagataggtgcctcactgattaagcattggtaactgtcagaccaagtttactcatatatactttagattgatttaaaacttcatttttaatttaaaaggatctaggtgaagatcctttttgataatctcatgaccaaaatcccttaacgtgagttttcgttccactgagcgtcagaccccgtagaaaagatcaaaggatcttcttgagatcctttttttctgcgcgtaatctgctgcttgcaaacaaaaaaaccaccgctaccagcggtggtttgtttgccggatcaagagctaccaactctttttccgaaggtaactggcttcagcagagcgcagataccaaatactgtccttctagtgtagccgtagttaggccaccacttcaagaactctgtagcaccgcctacatacctcgctctgctaatcctgttaccagtggctgctgccagtggcgataagtcgtgtcttaccgggttggactcaagacgatagttaccggataaggcgcagcggtcgggctgaacggggggttcgtgcacacagcccagcttggagcgaacgacctacaccgaactgagatacctacagcgtgagctatgagaaagcgccacgcttcccgaagggagaaaggcggacaggtatccggtaagcggcagggtcggaacaggagagcgcacgagggagcttccagggggaaacgcctggtatctttatagtcctgtcgggtttcgccacctctgacttgagcgtcgatttttgtgatgctcgtcaggggggcggagcctatggaaaaacgccagcaacgcggcctttttacggttcctggccttttgctggccttttgctcacatgtcctgcaggcagctgcgcgctcgctcgctcactgaggccgcccgggcaaagcccgggcgtcgggcgacctttggtcgcccggcctcagtgagcgagcgagcgcgcagagagggagtggccaactccatcactaggggttcctgcggccgcaaggtcgggcaggaagagggcctatttcccatgattccttcatatttgcatatacgatacaaggctgttagagagataattggaattaatttgactgtaaacacaaagatattagtacaaaatacgtgacgtagaaagtaataatttcttgggtagtttgcagttttaaaattatgttttaaaatggactatcatatgcttaccgtaacttgaaagtatttcgatttcttggctttatatatcttgtggaaaggacgaaacaccgggtcttcgagaagacctgttatagtactctggaaacagaatctactataacaaggcaaaatgccgtgtttatctcgtcaacttgttggcgagatttttttgaattcgtttaaacggtacccgttacataacttacggtaaatgg

SEQ ID NO: 27 - DNA, 6169 bp, Artificial
  Expression vector for Flp recombinase
ggcgcgccggattcgacattgattattgactagttattaatagtaatcaattacggggtcattagttcatagcccatatatggagttccgcgttacataacttacggtaaatggcccgcctggctgaccgcccaacgacccccgcccattgacgtcaataatgacgtatgttcccatagtaacgccaatagggactttccattgacgtcaatgggtggagtatttacggtaaactgcccacttggcagtacatcaagtgtatcatatgccaagtacgccccctattgacgtcaatgacggtaaatggcccgcctggcattatgcccagtacatgaccttatgggactttcctacttggcagtacatctacgtattagtcatcgctattaccatggtcgaggtgagccccacgttctgcttcactctccccatctcccccccctccccacccccaattttgtatttatttattttttaattattttgtgcagcgatgggggcggggggggggggggggcgcgcgccaggcggggcggggcggggcgaggggcggggcggggcgaggcggagaggtgcggcggcagccaatcagagcggcgcgctccgaaagtttccttttatggcgaggcggcggcggcggcggccctataaaaagcgaagcgcgcggcgggcgggagtcgctgcgtcgcgccttcgccccgtgccccgctccgccgccgcctcgcgccgcccgccccggctctgactgaccgcgttactcccacaggtgagcgggcgggacggcccttctcctccgggctgtaattagcgcttggtttaatgacggctcgtttcttttctgtggctgcgtgaaagccttaaagggctccgggagggccctttgtgcgggggggagcggctcggggggtgcgtgcgtgtgtgtgtgcgtggggagcgccgcgtgcggcccgcgctgcccggcggctgtgagcgctgcgggcgcggcgcggggctttgtgcgctccgcgtgtgcgcgaggggagcgcggccgggggcggtgccccgcggtgcgggggggctgcgaggggaacaaaggctgcgtgcggggtgtgtgcgtgggggggtgagcagggggtgtgggcgcggcggtcgggctgtaacccccccctgcacccccctccccgagttgctgagcacggcccggcttcgggtgcggggctccgtgcggggcgtggcgcggggctcgccgtgccgggcggggggtggcggcaggtgggggtgccgggcggggcggggccgcctcgggccggggagggctcgggggaggggcgcggcggccccggagcgccggcggctgtcgaggcgcggcgagccgcagccattgccttttatggtaatcgtgcgagagggcgcagggacttcctttgtcccaaatctggcggagccgaaatctgggaggcgccgccgcaccccctctagcgggcgcgggcgaagcggtgcggcgccggcaggaaggaaatgggcggggagggccttcgtgcgtcgccgcgccgccgtccccttctccatctccagcctcggggctgccgcagggggacggctgccttcgggggggacggggcagggcggggttcggcttctggcgtgtgaccggcggctctagagcctctgctaaccatgttcatgccttcttctttttcctacagatccttaattaataatacgactcactataggggccgccaccatgagccagttcgacatcctgtgcaagacccctccaaaggtgctcgtgcggcagttcgtggaaagattcgagaggcctagcggcgagaagatcgcctcttgtgctgccgagctgacctacctgtgctggatgatcacccacaacggcaccgccatcaagagggccaccttcatgagctacaacaccatcatcagcaacagcctgagcttcgacatcgtgaacaagagcctccagttcaagtacaagacccagaaggctaccatcctggaagccagcctgaagaagctgatccccgcctgggagttcacaatcatcccttacaacggccagaagcaccagagcgacatcacagacatcgtgtccagcctccagctccagttcgagtctagcgaggaagccgacaagggcaacagccacagcaagaagatgctgaaggccctgctgagcgagggcgagtctatctgggagatcacagagaagatcctgaacagcttcgagtacaccagccggttcaccaagacaaagaccctgtaccagttcctgttcctggctaccttcatcaactgcggcagattctccgacatcaagaacgtggaccccaagagcttcaagctggtgcagaacaagtacctgggcgtgatcattcagtgcctcgtgaccgagactaagaccagcgtgtccagacacatctactttttcagcgccagaggcagaatcgaccctctggtgtacctggacgagttcctgagaaacagcgagcccgtgctgaagagagtgaacagaaccggcaacagcagctccaacaagcaagagtaccagctgctgaaggacaacctcgtgcggtcctacaacaaggctctgaagaagaacgccccgtatcctatcttcgccattaagaacggccctaagagccacatcggcagacacctgatgaccagctttctgagcatgaagggcctgacagagctgaccaacgtcgtcggcaattggagcgataagagagcctctgccgtcgccagaaccacctacacacaccagatcacagctatccccgaccactacttcgccctggtgtctaggtactacgcctacgatcccatcagcaaagagatgatcgccctgaaggacgagacaaaccccatcgaggaatggcagcacatcgagcagctgaagggatctgccgagggcagcatcagataccctgcttggaacggcatcatctcccaagaggtgctggactacctgagcagctacatcaacagaagaatcggcggcagcggcggatcccctgctgctaaaagagtgaagctggactccggatgaacgcgtaaatgattgcagatccactagttctagagctcgctgatcagcctcgactgtgccttctagttgccagccatctgttgtttgcccctcccccgtgccttccttgaccctggaaggtgccactcccactgtcctttcctaataaaatgaggaaattgcatcgcattgtctgagtaggtgtcattctattctggggggtggggtggggcaggacagcaagggggaggattgggaagacaatagcaggcatgctggggatgcggtgggctctatggcttctgaggcggaaagaaccagctggggctcgagatccactagttctagcctcgaggctagagcggccgccactggccgtcgttttacaacgtcgtgactgggaaaaccctggcgttacccaacttaatcgccttgcagcacatccccctttcgccagctggcgtaatagcgaagaggcccgcaccgatcgcccttcccaacagttgcgcagcctgaatggcgaatgggacgcgccctgtagcggcgcattaagcgcggcgggtgtggtggttacgcgcagcgtgaccgctacacttgccagcgccctagcgcccgctcctttcgctttcttcccttcctttctcgccacgttcgccggctttccccgtcaagctctaaatcgggggctccctttagggttccgatttagtgctttacggcacctcgaccccaaaaaacttgattagggtgatggttcacgtagtgggccatcgccctgatagacggtttttcgccctttgacgttggagtccacgttctttaatagtggactcttgttccaaactggaacaacactcaaccctatctcggtctattcttttgatttataagggattttgccgatttcggcctattggttaaaaaatgagctgatttaacaaaaatttaacgcgaattttaacaaaatattaacgcttacaatttaggtggcacttttcggggaaatgtgcgcggaacccctatttgtttatttttctaaatacattcaaatatgtatccgctcatgagacaataaccctgataaatgcttcaataatattgaaaaaggaagagtatgagtattcaacatttccgtgtcgcccttattcccttttttgcggcattttgccttcctgtttttgctcacccagaaacgctggtgaaagtaaaagatgctgaagatcagttgggtgcacgagtgggttacatcgaactggatctcaacagcggtaagatccttgagagttttcgccccgaagaacgttttccaatgatgagcacttttaaagttctgctatgtggcgcggtattatcccgtattgacgccgggcaagagcaactcggtcgccgcatacactattctcagaatgacttggttgagtactcaccagtcacagaaaagcatcttacggatggcatgacagtaagagaattatgcagtgctgccataaccatgagtgataacactgcggccaacttacttctgacaacgatcggaggaccgaaggagctaaccgcttttttgcacaacatgggggatcatgtaactcgccttgatcgttgggaaccggagctgaatgaagccataccaaacgacgagcgtgacaccacgatgcctgtagcaatggcaacaacgttgcgcaaactattaactggcgaactacttactctagcttcccggcaacaattaatagactggatggaggcggataaagttgcaggaccacttctgcgctcggcccttccggctggctggtttattgctgataaatctggagccggtgagcgtgggtctcgcggtatcattgcagcactggggccagatggtaagccctcccgtatcgtagttatctacacgacggggagtcaggcaactatggatgaacgaaatagacagatcgctgagataggtgcctcactgattaagcattggtaactgtcagaccaagtttactcatatatactttagattgatttaaaacttcatttttaatttaaaaggatctaggtgaagatcctttttgataatctcatgaccaaaatcccttaacgtgagttttcgttccactgagcgtcagaccccgtagaaaagatcaaaggatcttcttgagatcctttttttctgcgcgtaatctgctgcttgcaaacaaaaaaaccaccgctaccagcggtggtttgtttgccggatcaagagctaccaactctttttccgaaggtaactggcttcagcagagcgcagataccaaatactgtccttctagtgtagccgtagttaggccaccacttcaagaactctgtagcaccgcctacatacctcgctctgctaatcctgttaccagtggctgctgccagtggcgataagtcgtgtcttaccgggttggactcaagacgatagttaccggataaggcgcagcggtcgggctgaacggggggttcgtgcacacagcccagcttggagcgaacgacctacaccgaactgagatacctacagcgtgagctatgagaaagcgccacgcttcccgaagggagaaaggcggacaggtatccggtaagcggcagggtcggaacaggagagcgcacgagggagcttccagggggaaacgcctggtatctttatagtcctgtcgggtttcgccacctctgacttgagcgtcgatttttgtgatgctcgtcaggggggcggagcctatggaaaaacgccagcaacgcggcctttttacggttcctggccttttgctggccttttgctcacatgttctttcctgcgttatcccctgattctgtggataaccgtattaccgcctttgagtgagctgataccgctcgccgcagccgaacgaccgagcgcagcgagtcagtgagcgaggaagcggaagagcgcccaatacgcaaaccgcctctccccgcgcgttggccgattcattaatgcagctggcacgacaggtttcccgactggaaagcgggcagtgagcgcaacgcaattaatgtgagttagctcactcattaggcaccccaggctttacactttatgcttccggctcgtatgttgtgtggaattgtgagcggataacaatttcacacaggaaacagctatgaccatga

SEQ ID NO: 28 - DNA, 5917 bp, Artificial
  Expression vector for Cre recombinase
ggcgcgccggattcgacattgattattgactagttattaatagtaatcaattacggggtcattagttcatagcccatatatggagttccgcgttacataacttacggtaaatggcccgcctggctgaccgcccaacgacccccgcccattgacgtcaataatgacgtatgttcccatagtaacgccaatagggactttccattgacgtcaatgggtggagtatttacggtaaactgcccacttggcagtacatcaagtgtatcatatgccaagtacgccccctattgacgtcaatgacggtaaatggcccgcctggcattatgcccagtacatgaccttatgggactttcctacttggcagtacatctacgtattagtcatcgctattaccatggtcgaggtgagccccacgttctgcttcactctccccatctcccccccctccccacccccaattttgtatttatttattttttaattattttgtgcagcgatgggggcggggggggggggggggcgcgcgccaggcggggcggggcggggcgaggggcggggcggggcgaggcggagaggtgcggcggcagccaatcagagcggcgcgctccgaaagtttccttttatggcgaggcggcggcggcggcggccctataaaaagcgaagcgcgcggcgggcgggagtcgctgcgtcgcgccttcgccccgtgccccgctccgccgccgcctcgcgccgcccgccccggctctgactgaccgcgttactcccacaggtgagcgggcgggacggcccttctcctccgggctgtaattagcgcttggtttaatgacggctcgtttcttttctgtggctgcgtgaaagccttaaagggctccgggagggccctttgtgcgggggggagcggctcggggggtgcgtgcgtgtgtgtgtgcgtggggagcgccgcgtgcggcccgcgctgcccggcggctgtgagcgctgcgggcgcggcgcggggctttgtgcgctccgcgtgtgcgcgaggggagcgcggccgggggcggtgccccgcggtgcgggggggctgcgaggggaacaaaggctgcgtgcggggtgtgtgcgtgggggggtgagcagggggtgtgggcgcggcggtcgggctgtaacccccccctgcacccccctccccgagttgctgagcacggcccggcttcgggtgcggggctccgtgcggggcgtggcgcggggctcgccgtgccgggcggggggtggcggcaggtgggggtgccgggcggggcggggccgcctcgggccggggagggctcgggggaggggcgcggcggccccggagcgccggcggctgtcgaggcgcggcgagccgcagccattgccttttatggtaatcgtgcgagagggcgcagggacttcctttgtcccaaatctggcggagccgaaatctgggaggcgccgccgcaccccctctagcgggcgcgggcgaagcggtgcggcgccggcaggaaggaaatgggcggggagggccttcgtgcgtcgccgcgccgccgtccccttctccatctccagcctcggggctgccgcagggggacggctgccttcgggggggacggggcagggcggggttcggcttctggcgtgtgaccggcggctctagagcctctgctaaccatgttcatgccttcttctttttcctacagatccttaattaataatacgactcactataggggccgccaccatgagcaacctgctgaccgtgcaccagaacctgcctgctctgcctgtggacgccacatctgatgaagtgcggaagaacctgatggacatgttcagagacagacaggccttcagcgagcacacctggaagatgctgctgagcgtgtgtagaagctgggccgcttggtgcaagctgaacaacagaaagtggttccccgccgagcctgaggacgtgcgagattacctgctgtacctgcaagctagaggcctggccgtgaaaaccatccagcagcacctgggccagctgaacatgctgcacagaagaagcggcctgcctagacctagcgacagcaacgctgtgtccctggtcatgagaaggattcggaaagaaaacgtggacgctggcgagagagctaagcaggctctggccttcgagagaaccgacttcgatcaagtgcgcagcctgatggaaaacagcgacagatgccaggatattcggaacctggccttcctgggaatcgcctacaacaccctgctgagaatcgccgagatcgccagaatcagagtgaaggacatcagcagaaccgacggcggcagaatgctgatccacatcggcagaacaaagaccctggtgtccacagctggcgtcgagaaggctctgagtctgggcgtgacaaagctggtggaaagatggatcagcgtgtccggcgtggccgacgatcctaacaactacctgttctgtcgcgtgcgcaagaacggcgtggcagctccttctgctacaagccagctgagcacaagagccctggaaggcatcttcgaggccacacacagactgatctacggcgccaaggatgacagcggccagagataccttgcttggagcggccacagtgctagagtgggcgctgctagagacatggctagagcaggcgtgtcaatccccgagatcatgcaagctggcggctggaccaacgtgaacatcgtgatgaactacatccgcaacctggacagcgagacaggcgctatggttcgactgcttgaagatggcgacggtggatccggtcctgccgctaagagagtgaagctggactgaacgcgtaaatgattgcagatccactagttctagagctcgctgatcagcctcgactgtgccttctagttgccagccatctgttgtttgcccctcccccgtgccttccttgaccctggaaggtgccactcccactgtcctttcctaataaaatgaggaaattgcatcgcattgtctgagtaggtgtcattctattctggggggtggggtggggcaggacagcaagggggaggattgggaagacaatagcaggcatgctggggatgcggtgggctctatggcttctgaggcggaaagaaccagctggggctcgagatccactagttctagcctcgaggctagagcggccgccactggccgtcgttttacaacgtcgtgactgggaaaaccctggcgttacccaacttaatcgccttgcagcacatccccctttcgccagctggcgtaatagcgaagaggcccgcaccgatcgcccttcccaacagttgcgcagcctgaatggcgaatgggacgcgccctgtagcggcgcattaagcgcggcgggtgtggtggttacgcgcagcgtgaccgctacacttgccagcgccctagcgcccgctcctttcgctttcttcccttcctttctcgccacgttcgccggctttccccgtcaagctctaaatcgggggctccctttagggttccgatttagtgctttacggcacctcgaccccaaaaaacttgattagggtgatggttcacgtagtgggccatcgccctgatagacggtttttcgccctttgacgttggagtccacgttctttaatagtggactcttgttccaaactggaacaacactcaaccctatctcggtctattcttttgatttataagggattttgccgatttcggcctattggttaaaaaatgagctgatttaacaaaaatttaacgcgaattttaacaaaatattaacgcttacaatttaggtggcacttttcggggaaatgtgcgcggaacccctatttgtttatttttctaaatacattcaaatatgtatccgctcatgagacaataaccctgataaatgcttcaataatattgaaaaaggaagagtatgagtattcaacatttccgtgtcgcccttattcccttttttgcggcattttgccttcctgtttttgctcacccagaaacgctggtgaaagtaaaagatgctgaagatcagttgggtgcacgagtgggttacatcgaactggatctcaacagcggtaagatccttgagagttttcgccccgaagaacgttttccaatgatgagcacttttaaagttctgctatgtggcgcggtattatcccgtattgacgccgggcaagagcaactcggtcgccgcatacactattctcagaatgacttggttgagtactcaccagtcacagaaaagcatcttacggatggcatgacagtaagagaattatgcagtgctgccataaccatgagtgataacactgcggccaacttacttctgacaacgatcggaggaccgaaggagctaaccgcttttttgcacaacatgggggatcatgtaactcgccttgatcgttgggaaccggagctgaatgaagccataccaaacgacgagcgtgacaccacgatgcctgtagcaatggcaacaacgttgcgcaaactattaactggcgaactacttactctagcttcccggcaacaattaatagactggatggaggcggataaagttgcaggaccacttctgcgctcggcccttccggctggctggtttattgctgataaatctggagccggtgagcgtgggtctcgcggtatcattgcagcactggggccagatggtaagccctcccgtatcgtagttatctacacgacggggagtcaggcaactatggatgaacgaaatagacagatcgctgagataggtgcctcactgattaagcattggtaactgtcagaccaagtttactcatatatactttagattgatttaaaacttcatttttaatttaaaaggatctaggtgaagatcctttttgataatctcatgaccaaaatcccttaacgtgagttttcgttccactgagcgtcagaccccgtagaaaagatcaaaggatcttcttgagatcctttttttctgcgcgtaatctgctgcttgcaaacaaaaaaaccaccgctaccagcggtggtttgtttgccggatcaagagctaccaactctttttccgaaggtaactggcttcagcagagcgcagataccaaatactgtccttctagtgtagccgtagttaggccaccacttcaagaactctgtagcaccgcctacatacctcgctctgctaatcctgttaccagtggctgctgccagtggcgataagtcgtgtcttaccgggttggactcaagacgatagttaccggataaggcgcagcggtcgggctgaacggggggttcgtgcacacagcccagcttggagcgaacgacctacaccgaactgagatacctacagcgtgagctatgagaaagcgccacgcttcccgaagggagaaaggcggacaggtatccggtaagcggcagggtcggaacaggagagcgcacgagggagcttccagggggaaacgcctggtatctttatagtcctgtcgggtttcgccacctctgacttgagcgtcgatttttgtgatgctcgtcaggggggcggagcctatggaaaaacgccagcaacgcggcctttttacggttcctggccttttgctggccttttgctcacatgttctttcctgcgttatcccctgattctgtggataaccgtattaccgcctttgagtgagctgataccgctcgccgcagccgaacgaccgagcgcagcgagtcagtgagcgaggaagcggaagagcgcccaatacgcaaaccgcctctccccgcgcgttggccgattcattaatgcagctggcacgacaggtttcccgactggaaagcgggcagtgagcgcaacgcaattaatgtgagttagctcactcattaggcaccccaggctttacactttatgcttccggctcgtatgttgtgtggaattgtgagcggataacaatttcacacaggaaacagctatgaccatga

SEQ ID NO: 29 - protein, 32 aa, Artificial
  synthetic coiled-coil domain
PEDELAANEEELQQNEQKLAQIKQKLQAIKYG

SEQ ID NO: 30 - protein, 28 aa, Artificial
  synthetic coiled-coil domain
EIQQLEEEIAQLEQKNAALKEKNQALKY

SEQ ID NO: 31 - protein, 28 aa, Artificial
  synthetic coiled-coil domain
KLQAIKYELAQNEEELAQIEEKLAANKE

SEQ ID NO: 32 - protein, 28 aa, Artificial
  synthetic coiled-coil domain
ENAALEEKIAQLKQKNAALKEEIQALEY

SEQ ID NO: 33 - protein, 550 aa, Artificial
  Firefly luciferase-x5
MEDAKNIKKGPAPRYPLEDGTAGEQLHKAMKRYAQVPGTIAFTDAHIEVNITYAEYFEMSVRLAEAMKRYGLNTNHRIVVCSENSLQFFMPVLGALFIGVAVAPANDIYNERELLNSMNISQPTVVFVSKKGLQKILNVQKKLPIIQKIIIMDSKTDYQGFQSMYTFVTSHLPPGFNEYDFKPESFDRDKTIALIMNSSGSTGLPKGVALPHRTACVRFSHARDPIFGNQIKPDTAILSVVPFHHGFGMFTTLGYLICGFRVVLMYRFEEELFLRSLQDYKIQSALLVPTLFSFFAKSTLIDKYDLSNLHEIASGGAPLSKEVGEAVAKRFHLPGIRQGYGLTETTSAILITPEGDDKPGAVGKVVPFFEAKVVDLDTGKTLGVNQRGELCVRGPMIMSGYVNNPEATNALIDKDGWLHSGDIAYWDEDEHFFIVDRLKSLIKYKGYQVAPAELESILLQHPNIRDAGVAGLPDDDAGELPAAVVVLEHGKTMTEKEIVDYVASQVTTAKKLRGGVVFVDEVPKGLTGKLDARKIREILIKAKKGGKIAV

SEQ ID NO: 34 - protein, 170 aa, Artificial
  NanoLuc
VFTLEDFVGDWRQTAGYNLDQVLEQGGVSSLFQNLGVSVTPIQRIVLSGENGLKIDIHVIIPYEGLSGDQMGQIEKIFKVVYPVDDHHFKVILHYGTLVIDGVTPNMIDYFGRPYEGIAVFDGKKITVTGTLWNGNKIIDERLINPDGSLLFRVTINGVTGWRLCERILA

SEQ ID NO: 35 - protein, 131 aa, Artificial
  blasticidin-S-deaminase
AKPLSQEESTLIERATATINSIPISEDYSVASAALSSDGRIFTGVNVYHFTGGPCAELVVLGTAAAAAAGNLTCIVAIGNENRGILSPCGRCRQVLLDLHPGIKAIVKDSDGQPTAVGIRELLPSGYVWEG

SEQ ID NO: 36 - protein, 295 aa, Artificial
  HaloTag
EIGTGFPFDPHYVEVLGERMHYVDVGPRDGTPVLFLHGNPTSSYVWRNIIPHVAPTHRVIAPDLIGMGKSDKPDLGYFFDDHVRFMDAFIEALGLEEVVLVIHDWGSALGFHWAKRNPERVKGIAFMEFIRPIPTWDEWPEFARETFQAFRTTDVGRKLIIDQNVFIEGTLPMGVVRPLTEVEMDHYREPFLNPVDREPLWRFPNELPIAGEPANIVALVEEYMDWLHQSPVPKLLFWGTPGVLIPPAEAARLAKSLPNAKAVDIGPGLNLLQEDNPDLIGSEIARWLSTLEISG

SEQ ID NO: 37 - protein, 556 aa, Artificial
  single chain Avidin
RKRTQPTFGFTVNWKFSESTTVFTGQCFIDRNGKEVLKTMWLLRSSVNDIGDDWKATRVGINIFTRLRTQKEGGSGGSARKCSLTGKWTNDLGSNMTIGAVNSRGEFTGTYITAVTATSNEIKESPLHGTQNTINKSGGSTTVFTGQCFIDRNGKEVLKTMWLLRSSVNDIGDDWKATRVGINIFTRLRTQKEGGSGGSARKCSLTGKWTNDLGSNMTIGAVNSRGEFTGTYITAVTATSNEIKESPLHGTQNTINKRTQPTFGFTVNWKFSEGGSGSGSGSGSGRTQPTFGFTVNWKFSESTTVFTGQCFIDRNGKEVLKTMWLLRSSVNDIGDDWKATRVGINIFTRLRTQKEGGSGGSARKCSLTGKWTNDLGSNMTIGAVNSRGEFTGTYITAVTATSNEIKESPLHGTQNTINKSGGSTTVFTGQCFIDRNGKEVLKTMWLLRSSVNDIGDDWKATRVGINIFTRLRTQKEGGSGGSARKCSLTGKWTNDLGSNMTIGAVNSRGEFTGTYITAVTATSNEIKESPLHGTQNTINKRTQPTFGFTVNWKFSE

SEQ ID NO: 38 - protein, 236 aa, Artificial
  TEV protease X3
GESLFKGPRDYNPISSTICHLTNESDGHTTSLYGIGFGPFIITNKHLFRRNNGTLVVQSLHGVFKVKNTTTLQQHLIDGRDMIIIRMPKDFPPFPQKLKFREPQREERICLVTTNFQTKSMSSMVSDTSCTFPSGDGIFWKHWIQTKDGQCGSPLVSTRDGFIVGIHSASNFTNTNNYFTSVPKNFMELLTNQEAQQWVSGWRLNADSVLWGGHKVFMVKPEEPFQPVKEATQLMN

SEQ ID NO: 39 - protein, 219 aa, Artificial
  modified Ulp1 from Saccharomyces cerevisiae
LVPELNEKDDDQVQKALASRENTQLMNRDNIEITVRDFKTLAPRRWLNSGIISFFMKYIEKSTPNTVAFNSFFYTNLSERGYQGVRRWMKRKKTQIDKLDKIFTPINLNQSHWALGIIDLKKKTIGYVDSLSNGPNAMSFAILTDLQKYVMEESKHTIGEDFDLIHLDCPQQPNGYDCGIYVCMNTLYGSADAPLDFDYKDAIRMRRFIAHLILTDALK

SEQ ID NO: 40 - protein, 235 aa, Artificial
  green fluorescent protein derivative
VSKGEEDNMASLPATHELHIFGSINGVDFDMVGQGTGNPNDGYEELNLKSTKGDLQFSPWILVPHIGYGFHQYLPYPDGMSPFQAAMVDGSGYQVHRTMQFEDGASLTVNYRYTYEGSHIKGEAQVKGTGFPADGPVMTNSLTAADWCRSKKTYPNDKTIISTFKWSYTTGNGKRYRSTARTTYTFAKPMAANYLKNQPMYVFRKTELKHSKTELNFKEWQKAFTDVMGMDELYK

SEQ ID NO: 41 - protein, 438 aa, Artificial
  Flp recombinase with C-terminal NLS
MSQFDILCKTPPKVLVRQFVERFERPSGEKIASCAAELTYLCWMITHNGTAIKRATFMSYNTIISNSLSFDIVNKSLQFKYKTQKATILEASLKKLIPAWEFTIIPYNGQKHQSDITDIVSSLQLQFESSEEADKGNSHSKKMLKALLSEGESIWEITEKILNSFEYTSRFTKTKTLYQFLFLATFINCGRFSDIKNVDPKSFKLVQNKYLGVIIQCLVTETKTSVSRHIYFFSARGRIDPLVYLDEFLRNSEPVLKRVNRTGNSSSNKQEYQLLKDNLVRSYNKALKKNAPYPIFAIKNGPKSHIGRHLMTSFLSMKGLTELTNVVGNWSDKRASAVARTTYTHQITAIPDHYFALVSRYYAYDPISKEMIALKDETNPIEEWQHIEQLKGSAEGSIRYPAWNGIISQEVLDYLSSYINRRIGGSGGSPAAKRVKLD

SEQ ID NO: 42 - protein, 356 aa, Artificial
  Cre recombinase with C-terminal NLS
MSNLLTVHQNLPALPVDATSDEVRKNLMDMFRDRQAFSEHTWKMLLSVCRSWAAWCKLNNRKWFPAEPEDVRDYLLYLQARGLAVKTIQQHLGQLNMLHRRSGLPRPSDSNAVSLVMRRIRKENVDAGERAKQALAFERTDFDQVRSLMENSDRCQDIRNLAFLGIAYNTLLRIAEIARIRVKDISRTDGGRMLIHIGRTKTLVSTAGVEKALSLGVTKLVERWISVSGVADDPNNYLFCRVRKNGVAAPSATSQLSTRALEGIFEATHRLIYGAKDDSGQRYLAWSGHSARVGAARDMARAGVSIPEIMQAGGWTNVNIVMNYIRNLDSETGAMVRLLEDGDGGSGPAAKRVKLD

SEQ ID NO: 43 - protein, 199 aa, Artificial
  Expression product from Puromycin resistance gene
MTEYKPTVRLATRDDVPRAVRTLAAAFADYPATRHTVDPDRHIERVTELQELFLTRVGLDIGKVWVADDGAAVAVWTTPESVEAGAVFAEIGPRMAELSGSRLAAQQQMEGLLAPHRPKEPAWFLATVGVSPDHQGKGLGSAVVLPGVEAAERAGVPAFLETSAPRNLPFYERLGFTVTADVEVPEGPRTWCMTRKPGA

SEQ ID NO: 44 - DNA, 5303 bp, Artificial
  Vector comprising split intein - heterologous polynucleotide construct
ctaaattgtaagcgttaatattttgttaaaattcgcgttaaatttttgttaaatcagctcattttttaaccaataggccgaaatcggcaaaatcccttataaatcaaaagaatagaccgagatagggttgagtgttgttccagtttggaacaagagtccactattaaagaacgtggactccaacgtcaaagggcgaaaaaccgtctatcagggcgatggcccactacgtgaaccatcaccctaatcaagttttttggggtcgaggtgccgtaaagcactaaatcggaaccctaaagggagcccccgatttagagcttgacggggaaagccggcgaacgtggcgagaaaggaagggaagaaagcgaaaggagcgggcgctagggcgctggcaagtgtagcggtcacgctgcgcgtaaccaccacacccgccgcgcttaatgcgccgctacagggcgcgtcccattcgccattcaggctgcgcaactgttgggaagggcgatcggtgcgggcctcttcgctattacgccagctggcgaaagggggatgtgctgcaaggcgattaagttgggtaacgccagggttttcccagtcacgacgttgtaaaacgacggccagtgagcgcgcgtaatacgactcactatagggcgaattggagctgaagactctgtctcgtgggcagcagcgagatcatcaccagaaactacggcaagaccaccatcaaagaggtggtcgagatcttcgacaacgacaagaacatccaggtgctggccttcaacacccacaccgacaacatcgagtgggcccctatcaaggccgctcagctgacaagacctaacgccgagctggtggaactggaaatcgacacactgcacggcgtgaaaaccatcagatgcacccctgatcaccccgtgtacaccaagaacagaggctacgtgcgggccgacgagctgacagatgatgacgaactggtggtggctatcggcggcggaggacctgaggatgaacttgctgccaacgaggaagaactgcaacagaacgaacagaagctggcccagattaagcagaagctccaggccattaagtacggcggatccggcggaggcggatctggtaccggaatggaagatgccaagaacatcaagaagggccctgctcctagataccctctggaagatggaaccgctggcgagcagctgcacaaggccatgaagagatacgctcaggtgcccggcacaatcgccttcacagatgcccacatcgaagtgaacatcacctacgccgagtacttcgagatgagcgtgcggctggccgaagctatgaagcgatacggcctgaacaccaaccacagaatcgtcgtgtgcagcgagaacagcctccagttcttcatgcctgtgctgggcgctctgttcatcggagtggctgtggctcctgccaacgacatctacaacgagcgcgagctgctgaacagcatgaacatcagccagcctaccgtggtgttcgtgtccaagaagggactgcaaaagatcctgaacgtgcagaagaagctgcccatcatccagaaaatcatcatcatggacagcaagaccgactaccagggcttccagagcatgtataccttcgtgaccagccatctgccaccaggcttcaacgagtacgacttcaagcccgagagcttcgacagagacaagacaatcgccctgatcatgaacagcagcggctctaccggactgcctaaaggcgttgccctgcctcacagaacagcttgcgtcagattcagccacgccagagatcccatcttcggcaaccagatcaagcctgacaccgctatcctgagcgtggtgccttttcaccacggcttcggcatgttcaccacactgggctacctgatctgcggcttcagagtggtgctgatgtatcgctttgaggaagaactgttcctgcggagcctccaggactacaagatccagtctgctctgctggtgcctactctgttcagcttctttgccaagagcaccctgatcgataagtacgacctgagcaacctgcacgagatcgcctctggcggagcccctctgtctaaagaagtgggcgaagccgtcgccaagagatttcatctgcccggcatcagacaaggctacggactgaccgagacaaccagcgccatcctgatcacacctgagggcgacgataagcctggcgctgtgggaaaagtggtgccattcttcgaggctaaggtggtggacctggacaccggcaaaacactgggagtgaatcagaggggcgagctgtgtgtcagaggccctatgatcatgagcggctacgtgaacaaccccgaggccaccaacgctctgatcgacaaggatggctggctgcacagcggcgacattgcctactgggacgaagatgagcacttcttcatcgtggacagactgaagtccctgatcaagtacaagggctaccaggtggcccctgccgagctggaatctatcctgctccagcatcctaacatccgcgacgctggtgttgctggcctgcctgacgatgatgctggcgaacttcctgctgccgtggtggtgctggaacacggcaagaccatgaccgagaaagaaatcgtggactacgtggcctctcaagtgaccaccgccaagaaactgagaggcggcgtggtgtttgtggacgaggtgccaaaaggcctgaccggcaagctggacgccagaaagatcagagagatcctcatcaaggccaagaaaggcggcaagatcgctgtcggaggatccggcggagactacaaggacgacgatgacaaagggtcacctggcataacttcgtatagtacacattatacgaagttatctggcgggtcacccgaggatgagatccagcagctggaagaggaaatcgcccagctggaacagaagaatgccgctctgaaagagaagaaccaggctctgaagtacggaggcggaggcatggaagccaagacctacatcggcaagctgaagtccagaaagatcgtgtccaacgaggacacctacgacatccagaccagcacacacaactttttcgccaacgacatcctggtgcacaactcgtcttcgtacccagcttttgttccctttagtgagggttaattgcgcgcttggcgtaatcatggtcatagctgtttcctgtgtgaaattgttatccgctcacaattccacacaacatacgagccggaagcataaagtgtaaagcctggggtgcctaatgagtgagctaactcacattaattgcgttgcgctcactgcccgctttccagtcgggaaacctgtcgtgccagctgcattaatgaatcggccaacgcgcggggagaggcggtttgcgtattgggcgctcttccgcttcctcgctcactgactcgctgcgctcggtcgttcggctgcggcgagcggtatcagctcactcaaaggcggtaatacggttatccacagaatcaggggataacgcaggaaagaacatgtgagcaaaaggccagcaaaaggccaggaaccgtaaaaaggccgcgttgctggcgtttttccataggctccgcccccctgacgagcatcacaaaaatcgacgctcaagtcagaggtggcgaaacccgacaggactataaagataccaggcgtttccccctggaagctccctcgtgcgctctcctgttccgaccctgccgcttaccggatacctgtccgcctttctcccttcgggaagcgtggcgctttctcatagctcacgctgtaggtatctcagttcggtgtaggtcgttcgctccaagctgggctgtgtgcacgaaccccccgttcagcccgaccgctgcgccttatccggtaactatcgtcttgagtccaacccggtaagacacgacttatcgccactggcagcagccactggtaacaggattagcagagcgaggtatgtaggcggtgctacagagttcttgaagtggtggcctaactacggctacactagaaggacagtatttggtatctgcgctctgctgaagccagttaccttcggaaaaagagttggtagctcttgatccggcaaacaaaccaccgctggtagcggtggtttttttgtttgcaagcagcagattacgcgcagaaaaaaaggatctcaagaagatcctttgatcttttctacggggtctgacgctcagtggaacgaaaactcacgttaagggattttggtcatgagattatcaaaaaggatcttcacctagatccttttaaattaaaaatgaagttttaaatcaatctaaagtatatatgagtaaacttggtctgacagttaccaatgcttaatcagtgaggcacctatctcagcgatctgtctatttcgttcatccatagttgcctgactccccgtcgtgtagataactacgatacgggagggcttaccatctggccccagtgctgcaatgataccgcgagacccacgctcaccggctccagatttatcagcaataaaccagccagccggaagggccgagcgcagaagtggtcctgcaactttatccgcctccatccagtctattaattgttgccgggaagctagagtaagtagttcgccagttaatagtttgcgcaacgttgttgccattgctacaggcatcgtggtgtcacgctcgtcgtttggtatggcttcattcagctccggttcccaacgatcaaggcgagttacatgatcccccatgttgtgcaaaaaagcggttagctccttcggtcctccgatcgttgtcagaagtaagttggccgcagtgttatcactcatggttatggcagcactgcataattctcttactgtcatgccatccgtaagatgcttttctgtgactggtgagtactcaaccaagtcattctgagaatagtgtatgcggcgaccgagttgctcttgcccggcgtcaatacgggataataccgcgccacatagcagaactttaaaagtgctcatcattggaaaacgttcttcggggcgaaaactctcaaggatcttaccgctgttgagatccagttcgatgtaacccactcgtgcacccaactgatcttcagcatcttttactttcaccagcgtttctgggtgagcaaaaacaggaaggcaaaatgccgcaaaaaagggaataagggcgacacggaaatgttgaatactcatactcttcctttttcaatattattgaagcatttatcagggttattgtctcatgagcggatacatatttgaatgtatttagaaaaataaacaaataggggttccgcgcacatttccccgaaaagtgccac

SEQ ID NO: 45 - DNA, 7602 bp, Artificial
  Vector comprising split intein - heterologous polynucleotide construct
ctaaattgtaagcgttaatattttgttaaaattcgcgttaaatttttgttaaatcagctcattttttaaccaataggccgaaatcggcaaaatcccttataaatcaaaagaatagaccgagatagggttgagtgttgttccagtttggaacaagagtccactattaaagaacgtggactccaacgtcaaagggcgaaaaaccgtctatcagggcgatggcccactacgtgaaccatcaccctaatcaagttttttggggtcgaggtgccgtaaagcactaaatcggaaccctaaagggagcccccgatttagagcttgacggggaaagccggcgaacgtggcgagaaaggaagggaagaaagcgaaaggagcgggcgctagggcgctggcaagtgtagcggtcacgctgcgcgtaaccaccacacccgccgcgcttaatgcgccgctacagggcgcgtcccattcgccattcaggctgcgcaactgttgggaagggcgatcggtgcgggcctcttcgctattacgccagctggcgaaagggggatgtgctgcaaggcgattaagttgggtaacgccagggttttcccagtcacgacgttgtaaaacgacggccagtgagcgcgcgtaatacgactcactatagggcgaattggagctgaagactctgtctcgtgggcagcagcgagatcatcaccagaaactacggcaagaccaccatcaaagaggtggtcgagatcttcgacaacgacaagaacatccaggtgctggccttcaacacccacaccgacaacatcgagtgggcccctatcaaggccgctcagctgacaagacctaacgccgagctggtggaactggaaatcgacacactgcacggcgtgaaaaccatcagatgcacccctgatcaccccgtgtacaccaagaacagaggctacgtgcgggccgacgagctgacagatgatgacgaactggtggtggctatcggcggcggaggacctgaggatgaacttgctgccaacgaggaagaactgcaacagaacgaacagaagctggcccagattaagcagaagctccaggccattaagtacggcggatccggcggaggcggatctggtaccggaatggaagatgccaagaacatcaagaagggccctgctcctagataccctctggaagatggaaccgctggcgagcagctgcacaaggccatgaagagatacgctcaggtgcccggcacaatcgccttcacagatgcccacatcgaagtgaacatcacctacgccgagtacttcgagatgagcgtgcggctggccgaagctatgaagcgatacggcctgaacaccaaccacagaatcgtcgtgtgcagcgagaacagcctccagttcttcatgcctgtgctgggcgctctgttcatcggagtggctgtggctcctgccaacgacatctacaacgagcgcgagctgctgaacagcatgaacatcagccagcctaccgtggtgttcgtgtccaagaagggactgcaaaagatcctgaacgtgcagaagaagctgcccatcatccagaaaatcatcatcatggacagcaagaccgactaccagggcttccagagcatgtataccttcgtgaccagccatctgccaccaggcttcaacgagtacgacttcaagcccgagagcttcgacagagacaagacaatcgccctgatcatgaacagcagcggctctaccggactgcctaaaggcgttgccctgcctcacagaacagcttgcgtcagattcagccacgccagagatcccatcttcggcaaccagatcaagcctgacaccgctatcctgagcgtggtgccttttcaccacggcttcggcatgttcaccacactgggctacctgatctgcggcttcagagtggtgctgatgtatcgctttgaggaagaactgttcctgcggagcctccaggactacaagatccagtctgctctgctggtgcctactctgttcagcttctttgccaagagcaccctgatcgataagtacgacctgagcaacctgcacgagatcgcctctggcggagcccctctgtctaaagaagtgggcgaagccgtcgccaagagatttcatctgcccggcatcagacaaggctacggactgaccgagacaaccagcgccatcctgatcacacctgagggcgacgataagcctggcgctgtgggaaaagtggtgccattcttcgaggctaaggtggtggacctggacaccggcaaaacactgggagtgaatcagaggggcgagctgtgtgtcagaggccctatgatcatgagcggctacgtgaacaaccccgaggccaccaacgctctgatcgacaaggatggctggctgcacagcggcgacattgcctactgggacgaagatgagcacttcttcatcgtggacagactgaagtccctgatcaagtacaagggctaccaggtggcccctgccgagctggaatctatcctgctccagcatcctaacatccgcgacgctggtgttgctggcctgcctgacgatgatgctggcgaacttcctgctgccgtggtggtgctggaacacggcaagaccatgaccgagaaagaaatcgtggactacgtggcctctcaagtgaccaccgccaagaaactgagaggcggcgtggtgtttgtggacgaggtgccaaaaggcctgaccggcaagctggacgccagaaagatcagagagatcctcatcaaggccaagaaaggcggcaagatcgctgtcggaggatccggcggagactacaaggacgacgatgacaaagggtcacctggcataacttcgtatagtacacattatacgaagttatccggacaggtaagtatcctttttacagcacaacttaatgagacagatagaaactggtcttgtagaaacagagtaggctagcccccagctggttctttccgcctcagaagccatagagcccaccgcatccccagcatgcctgctattctcttcccaatcctcccccttgctgtcctgccccaccccaccccccagaatagaatgacacctactcagacaatgcgatgcaatttcctcattttattaggaaaggacagtgggagtggcaccttccagggtcaaggaaggcacgggggaggggcaaacaacagatggctggcaactagaaggcacagtcgaggctgatcagcgagccgccggcgtctagagaattgatcccctcaggcgccaggctttctggtcatgcaccaggttctagggccctcaggcacttccacgtcggcggtcacggtgaagcccagtctctcgtagaagggcaggtttctgggggcgcttgtttccaggaaggcgggcacgccagccctttcagcagcttccaccccaggcagcaccacagcagatcccagtcccttgccctggtggtcaggtgacacgcccacggtggccagaaaccaggcaggctcttttggtctgtggggggccagcaggccttccatctgctgctgggcagccagtctagagccgctcagctcggccattctaggtccgatctcggcgaacacagcgccggcttccacagactcaggggttgtccacacagccacagcggcgccatcatcggccacccacactttgccgatgtccaggcccactctggtcagaaacagttcctgcagctcggtcactctctcgatgtgccggtcggggtccacggtgtgtcttgtggcagggtaatcggcgaaggcagcggccagtgtccgcacagctcttggcacatcgtccctggtggccagccgcactgtgggcttgtactcggtcatggtggcgcgccttttaggggtagttttcacgacacctgaaatggaagaaaaaaactttgaaccactgtctgaggcttgagaatgaaccaagatccaaactcaaaaagggcaaattccaaggagaattacatcaagtgccaagctggcctaacttcagtctccacccactcagtgtggggaaactccatcgcataaaacccctccccccaacctaaagacgacgtactccaaaagctcgagaactaatcgaggtgcctggacggcgcccggtactccgtggagtcacatgaagcgacggctgaggacggaaaggcccttttcctttgtgtgggtgactcacccgcccgctctcccgagcgccgcgtcctccattttgagctccctgcagcagggccgggaagcggccatctttccgctcacgcaactggtgccgaccgggccagccttgccgcccagggcggggcgatacacggcggcgcgaggccaggcaccagagcaggccggccagcttgagactacccccgtccgattctcggtggccgcgctcgcaggccccgcctcgccgaacatgtgcgctgggacgcacgggccccgtcgccgcccgcggccccaaaaaccgaaataccagtgtgcagatcttggcccgcatttacaagactatcttgccagaaaaaaagcgtcgcagcaggtcatcaaaaattttaaatggctagagacttatcgaaagcagcgagacaggcgcgaaggtgccaccagattcgcacgcggcggccccagcgcccaggccaggcctcaactcaagcacgaggcgaaggggctccttaagcgcaaggcctcgaactctcccacccacttccaacccgaagctcgggatcaagaatcacgtactgcagccaggggcgtggaagtaattcaaggcacgcaagggccataacccgtaaagaggccaggcccgcgggaaccacacacggcacttacctgtgttctggcggcaaacccgttgcgaaaaagaacgttcacggcgactactgcacttatatacggttctcccccaccctcgggaaaaaggcggagccagtacacgacatcactttcccagtttaccccgcgccaccttctctaggcaccggttcaattgccgacccctccccccaacttctcggggactgtgggcgatgtgcgctctgcccactgacgggcaccggagccaattcgaatcgcctgcttttctgcctggtactaacttctctcccctctcctcttttctttttctgcagggcggccgcataacttcgtatagtacacattatacgaagttatctggcgggtcacccgaggatgagatccagcagctggaagaggaaatcgcccagctggaacagaagaatgccgctctgaaagagaagaaccaggctctgaagtacggaggcggaggcatggaagccaagacctacatcggcaagctgaagtccagaaagatcgtgtccaacgaggacacctacgacatccagaccagcacacacaactttttcgccaacgacatcctggtgcacaactcgtcttcgtacccagcttttgttccctttagtgagggttaattgcgcgcttggcgtaatcatggtcatagctgtttcctgtgtgaaattgttatccgctcacaattccacacaacatacgagccggaagcataaagtgtaaagcctggggtgcctaatgagtgagctaactcacattaattgcgttgcgctcactgcccgctttccagtcgggaaacctgtcgtgccagctgcattaatgaatcggccaacgcgcggggagaggcggtttgcgtattgggcgctcttccgcttcctcgctcactgactcgctgcgctcggtcgttcggctgcggcgagcggtatcagctcactcaaaggcggtaatacggttatccacagaatcaggggataacgcaggaaagaacatgtgagcaaaaggccagcaaaaggccaggaaccgtaaaaaggccgcgttgctggcgtttttccataggctccgcccccctgacgagcatcacaaaaatcgacgctcaagtcagaggtggcgaaacccgacaggactataaagataccaggcgtttccccctggaagctccctcgtgcgctctcctgttccgaccctgccgcttaccggatacctgtccgcctttctcccttcgggaagcgtggcgctttctcatagctcacgctgtaggtatctcagttcggtgtaggtcgttcgctccaagctgggctgtgtgcacgaaccccccgttcagcccgaccgctgcgccttatccggtaactatcgtcttgagtccaacccggtaagacacgacttatcgccactggcagcagccactggtaacaggattagcagagcgaggtatgtaggcggtgctacagagttcttgaagtggtggcctaactacggctacactagaaggacagtatttggtatctgcgctctgctgaagccagttaccttcggaaaaagagttggtagctcttgatccggcaaacaaaccaccgctggtagcggtggtttttttgtttgcaagcagcagattacgcgcagaaaaaaaggatctcaagaagatcctttgatcttttctacggggtctgacgctcagtggaacgaaaactcacgttaagggattttggtcatgagattatcaaaaaggatcttcacctagatccttttaaattaaaaatgaagttttaaatcaatctaaagtatatatgagtaaacttggtctgacagttaccaatgcttaatcagtgaggcacctatctcagcgatctgtctatttcgttcatccatagttgcctgactccccgtcgtgtagataactacgatacgggagggcttaccatctggccccagtgctgcaatgataccgcgagacccacgctcaccggctccagatttatcagcaataaaccagccagccggaagggccgagcgcagaagtggtcctgcaactttatccgcctccatccagtctattaattgttgccgggaagctagagtaagtagttcgccagttaatagtttgcgcaacgttgttgccattgctacaggcatcgtggtgtcacgctcgtcgtttggtatggcttcattcagctccggttcccaacgatcaaggcgagttacatgatcccccatgttgtgcaaaaaagcggttagctccttcggtcctccgatcgttgtcagaagtaagttggccgcagtgttatcactcatggttatggcagcactgcataattctcttactgtcatgccatccgtaagatgcttttctgtgactggtgagtactcaaccaagtcattctgagaatagtgtatgcggcgaccgagttgctcttgcccggcgtcaatacgggataataccgcgccacatagcagaactttaaaagtgctcatcattggaaaacgttcttcggggcgaaaactctcaaggatcttaccgctgttgagatccagttcgatgtaacccactcgtgcacccaactgatcttcagcatcttttactttcaccagcgtttctgggtgagcaaaaacaggaaggcaaaatgccgcaaaaaagggaataagggcgacacggaaatgttgaatactcatactcttcctttttcaatattattgaagcatttatcagggttattgtctcatgagcggatacatatttgaatgtatttagaaaaataaacaaataggggttccgcgcacatttccccgaaaagtgccac

SEQ ID NO: 46 - DNA, 4121 bp, Artificial
  Vector comprising split intein - heterologous polynucleotide construct
ctaaattgtaagcgttaatattttgttaaaattcgcgttaaatttttgttaaatcagctcattttttaaccaataggccgaaatcggcaaaatcccttataaatcaaaagaatagaccgagatagggttgagtgttgttccagtttggaacaagagtccactattaaagaacgtggactccaacgtcaaagggcgaaaaaccgtctatcagggcgatggcccactacgtgaaccatcaccctaatcaagttttttggggtcgaggtgccgtaaagcactaaatcggaaccctaaagggagcccccgatttagagcttgacggggaaagccggcgaacgtggcgagaaaggaagggaagaaagcgaaaggagcgggcgctagggcgctggcaagtgtagcggtcacgctgcgcgtaaccaccacacccgccgcgcttaatgcgccgctacagggcgcgtcccattcgccattcaggctgcgcaactgttgggaagggcgatcggtgcgggcctcttcgctattacgccagctggcgaaagggggatgtgctgcaaggcgattaagttgggtaacgccagggttttcccagtcacgacgttgtaaaacgacggccagtgagcgcgcgtaatacgactcactatagggcgaattggagctgaagactctgcctggaccttaagacccaggtgcagaccccccagggcatgaaggaaatcagcaacatccaagtgggcgacctggtgctgagcaacaccggctacaacgaggtgctgaacgtgttccccaagagcaagaagaagtcctacaagatcaccctggaagatggcaaagagatcatctgctccgaggaacacctgttcccaacccagaccggcgagatgaacatctctggcggcctgaaagagggcatgtgcctgtacgtgaaagaaggcggcggaggacctgaggataagctccaggccattaagtacgagctggcccagaacgaggaagaactggctcagatcgaagagaagctggccgccaacaaagaaggcggatccggcggaggcggatctggaaccggttttgctaatgagctgggccccagactgatgggcaaaggcagcggaggaggcggaagcggagtctttacactggaagatttcgtcggcgactggcggcagacagctggctacaatctggaccaggtgctggaacaaggcggcgtgtcctctctgtttcagaacctgggagtgtctgtgacccctatccagagaatcgtgctgagcggcgagaacggcctgaagatcgacatccacgtgatcatcccttacgagggcctgtccggcgatcagatgggacagatcgagaagatctttaaggtggtgtaccccgtggacgaccaccacttcaaagtgatcctgcactacggcaccctggtcatcgatggcgtgaccccaaacatgatcgactacttcggcagaccctacgagggaatcgccgtgttcgacggcaagaaaatcaccgtgaccggcacactgtggaacggcaacaagatcatcgacgagagactgatcaaccccgacggcagcctgctgttcagagtgacaatcaacggcgtgacaggctggcggctgtgcgaaagaatccttgctggttccggaggaagttcctatacttcaaatagaataggaacttccggcgggtcacccgaggatgagaatgctgctctggaagagaagatcgcccagctgaagcagaagaacgccgctctgaaagaagagatccaggctctggaatacggaggcggaggcatgatgctgaagaagatcctgaagatcgaagaactggacgagcgcgagctgatcgacatcgaggtgtccggcaaccacctgttctacgccaacgatatcctgacccacaactcgtcttcgtacccagcttttgttccctttagtgagggttaattgcgcgcttggcgtaatcatggtcatagctgtttcctgtgtgaaattgttatccgctcacaattccacacaacatacgagccggaagcataaagtgtaaagcctggggtgcctaatgagtgagctaactcacattaattgcgttgcgctcactgcccgctttccagtcgggaaacctgtcgtgccagctgcattaatgaatcggccaacgcgcggggagaggcggtttgcgtattgggcgctcttccgcttcctcgctcactgactcgctgcgctcggtcgttcggctgcggcgagcggtatcagctcactcaaaggcggtaatacggttatccacagaatcaggggataacgcaggaaagaacatgtgagcaaaaggccagcaaaaggccaggaaccgtaaaaaggccgcgttgctggcgtttttccataggctccgcccccctgacgagcatcacaaaaatcgacgctcaagtcagaggtggcgaaacccgacaggactataaagataccaggcgtttccccctggaagctccctcgtgcgctctcctgttccgaccctgccgcttaccggatacctgtccgcctttctcccttcgggaagcgtggcgctttctcatagctcacgctgtaggtatctcagttcggtgtaggtcgttcgctccaagctgggctgtgtgcacgaaccccccgttcagcccgaccgctgcgccttatccggtaactatcgtcttgagtccaacccggtaagacacgacttatcgccactggcagcagccactggtaacaggattagcagagcgaggtatgtaggcggtgctacagagttcttgaagtggtggcctaactacggctacactagaaggacagtatttggtatctgcgctctgctgaagccagttaccttcggaaaaagagttggtagctcttgatccggcaaacaaaccaccgctggtagcggtggtttttttgtttgcaagcagcagattacgcgcagaaaaaaaggatctcaagaagatcctttgatcttttctacggggtctgacgctcagtggaacgaaaactcacgttaagggattttggtcatgagattatcaaaaaggatcttcacctagatccttttaaattaaaaatgaagttttaaatcaatctaaagtatatatgagtaaacttggtctgacagttaccaatgcttaatcagtgaggcacctatctcagcgatctgtctatttcgttcatccatagttgcctgactccccgtcgtgtagataactacgatacgggagggcttaccatctggccccagtgctgcaatgataccgcgagacccacgctcaccggctccagatttatcagcaataaaccagccagccggaagggccgagcgcagaagtggtcctgcaactttatccgcctccatccagtctattaattgttgccgggaagctagagtaagtagttcgccagttaatagtttgcgcaacgttgttgccattgctacaggcatcgtggtgtcacgctcgtcgtttggtatggcttcattcagctccggttcccaacgatcaaggcgagttacatgatcccccatgttgtgcaaaaaagcggttagctccttcggtcctccgatcgttgtcagaagtaagttggccgcagtgttatcactcatggttatggcagcactgcataattctcttactgtcatgccatccgtaagatgcttttctgtgactggtgagtactcaaccaagtcattctgagaatagtgtatgcggcgaccgagttgctcttgcccggcgtcaatacgggataataccgcgccacatagcagaactttaaaagtgctcatcattggaaaacgttcttcggggcgaaaactctcaaggatcttaccgctgttgagatccagttcgatgtaacccactcgtgcacccaactgatcttcagcatcttttactttcaccagcgtttctgggtgagcaaaaacaggaaggcaaaatgccgcaaaaaagggaataagggcgacacggaaatgttgaatactcatactcttcctttttcaatattattgaagcatttatcagggttattgtctcatgagcggatacatatttgaatgtatttagaaaaataaacaaataggggttccgcgcacatttccccgaaaagtgccac

SEQ ID NO: 47 - DNA, 6276 bp, Artificial
  Vector comprising split intein - heterologous polynucleotide construct
ctaaattgtaagcgttaatattttgttaaaattcgcgttaaatttttgttaaatcagctcattttttaaccaataggccgaaatcggcaaaatcccttataaatcaaaagaatagaccgagatagggttgagtgttgttccagtttggaacaagagtccactattaaagaacgtggactccaacgtcaaagggcgaaaaaccgtctatcagggcgatggcccactacgtgaaccatcaccctaatcaagttttttggggtcgaggtgccgtaaagcactaaatcggaaccctaaagggagcccccgatttagagcttgacggggaaagccggcgaacgtggcgagaaaggaagggaagaaagcgaaaggagcgggcgctagggcgctggcaagtgtagcggtcacgctgcgcgtaaccaccacacccgccgcgcttaatgcgccgctacagggcgcgtcccattcgccattcaggctgcgcaactgttgggaagggcgatcggtgcgggcctcttcgctattacgccagctggcgaaagggggatgtgctgcaaggcgattaagttgggtaacgccagggttttcccagtcacgacgttgtaaaacgacggccagtgagcgcgcgtaatacgactcactatagggcgaattggagctgaagactctgcctggaccttaagacccaggtgcagaccccccagggcatgaaggaaatcagcaacatccaagtgggcgacctggtgctgagcaacaccggctacaacgaggtgctgaacgtgttccccaagagcaagaagaagtcctacaagatcaccctggaagatggcaaagagatcatctgctccgaggaacacctgttcccaacccagaccggcgagatgaacatctctggcggcctgaaagagggcatgtgcctgtacgtgaaagaaggcggcggaggacctgaggataagctccaggccattaagtacgagctggcccagaacgaggaagaactggctcagatcgaagagaagctggccgccaacaaagaaggcggatccggcggaggcggatctggaaccggttttgctaatgagctgggccccagactgatgggcaaaggcagcggaggaggcggaagcggagtctttacactggaagatttcgtcggcgactggcggcagacagctggctacaatctggaccaggtgctggaacaaggcggcgtgtcctctctgtttcagaacctgggagtgtctgtgacccctatccagagaatcgtgctgagcggcgagaacggcctgaagatcgacatccacgtgatcatcccttacgagggcctgtccggcgatcagatgggacagatcgagaagatctttaaggtggtgtaccccgtggacgaccaccacttcaaagtgatcctgcactacggcaccctggtcatcgatggcgtgaccccaaacatgatcgactacttcggcagaccctacgagggaatcgccgtgttcgacggcaagaaaatcaccgtgaccggcacactgtggaacggcaacaagatcatcgacgagagactgatcaaccccgacggcagcctgctgttcagagtgacaatcaacggcgtgacaggctggcggctgtgcgaaagaatccttgctggttccggaggaagttcctatacttcaaatagaataggaacttcgaattggctccggtgcccgtcagtgggcagagcgcacatcgcccacagtccccgagaagttggggggaggggtcggcaattgaaccggtgcctagagaaggtggcgcggggtaaactgggaaagtgatgtcgtgtactggctccgcctttttcccgagggtgggggagaaccgtatataagtgcagtagtcgccgtgaacgttctttttcgcaacgggtttgccgccagaacacaggtaagtgccgtgtgtggttcccgcgggcctggcctctttacgggttatggcccttgcgtgccttgaattacttccacgcccctggctgcagtacgtgattcttgatcccgagcttcgggttggaagtgggtgggagagttcgaggccttgcgcttaaggagccccttcgcctcgtgcttgagttgaggcctggcctgggcgctggggccgccgcgtgcgaatctggtggcaccttcgcgcctgtctcgctgctttcgataagtctctagccatttaaaatttttgatgacctgctgcgacgctttttttctggcaagatagtcttgtaaatgcgggccaagatctgcacactggtatttcggtttttggggccgcgggcggcgacggggcccgtgcgtcccagcgcacatgttcggcgaggcggggcctgcgagcgcggccaccgagaatcggacgggggtagtctcaagctggccggcctgctctggtgcctggcctcgcgccgccgtgtatcgccccgccctgggcggcaaggctggcccggtcggcaccagttgcgtgagcggaaagatggccgcttcccggccctgctgcagggagctcaaaatggaggacgcggcgctcgggagagcgggcgggtgagtcacccacacaaaggaaaagggcctttccgtcctcagccgtcgcttcatgtgactccacggagtaccgggcgccgtccaggcacctcgattagttctcgagcttttggagtacgtcgtctttaggttggggggaggggttttatgcgatggagtttccccacactgagtgggtggagactgaagttaggccagcttggcacttgatgtaattctccttggaatttgccctttttgagtttggatcttggttcattctcaagcctcagacagtggttcaaagtttttttcttccatttcaggtgtcgtgaaaactacccctaaaaggcgcgccaccatgaccgagtacaagcccacagtgcggctggccaccagggacgatgtgccaagagctgtgcggacactggccgctgccttcgccgattaccctgccacaagacacaccgtggaccccgaccggcacatcgagagagtgaccgagctgcaggaactgtttctgaccagagtgggcctggacatcggcaaagtgtgggtggccgatgatggcgccgctgtggctgtgtggacaacccctgagtctgtggaagccggcgctgtgttcgccgagatcggacctagaatggccgagctgagcggctctagactggctgcccagcagcagatggaaggcctgctggccccccacagaccaaaagagcctgcctggtttctggccaccgtgggcgtgtcacctgaccaccagggcaagggactgggatctgctgtggtgctgcctggggtggaagctgctgaaagggctggcgtgcccgccttcctggaaacaagcgcccccagaaacctgcccttctacgagagactgggcttcaccgtgaccgccgacgtggaagtgcctgagggccctagaacctggtgcatgaccagaaagcctggcgcctgaggggatcaattctctagacgccggcggctcgctgatcagcctcgactgtgccttctagttgccagccatctgttgtttgcccctcccccgtgccttccttgaccctggaaggtgccactcccactgtcctttcctaataaaatgaggaaattgcatcgcattgtctgagtaggtgtcattctattctggggggtggggtggggcaggacagcaagggggaggattgggaagagaatagcaggcatgctggggatgcggtgggctctatggcttctgaggcggaaagaaccagctgggggcggccgcggaagttcctatacttcaaatagaataggaacttccggcgggtcacccgaggatgagaatgctgctctggaagagaagatcgcccagctgaagcagaagaacgccgctctgaaagaagagatccaggctctggaatacggaggcggaggcatgatgctgaagaagatcctgaagatcgaagaactggacgagcgcgagctgatcgacatcgaggtgtccggcaaccacctgttctacgccaacgatatcctgacccacaactcgtcttcgtacccagcttttgttccctttagtgagggttaattgcgcgcttggcgtaatcatggtcatagctgtttcctgtgtgaaattgttatccgctcacaattccacacaacatacgagccggaagcataaagtgtaaagcctggggtgcctaatgagtgagctaactcacattaattgcgttgcgctcactgcccgctttccagtcgggaaacctgtcgtgccagctgcattaatgaatcggccaacgcgcggggagaggcggtttgcgtattgggcgctcttccgcttcctcgctcactgactcgctgcgctcggtcgttcggctgcggcgagcggtatcagctcactcaaaggcggtaatacggttatccacagaatcaggggataacgcaggaaagaacatgtgagcaaaaggccagcaaaaggccaggaaccgtaaaaaggccgcgttgctggcgtttttccataggctccgcccccctgacgagcatcacaaaaatcgacgctcaagtcagaggtggcgaaacccgacaggactataaagataccaggcgtttccccctggaagctccctcgtgcgctctcctgttccgaccctgccgcttaccggatacctgtccgcctttctcccttcgggaagcgtggcgctttctcatagctcacgctgtaggtatctcagttcggtgtaggtcgttcgctccaagctgggctgtgtgcacgaaccccccgttcagcccgaccgctgcgccttatccggtaactatcgtcttgagtccaacccggtaagacacgacttatcgccactggcagcagccactggtaacaggattagcagagcgaggtatgtaggcggtgctacagagttcttgaagtggtggcctaactacggctacactagaaggacagtatttggtatctgcgctctgctgaagccagttaccttcggaaaaagagttggtagctcttgatccggcaaacaaaccaccgctggtagcggtggtttttttgtttgcaagcagcagattacgcgcagaaaaaaaggatctcaagaagatcctttgatcttttctacggggtctgacgctcagtggaacgaaaactcacgttaagggattttggtcatgagattatcaaaaaggatcttcacctagatccttttaaattaaaaatgaagttttaaatcaatctaaagtatatatgagtaaacttggtctgacagttaccaatgcttaatcagtgaggcacctatctcagcgatctgtctatttcgttcatccatagttgcctgactccccgtcgtgtagataactacgatacgggagggcttaccatctggccccagtgctgcaatgataccgcgagacccacgctcaccggctccagatttatcagcaataaaccagccagccggaagggccgagcgcagaagtggtcctgcaactttatccgcctccatccagtctattaattgttgccgggaagctagagtaagtagttcgccagttaatagtttgcgcaacgttgttgccattgctacaggcatcgtggtgtcacgctcgtcgtttggtatggcttcattcagctccggttcccaacgatcaaggcgagttacatgatcccccatgttgtgcaaaaaagcggttagctccttcggtcctccgatcgttgtcagaagtaagttggccgcagtgttatcactcatggttatggcagcactgcataattctcttactgtcatgccatccgtaagatgcttttctgtgactggtgagtactcaaccaagtcattctgagaatagtgtatgcggcgaccgagttgctcttgcccggcgtcaatacgggataataccgcgccacatagcagaactttaaaagtgctcatcattggaaaacgttcttcggggcgaaaactctcaaggatcttaccgctgttgagatccagttcgatgtaacccactcgtgcacccaactgatcttcagcatcttttactttcaccagcgtttctgggtgagcaaaaacaggaaggcaaaatgccgcaaaaaagggaataagggcgacacggaaatgttgaatactcatactcttcctttttcaatattattgaagcatttatcagggttattgtctcatgagcggatacatatttgaatgtatttagaaaaataaacaaataggggttccgcgcacatttccccgaaaagtgccac

SEQ ID NO: 48 - DNA, 6417 bp, Artificial
  Vector comprising split intein - heterologous polynucleotide construct
ctaaattgtaagcgttaatattttgttaaaattcgcgttaaatttttgttaaatcagctcattttttaaccaataggccgaaatcggcaaaatcccttataaatcaaaagaatagaccgagatagggttgagtgttgttccagtttggaacaagagtccactattaaagaacgtggactccaacgtcaaagggcgaaaaaccgtctatcagggcgatggcccactacgtgaaccatcaccctaatcaagttttttggggtcgaggtgccgtaaagcactaaatcggaaccctaaagggagcccccgatttagagcttgacggggaaagccggcgaacgtggcgagaaaggaagggaagaaagcgaaaggagcgggcgctagggcgctggcaagtgtagcggtcacgctgcgcgtaaccaccacacccgccgcgcttaatgcgccgctacagggcgcgtcccattcgccattcaggctgcgcaactgttgggaagggcgatcggtgcgggcctcttcgctattacgccagctggcgaaagggggatgtgctgcaaggcgattaagttgggtaacgccagggttttcccagtcacgacgttgtaaaacgacggccagtgagcgcgcgtaatacgactcactatagggcgaattggagctgaagactctgcctggaccttaagacccaggtgcagaccccccagggcatgaaggaaatcagcaacatccaagtgggcgacctggtgctgagcaacaccggctacaacgaggtgctgaacgtgttccccaagagcaagaagaagtcctacaagatcaccctggaagatggcaaagagatcatctgctccgaggaacacctgttcccaacccagaccggcgagatgaacatctctggcggcctgaaagagggcatgtgcctgtacgtgaaagaaggcggcggaggacctgaggataagctccaggccattaagtacgagctggcccagaacgaggaagaactggctcagatcgaagagaagctggccgccaacaaagaaggcggatccggcggaggcggatctggaaccggttttgctaatgagctgggccccagactgatgggcaaaggcagcggaggaggcggaagcggagtctttacactggaagatttcgtcggcgactggcggcagacagctggctacaatctggaccaggtgctggaacaaggcggcgtgtcctctctgtttcagaacctgggagtgtctgtgacccctatccagagaatcgtgctgagcggcgagaacggcctgaagatcgacatccacgtgatcatcccttacgagggcctgtccggcgatcagatgggacagatcgagaagatctttaaggtggtgtaccccgtggacgaccaccacttcaaagtgatcctgcactacggcaccctggtcatcgatggcgtgaccccaaacatgatcgactacttcggcagaccctacgagggaatcgccgtgttcgacggcaagaaaatcaccgtgaccggcacactgtggaacggcaacaagatcatcgacgagagactgatcaaccccgacggcagcctgctgttcagagtgacaatcaacggcgtgacaggctggcggctgtgcgaaagaatccttgctggttccggaggaagttcctatacttcaaatagaataggaacttcgcaggtaagtatcctttttacagcacaacttaatgagacagatagaaactggtcttgtagaaacagagtaggctagcccccagctggttctttccgcctcagaagccatagagcccaccgcatccccagcatgcctgctattctcttcccaatcctcccccttgctgtcctgccccaccccaccccccagaatagaatgacacctactcagacaatgcgatgcaatttcctcattttattaggaaaggacagtgggagtggcaccttccagggtcaaggaaggcacgggggaggggcaaacaacagatggctggcaactagaaggcacagtcgaggctgatcagcgagccgccggcgtctagagaattgatcccctcaggcgccaggctttctggtcatgcaccaggttctagggccctcaggcacttccacgtcggcggtcacggtgaagcccagtctctcgtagaagggcaggtttctgggggcgcttgtttccaggaaggcgggcacgccagccctttcagcagcttccaccccaggcagcaccacagcagatcccagtcccttgccctggtggtcaggtgacacgcccacggtggccagaaaccaggcaggctcttttggtctgtggggggccagcaggccttccatctgctgctgggcagccagtctagagccgctcagctcggccattctaggtccgatctcggcgaacacagcgccggcttccacagactcaggggttgtccacacagccacagcggcgccatcatcggccacccacactttgccgatgtccaggcccactctggtcagaaacagttcctgcagctcggtcactctctcgatgtgccggtcggggtccacggtgtgtcttgtggcagggtaatcggcgaaggcagcggccagtgtccgcacagctcttggcacatcgtccctggtggccagccgcactgtgggcttgtactcggtcatggtggcgcgccttttaggggtagttttcacgacacctgaaatggaagaaaaaaactttgaaccactgtctgaggcttgagaatgaaccaagatccaaactcaaaaagggcaaattccaaggagaattacatcaagtgccaagctggcctaacttcagtctccacccactcagtgtggggaaactccatcgcataaaacccctccccccaacctaaagacgacgtactccaaaagctcgagaactaatcgaggtgcctggacggcgcccggtactccgtggagtcacatgaagcgacggctgaggacggaaaggcccttttcctttgtgtgggtgactcacccgcccgctctcccgagcgccgcgtcctccattttgagctccctgcagcagggccgggaagcggccatctttccgctcacgcaactggtgccgaccgggccagccttgccgcccagggcggggcgatacacggcggcgcgaggccaggcaccagagcaggccggccagcttgagactacccccgtccgattctcggtggccgcgctcgcaggccccgcctcgccgaacatgtgcgctgggacgcacgggccccgtcgccgcccgcggccccaaaaaccgaaataccagtgtgcagatcttggcccgcatttacaagactatcttgccagaaaaaaagcgtcgcagcaggtcatcaaaaattttaaatggctagagacttatcgaaagcagcgagacaggcgcgaaggtgccaccagattcgcacgcggcggccccagcgcccaggccaggcctcaactcaagcacgaggcgaaggggctccttaagcgcaaggcctcgaactctcccacccacttccaacccgaagctcgggatcaagaatcacgtactgcagccaggggcgtggaagtaattcaaggcacgcaagggccataacccgtaaagaggccaggcccgcgggaaccacacacggcacttacctgtgttctggcggcaaacccgttgcgaaaaagaacgttcacggcgactactgcacttatatacggttctcccccaccctcgggaaaaaggcggagccagtacacgacatcactttcccagtttaccccgcgccaccttctctaggcaccggttcaattgccgacccctccccccaacttctcggggactgtgggcgatgtgcgctctgcccactgacgggcaccggagccaattcgaatcgcctgcttttctgcctggtactaacttctctcccctctcctcttttctttttctgcagggcggccgcggaagttcctatacttcaaatagaataggaacttccggcgggtcacccgaggatgagaatgctgctctggaagagaagatcgcccagctgaagcagaagaacgccgctctgaaagaagagatccaggctctggaatacggaggcggaggcatgatgctgaagaagatcctgaagatcgaagaactggacgagcgcgagctgatcgacatcgaggtgtccggcaaccacctgttctacgccaacgatatcctgacccacaactcgtcttcgtacccagcttttgttccctttagtgagggttaattgcgcgcttggcgtaatcatggtcatagctgtttcctgtgtgaaattgttatccgctcacaattccacacaacatacgagccggaagcataaagtgtaaagcctggggtgcctaatgagtgagctaactcacattaattgcgttgcgctcactgcccgctttccagtcgggaaacctgtcgtgccagctgcattaatgaatcggccaacgcgcggggagaggcggtttgcgtattgggcgctcttccgcttcctcgctcactgactcgctgcgctcggtcgttcggctgcggcgagcggtatcagctcactcaaaggcggtaatacggttatccacagaatcaggggataacgcaggaaagaacatgtgagcaaaaggccagcaaaaggccaggaaccgtaaaaaggccgcgttgctggcgtttttccataggctccgcccccctgacgagcatcacaaaaatcgacgctcaagtcagaggtggcgaaacccgacaggactataaagataccaggcgtttccccctggaagctccctcgtgcgctctcctgttccgaccctgccgcttaccggatacctgtccgcctttctcccttcgggaagcgtggcgctttctcatagctcacgctgtaggtatctcagttcggtgtaggtcgttcgctccaagctgggctgtgtgcacgaaccccccgttcagcccgaccgctgcgccttatccggtaactatcgtcttgagtccaacccggtaagacacgacttatcgccactggcagcagccactggtaacaggattagcagagcgaggtatgtaggcggtgctacagagttcttgaagtggtggcctaactacggctacactagaaggacagtatttggtatctgcgctctgctgaagccagttaccttcggaaaaagagttggtagctcttgatccggcaaacaaaccaccgctggtagcggtggtttttttgtttgcaagcagcagattacgcgcagaaaaaaaggatctcaagaagatcctttgatcttttctacggggtctgacgctcagtggaacgaaaactcacgttaagggattttggtcatgagattatcaaaaaggatcttcacctagatccttttaaattaaaaatgaagttttaaatcaatctaaagtatatatgagtaaacttggtctgacagttaccaatgcttaatcagtgaggcacctatctcagcgatctgtctatttcgttcatccatagttgcctgactccccgtcgtgtagataactacgatacgggagggcttaccatctggccccagtgctgcaatgataccgcgagacccacgctcaccggctccagatttatcagcaataaaccagccagccggaagggccgagcgcagaagtggtcctgcaactttatccgcctccatccagtctattaattgttgccgggaagctagagtaagtagttcgccagttaatagtttgcgcaacgttgttgccattgctacaggcatcgtggtgtcacgctcgtcgtttggtatggcttcattcagctccggttcccaacgatcaaggcgagttacatgatcccccatgttgtgcaaaaaagcggttagctccttcggtcctccgatcgttgtcagaagtaagttggccgcagtgttatcactcatggttatggcagcactgcataattctcttactgtcatgccatccgtaagatgcttttctgtgactggtgagtactcaaccaagtcattctgagaatagtgtatgcggcgaccgagttgctcttgcccggcgtcaatacgggataataccgcgccacatagcagaactttaaaagtgctcatcattggaaaacgttcttcggggcgaaaactctcaaggatcttaccgctgttgagatccagttcgatgtaacccactcgtgcacccaactgatcttcagcatcttttactttcaccagcgtttctgggtgagcaaaaacaggaaggcaaaatgccgcaaaaaagggaataagggcgacacggaaatgttgaatactcatactcttcctttttcaatattattgaagcatttatcagggttattgtctcatgagcggatacatatttgaatgtatttagaaaaataaacaaataggggttccgcgcacatttccccgaaaagtgccac

SEQ ID NO: 49 - DNA, 6321 bp, Artificial
  Vector comprising split intein - heterologous polynucleotide construct
ctaaattgtaagcgttaatattttgttaaaattcgcgttaaatttttgttaaatcagctcattttttaaccaataggccgaaatcggcaaaatcccttataaatcaaaagaatagaccgagatagggttgagtgttgttccagtttggaacaagagtccactattaaagaacgtggactccaacgtcaaagggcgaaaaaccgtctatcagggcgatggcccactacgtgaaccatcaccctaatcaagttttttggggtcgaggtgccgtaaagcactaaatcggaaccctaaagggagcccccgatttagagcttgacggggaaagccggcgaacgtggcgagaaaggaagggaagaaagcgaaaggagcgggcgctagggcgctggcaagtgtagcggtcacgctgcgcgtaaccaccacacccgccgcgcttaatgcgccgctacagggcgcgtcccattcgccattcaggctgcgcaactgttgggaagggcgatcggtgcgggcctcttcgctattacgccagctggcgaaagggggatgtgctgcaaggcgattaagttgggtaacgccagggttttcccagtcacgacgttgtaaaacgacggccagtgagcgcgcgtaatacgactcactatagggcgaattggagctgaagactctgcctggaccttaagacccaggtgcagaccccccagggcatgaaggaaatcagcaacatccaagtgggcgacctggtgctgagcaacaccggctacaacgaggtgctgaacgtgttccccaagagcaagaagaagtcctacaagatcaccctggaagatggcaaagagatcatctgctccgaggaacacctgttcccaacccagaccggcgagatgaacatctctggcggcctgaaagagggcatgtgcctgtacgtgaaagaaggcggcggaggacctgaggataagctccaggccattaagtacgagctggcccagaacgaggaagaactggctcagatcgaagagaagctggccgccaacaaagaaggcggatccggcggaggtggaagcggaggcggaggatctggtggtggtggatctgctaagcccctgagccaagaggaaagcaccctgatcgagagagccaccgccaccatcaacagcatccctatcagcgaggactacagcgtggcctctgctgctctgtctagcgacggcagaatcttcacaggcgtgaacgtgtaccactttacaggcggcccttgtgccgaactggtggtgcttggaacagccgctgccgctgctgctggaaacctgacatgtatcgtggctatcggcaacgagaacagaggcatcctgtctccatgcggcagatgcagacaggtcctgctcgatctgcaccctggcatcaaggccatcgtgaaggactctgacggccagcctacagccgtgggaatcagagaactgctgcctagcggctacgtgtgggaaggtggtggcggaggaagcggcacaggatttgctaatgagctgggccctagactgatgggcaaaggctccggaggaagttcctatacttcaaatagaataggaacttcgcaggtaagtatcctttttacagcacaacttaatgagacagatagaaactggtcttgtagaaacagagtaggctagcccccagctggttctttccgcctcagaagccatagagcccaccgcatccccagcatgcctgctattctcttcccaatcctcccccttgctgtcctgccccaccccaccccccagaatagaatgacacctactcagacaatgcgatgcaatttcctcattttattaggaaaggacagtgggagtggcaccttccagggtcaaggaaggcacgggggaggggcaaacaacagatggctggcaactagaaggcacagtcgaggctgatcagcgagccgccggcgtctagagaattgatcccctcaggcgccaggctttctggtcatgcaccaggttctagggccctcaggcacttccacgtcggcggtcacggtgaagcccagtctctcgtagaagggcaggtttctgggggcgcttgtttccaggaaggcgggcacgccagccctttcagcagcttccaccccaggcagcaccacagcagatcccagtcccttgccctggtggtcaggtgacacgcccacggtggccagaaaccaggcaggctcttttggtctgtggggggccagcaggccttccatctgctgctgggcagccagtctagagccgctcagctcggccattctaggtccgatctcggcgaacacagcgccggcttccacagactcaggggttgtccacacagccacagcggcgccatcatcggccacccacactttgccgatgtccaggcccactctggtcagaaacagttcctgcagctcggtcactctctcgatgtgccggtcggggtccacggtgtgtcttgtggcagggtaatcggcgaaggcagcggccagtgtccgcacagctcttggcacatcgtccctggtggccagccgcactgtgggcttgtactcggtcatggtggcgcgccttttaggggtagttttcacgacacctgaaatggaagaaaaaaactttgaaccactgtctgaggcttgagaatgaaccaagatccaaactcaaaaagggcaaattccaaggagaattacatcaagtgccaagctggcctaacttcagtctccacccactcagtgtggggaaactccatcgcataaaacccctccccccaacctaaagacgacgtactccaaaagctcgagaactaatcgaggtgcctggacggcgcccggtactccgtggagtcacatgaagcgacggctgaggacggaaaggcccttttcctttgtgtgggtgactcacccgcccgctctcccgagcgccgcgtcctccattttgagctccctgcagcagggccgggaagcggccatctttccgctcacgcaactggtgccgaccgggccagccttgccgcccagggcggggcgatacacggcggcgcgaggccaggcaccagagcaggccggccagcttgagactacccccgtccgattctcggtggccgcgctcgcaggccccgcctcgccgaacatgtgcgctgggacgcacgggccccgtcgccgcccgcggccccaaaaaccgaaataccagtgtgcagatcttggcccgcatttacaagactatcttgccagaaaaaaagcgtcgcagcaggtcatcaaaaattttaaatggctagagacttatcgaaagcagcgagacaggcgcgaaggtgccaccagattcgcacgcggcggccccagcgcccaggccaggcctcaactcaagcacgaggcgaaggggctccttaagcgcaaggcctcgaactctcccacccacttccaacccgaagctcgggatcaagaatcacgtactgcagccaggggcgtggaagtaattcaaggcacgcaagggccataacccgtaaagaggccaggcccgcgggaaccacacacggcacttacctgtgttctggcggcaaacccgttgcgaaaaagaacgttcacggcgactactgcacttatatacggttctcccccaccctcgggaaaaaggcggagccagtacacgacatcactttcccagtttaccccgcgccaccttctctaggcaccggttcaattgccgacccctccccccaacttctcggggactgtgggcgatgtgcgctctgcccactgacgggcaccggagccaattcgaatcgcctgcttttctgcctggtactaacttctctcccctctcctcttttctttttctgcagggcggccgcggaagttcctatacttcaaatagaataggaacttccggcgggtcacccgaggatgagaatgctgctctggaagagaagatcgcccagctgaagcagaagaacgccgctctgaaagaagagatccaggctctggaatacggaggcggaggcatgatgctgaagaagatcctgaagatcgaagaactggacgagcgcgagctgatcgacatcgaggtgtccggcaaccacctgttctacgccaacgatatcctgacccacaactcgtcttcgtacccagcttttgttccctttagtgagggttaattgcgcgcttggcgtaatcatggtcatagctgtttcctgtgtgaaattgttatccgctcacaattccacacaacatacgagccggaagcataaagtgtaaagcctggggtgcctaatgagtgagctaactcacattaattgcgttgcgctcactgcccgctttccagtcgggaaacctgtcgtgccagctgcattaatgaatcggccaacgcgcggggagaggcggtttgcgtattgggcgctcttccgcttcctcgctcactgactcgctgcgctcggtcgttcggctgcggcgagcggtatcagctcactcaaaggcggtaatacggttatccacagaatcaggggataacgcaggaaagaacatgtgagcaaaaggccagcaaaaggccaggaaccgtaaaaaggccgcgttgctggcgtttttccataggctccgcccccctgacgagcatcacaaaaatcgacgctcaagtcagaggtggcgaaacccgacaggactataaagataccaggcgtttccccctggaagctccctcgtgcgctctcctgttccgaccctgccgcttaccggatacctgtccgcctttctcccttcgggaagcgtggcgctttctcatagctcacgctgtaggtatctcagttcggtgtaggtcgttcgctccaagctgggctgtgtgcacgaaccccccgttcagcccgaccgctgcgccttatccggtaactatcgtcttgagtccaacccggtaagacacgacttatcgccactggcagcagccactggtaacaggattagcagagcgaggtatgtaggcggtgctacagagttcttgaagtggtggcctaactacggctacactagaaggacagtatttggtatctgcgctctgctgaagccagttaccttcggaaaaagagttggtagctcttgatccggcaaacaaaccaccgctggtagcggtggtttttttgtttgcaagcagcagattacgcgcagaaaaaaaggatctcaagaagatcctttgatcttttctacggggtctgacgctcagtggaacgaaaactcacgttaagggattttggtcatgagattatcaaaaaggatcttcacctagatccttttaaattaaaaatgaagttttaaatcaatctaaagtatatatgagtaaacttggtctgacagttaccaatgcttaatcagtgaggcacctatctcagcgatctgtctatttcgttcatccatagttgcctgactccccgtcgtgtagataactacgatacgggagggcttaccatctggccccagtgctgcaatgataccgcgagacccacgctcaccggctccagatttatcagcaataaaccagccagccggaagggccgagcgcagaagtggtcctgcaactttatccgcctccatccagtctattaattgttgccgggaagctagagtaagtagttcgccagttaatagtttgcgcaacgttgttgccattgctacaggcatcgtggtgtcacgctcgtcgtttggtatggcttcattcagctccggttcccaacgatcaaggcgagttacatgatcccccatgttgtgcaaaaaagcggttagctccttcggtcctccgatcgttgtcagaagtaagttggccgcagtgttatcactcatggttatggcagcactgcataattctcttactgtcatgccatccgtaagatgcttttctgtgactggtgagtactcaaccaagtcattctgagaatagtgtatgcggcgaccgagttgctcttgcccggcgtcaatacgggataataccgcgccacatagcagaactttaaaagtgctcatcattggaaaacgttcttcggggcgaaaactctcaaggatcttaccgctgttgagatccagttcgatgtaacccactcgtgcacccaactgatcttcagcatcttttactttcaccagcgtttctgggtgagcaaaaacaggaaggcaaaatgccgcaaaaaagggaataagggcgacacggaaatgttgaatactcatactcttcctttttcaatattattgaagcatttatcagggttattgtctcatgagcggatacatatttgaatgtatttagaaaaataaacaaataggggttccgcgcacatttccccgaaaagtgccac

SEQ ID NO: 50 - DNA, 7284 bp, Artificial
  Vector comprising split intein - heterologous polynucleotide construct
ctaaattgtaagcgttaatattttgttaaaattcgcgttaaatttttgttaaatcagctcattttttaaccaataggccgaaatcggcaaaatcccttataaatcaaaagaatagaccgagatagggttgagtgttgttccagtttggaacaagagtccactattaaagaacgtggactccaacgtcaaagggcgaaaaaccgtctatcagggcgatggcccactacgtgaaccatcaccctaatcaagttttttggggtcgaggtgccgtaaagcactaaatcggaaccctaaagggagcccccgatttagagcttgacggggaaagccggcgaacgtggcgagaaaggaagggaagaaagcgaaaggagcgggcgctagggcgctggcaagtgtagcggtcacgctgcgcgtaaccaccacacccgccgcgcttaatgcgccgctacagggcgcgtcccattcgccattcaggctgcgcaactgttgggaagggcgatcggtgcgggcctcttcgctattacgccagctggcgaaagggggatgtgctgcaaggcgattaagttgggtaacgccagggttttcccagtcacgacgttgtaaaacgacggccagtgagcgcgcgtaatacgactcactatagggcgaattggagctgaagactctgcctggaccttaagacccaggtgcagaccccccagggcatgaaggaaatcagcaacatccaagtgggcgacctggtgctgagcaacaccggctacaacgaggtgctgaacgtgttccccaagagcaagaagaagtcctacaagatcaccctggaagatggcaaagagatcatctgctccgaggaacacctgttcccaacccagaccggcgagatgaacatctctggcggcctgaaagagggcatgtgcctgtacgtgaaagaaggcggcggaggacctgaggataagctccaggccattaagtacgagctggcccagaacgaggaagaactggctcagatcgaagagaagctggccgccaacaaagaaggcggatccggcggaggcggatctggaaccggttttgctaatgagctgggccccagactgatgggcaaaggcagcggaggaggcggaagcggacctcctaggaagagatgttgttgcgctagaagaggcacccagctgatgctcgtgggcctgctgtctacagctatgtgggctggactgctggctctgctgctgctttggcattgggagacggaaggtggtggtggatctggtggcggaggctctgaaatcggcacaggcttccctttcgaccctcactacgtggaagtgctgggcgagagaatgcactatgtggatgtgggccctagagatggaacccctgtgctgtttctgcacggcaaccctaccagctcttacgtgtggcggaacatcatccctcacgtggcccctacacacagagtgatcgcccctgatctgatcggcatgggcaagagcgacaagcctgacctgggctacttcttcgacgaccacgtgcggttcatggacgccttcatcgaggctctgggactcgaagaggtggtgctggtcatccacgattggggctctgctctgggcttccactgggccaagagaaaccccgaaagagtgaagggaatcgccttcatggagttcatcagacccattcctacctgggacgagtggcccgagttcgccagagagacattccaggccttcagaacaaccgacgtgggcagaaagctgatcatcgaccagaatgtgtttatcgagggcaccctgcctatgggcgtcgtcagacctctgaccgaggtggaaatggaccactacagagagccttttctgaaccccgtggatagagaacctctgtggcggttccctaacgagctgcctattgctggcgagcccgctaacattgtggccctggtcgaagagtacatggactggctgcatcagagccccgtgcctaagctgctgttttggggaactcccggcgtgctgatccctcctgctgaagctgctagactggctaagagcctgcctaacgctaaggccgtggacatcggacctggcctgaatctgctgcaagaggataaccccgacctgatcggctctgagatcgccagatggctgagcacactggaaatttctggcggtggtggcggtagcggtggcggtggaagcgctcaccactttagcgagcccgagatcaccctgatcatcttcggcgtgatggccctcgtgatcggcaccatcctgctgatctcttacggcatcagacggctgatcaagaagtccccctcaggcggaggcggctctaccggttccggaggcagcggcttctgctacgagaacgaagtcggcagtggcaggtccagattcgtgaagaaggacggccactgcaacgtgcagttcatcaacgtcggaagcggcaagagcagaatcacctctgagggcgagtacatccctctggaccagatcgatattaatgtcggttccggaggaagttcctatacttcaaatagaataggaacttcgcaggtaagtatcctttttacagcacaacttaatgagacagatagaaactggtcttgtagaaacagagtaggctagcccccagctggttctttccgcctcagaagccatagagcccaccgcatccccagcatgcctgctattctcttcccaatcctcccccttgctgtcctgccccaccccaccccccagaatagaatgacacctactcagacaatgcgatgcaatttcctcattttattaggaaaggacagtgggagtggcaccttccagggtcaaggaaggcacgggggaggggcaaacaacagatggctggcaactagaaggcacagtcgaggctgatcagcgagccgccggcgtctagagaattgatcccctcaggcgccaggctttctggtcatgcaccaggttctagggccctcaggcacttccacgtcggcggtcacggtgaagcccagtctctcgtagaagggcaggtttctgggggcgcttgtttccaggaaggcgggcacgccagccctttcagcagcttccaccccaggcagcaccacagcagatcccagtcccttgccctggtggtcaggtgacacgcccacggtggccagaaaccaggcaggctcttttggtctgtggggggccagcaggccttccatctgctgctgggcagccagtctagagccgctcagctcggccattctaggtccgatctcggcgaacacagcgccggcttccacagactcaggggttgtccacacagccacagcggcgccatcatcggccacccacactttgccgatgtccaggcccactctggtcagaaacagttcctgcagctcggtcactctctcgatgtgccggtcggggtccacggtgtgtcttgtggcagggtaatcggcgaaggcagcggccagtgtccgcacagctcttggcacatcgtccctggtggccagccgcactgtgggcttgtactcggtcatggtggcgcgccttttaggggtagttttcacgacacctgaaatggaagaaaaaaactttgaaccactgtctgaggcttgagaatgaaccaagatccaaactcaaaaagggcaaattccaaggagaattacatcaagtgccaagctggcctaacttcagtctccacccactcagtgtggggaaactccatcgcataaaacccctccccccaacctaaagacgacgtactccaaaagctcgagaactaatcgaggtgcctggacggcgcccggtactccgtggagtcacatgaagcgacggctgaggacggaaaggcccttttcctttgtgtgggtgactcacccgcccgctctcccgagcgccgcgtcctccattttgagctccctgcagcagggccgggaagcggccatctttccgctcacgcaactggtgccgaccgggccagccttgccgcccagggcggggcgatacacggcggcgcgaggccaggcaccagagcaggccggccagcttgagactacccccgtccgattctcggtggccgcgctcgcaggccccgcctcgccgaacatgtgcgctgggacgcacgggccccgtcgccgcccgcggccccaaaaaccgaaataccagtgtgcagatcttggcccgcatttacaagactatcttgccagaaaaaaagcgtcgcagcaggtcatcaaaaattttaaatggctagagacttatcgaaagcagcgagacaggcgcgaaggtgccaccagattcgcacgcggcggccccagcgcccaggccaggcctcaactcaagcacgaggcgaaggggctccttaagcgcaaggcctcgaactctcccacccacttccaacccgaagctcgggatcaagaatcacgtactgcagccaggggcgtggaagtaattcaaggcacgcaagggccataacccgtaaagaggccaggcccgcgggaaccacacacggcacttacctgtgttctggcggcaaacccgttgcgaaaaagaacgttcacggcgactactgcacttatatacggttctcccccaccctcgggaaaaaggcggagccagtacacgacatcactttcccagtttaccccgcgccaccttctctaggcaccggttcaattgccgacccctccccccaacttctcggggactgtgggcgatgtgcgctctgcccactgacgggcaccggagccaattcgaatcgcctgcttttctgcctggtactaacttctctcccctctcctcttttctttttctgcagggcggccgcggaagttcctatacttcaaatagaataggaacttccggcgggtcacccgaggatgagaatgctgctctggaagagaagatcgcccagctgaagcagaagaacgccgctctgaaagaagagatccaggctctggaatacggaggcggaggcatgatgctgaagaagatcctgaagatcgaagaactggacgagcgcgagctgatcgacatcgaggtgtccggcaaccacctgttctacgccaacgatatcctgacccacaactcgtcttcgtacccagcttttgttccctttagtgagggttaattgcgcgcttggcgtaatcatggtcatagctgtttcctgtgtgaaattgttatccgctcacaattccacacaacatacgagccggaagcataaagtgtaaagcctggggtgcctaatgagtgagctaactcacattaattgcgttgcgctcactgcccgctttccagtcgggaaacctgtcgtgccagctgcattaatgaatcggccaacgcgcggggagaggcggtttgcgtattgggcgctcttccgcttcctcgctcactgactcgctgcgctcggtcgttcggctgcggcgagcggtatcagctcactcaaaggcggtaatacggttatccacagaatcaggggataacgcaggaaagaacatgtgagcaaaaggccagcaaaaggccaggaaccgtaaaaaggccgcgttgctggcgtttttccataggctccgcccccctgacgagcatcacaaaaatcgacgctcaagtcagaggtggcgaaacccgacaggactataaagataccaggcgtttccccctggaagctccctcgtgcgctctcctgttccgaccctgccgcttaccggatacctgtccgcctttctcccttcgggaagcgtggcgctttctcatagctcacgctgtaggtatctcagttcggtgtaggtcgttcgctccaagctgggctgtgtgcacgaaccccccgttcagcccgaccgctgcgccttatccggtaactatcgtcttgagtccaacccggtaagacacgacttatcgccactggcagcagccactggtaacaggattagcagagcgaggtatgtaggcggtgctacagagttcttgaagtggtggcctaactacggctacactagaaggacagtatttggtatctgcgctctgctgaagccagttaccttcggaaaaagagttggtagctcttgatccggcaaacaaaccaccgctggtagcggtggtttttttgtttgcaagcagcagattacgcgcagaaaaaaaggatctcaagaagatcctttgatcttttctacggggtctgacgctcagtggaacgaaaactcacgttaagggattttggtcatgagattatcaaaaaggatcttcacctagatccttttaaattaaaaatgaagttttaaatcaatctaaagtatatatgagtaaacttggtctgacagttaccaatgcttaatcagtgaggcacctatctcagcgatctgtctatttcgttcatccatagttgcctgactccccgtcgtgtagataactacgatacgggagggcttaccatctggccccagtgctgcaatgataccgcgagacccacgctcaccggctccagatttatcagcaataaaccagccagccggaagggccgagcgcagaagtggtcctgcaactttatccgcctccatccagtctattaattgttgccgggaagctagagtaagtagttcgccagttaatagtttgcgcaacgttgttgccattgctacaggcatcgtggtgtcacgctcgtcgtttggtatggcttcattcagctccggttcccaacgatcaaggcgagttacatgatcccccatgttgtgcaaaaaagcggttagctccttcggtcctccgatcgttgtcagaagtaagttggccgcagtgttatcactcatggttatggcagcactgcataattctcttactgtcatgccatccgtaagatgcttttctgtgactggtgagtactcaaccaagtcattctgagaatagtgtatgcggcgaccgagttgctcttgcccggcgtcaatacgggataataccgcgccacatagcagaactttaaaagtgctcatcattggaaaacgttcttcggggcgaaaactctcaaggatcttaccgctgttgagatccagttcgatgtaacccactcgtgcacccaactgatcttcagcatcttttactttcaccagcgtttctgggtgagcaaaaacaggaaggcaaaatgccgcaaaaaagggaataagggcgacacggaaatgttgaatactcatactcttcctttttcaatattattgaagcatttatcagggttattgtctcatgagcggatacatatttgaatgtatttagaaaaataaacaaataggggttccgcgcacatttccccgaaaagtgccac

SEQ ID NO: 51 - DNA, 8127 bp, Artificial
  Vector comprising split intein - heterologous polynucleotide construct
ctaaattgtaagcgttaatattttgttaaaattcgcgttaaatttttgttaaatcagctcattttttaaccaataggccgaaatcggcaaaatcccttataaatcaaaagaatagaccgagatagggttgagtgttgttccagtttggaacaagagtccactattaaagaacgtggactccaacgtcaaagggcgaaaaaccgtctatcagggcgatggcccactacgtgaaccatcaccctaatcaagttttttggggtcgaggtgccgtaaagcactaaatcggaaccctaaagggagcccccgatttagagcttgacggggaaagccggcgaacgtggcgagaaaggaagggaagaaagcgaaaggagcgggcgctagggcgctggcaagtgtagcggtcacgctgcgcgtaaccaccacacccgccgcgcttaatgcgccgctacagggcgcgtcccattcgccattcaggctgcgcaactgttgggaagggcgatcggtgcgggcctcttcgctattacgccagctggcgaaagggggatgtgctgcaaggcgattaagttgggtaacgccagggttttcccagtcacgacgttgtaaaacgacggccagtgagcgcgcgtaatacgactcactatagggcgaattggagctgaagactctgcctggaccttaagacccaggtgcagaccccccagggcatgaaggaaatcagcaacatccaagtgggcgacctggtgctgagcaacaccggctacaacgaggtgctgaacgtgttccccaagagcaagaagaagtcctacaagatcaccctggaagatggcaaagagatcatctgctccgaggaacacctgttcccaacccagaccggcgagatgaacatctctggcggcctgaaagagggcatgtgcctgtacgtgaaagaaggcggcggaggacctgaggataagctccaggccattaagtacgagctggcccagaacgaggaagaactggctcagatcgaagagaagctggccgccaacaaagaaggcggatccggcggaggcggatctggaaccggttttgctaatgagctgggccccagactgatgggcaaaggcagcggaggaggcggaagcggacctcctaggaagagatgttgttgcgctagaagaggcacccagctgatgctcgtgggcctgctgtctacagctatgtgggctggactgctggctctgctgctgctttggcattgggagacggaaggtggtggtggatctggtggcggaggtagcggtggtggcggtagcggaggcggtggatctagaaaacgtacccagcctaccttcggcttcaccgtgaactggaagttcagcgagagcaccaccgtgttcaccggccagtgcttcatcgacagaaacggcaaagaggtgctgaaaaccatgtggctgctgagaagcagcgtgaacgacatcggcgacgactggaaggccaccagagtgggcatcaacatcttcaccagactgaggacccagaaagagggcggctctggcggaagcgccagaaagtgtagcctgaccggcaagtggaccaacgacctgggcagcaacatgaccatcggcgccgtgaacagcagaggcgagttcacaggcacctacatcaccgccgtgaccgccaccagcaacgagatcaaagagagccccctgcacggcacccagaacaccatcaacaagagcggcggcagcacaacagtgtttacaggacagtgttttatcgaccggaatgggaaagaagtgctgaaaacaatgtggctgctgcggtcctccgtgaacgacattggagatgattggaaagctacacgagtggggattaacatttttacccggctgcgcacacagaaagaagggggcagcggcggctccgctagaaagtgttctctgactggaaaatggacaaacgatctggggtccaatatgacaatcggggcagtgaactctaggggcgagtttaccggaacatatattacagccgtgacagctacctctaacgaaatcaaagagtctcctctgcacgggacacagaataccattaacaaaagaacccagcccacattcgggtttacagtgaattggaaattctccgagggcggcagcggaagcggatctggctctggatctggcaggacacagcccacctttggattcactgtgaattggaagttttctgagtctaccacagtgttcactgggcagtgtttcattgatcgcaatggaaaagaggtgctgaaaactatgtggctgctgcgctcaagtgtgaatgacatcggggatgattggaaggcaactcgcgtgggaatcaatatctttacacggctgagaactcagaaagaggggggaagcggaggcagcgcccggaaatgctctctgacagggaagtggactaatgatctgggctctaacatgactattggagctgtgaatagccggggagagttcaccgggacttatatcactgctgtgactgccacctcaaatgagatcaaagaatcccccctgcatggaacacagaacactattaacaagtccggcggctccacaaccgtgttcacagggcagtgctttattgaccggaacggcaaagaggtgctgaaaacaatgtggctgctgcgaagctctgtgaatgatattggggacgactggaaagcaactagagtggggatcaatattttcactcgcctgcggacccagaaagaaggcggaagcggaggatctgccagaaagtgctcactgacaggcaaatggacaaatgacctggggagtaatatgactattggggccgtgaacagtcgcggcgagtttactgggacttacattaccgcagtgacagcaacatccaatgagatcaaagaaagtcctctgcatggcactcagaacacaatcaacaaaaggacccagccaacctttggctttaccgtgaattggaagttctctgaaggcggcggaggatccggcggagggggaagtggcgggggaggcagtgggggcggaggaagcgctcaccactttagcgagcccgagatcaccctgatcatcttcggcgtgatggccctcgtgatcggcaccatcctgctgatctcttacggcatcagacggctgatcaagaagtccccctcaggcggaggcggctctaccggttccggaggcagcggcttctgctacgagaacgaagtcggcagtggcaggtccagattcgtgaagaaggacggccactgcaacgtgcagttcatcaacgtcggaagcggcaagagcagaatcacctctgagggcgagtacatccctctggaccagatcgatattaatgtcggttccggaggaagttcctatacttcaaatagaataggaacttcgcaggtaagtatcctttttacagcacaacttaatgagacagatagaaactggtcttgtagaaacagagtaggctagcccccagctggttctttccgcctcagaagccatagagcccaccgcatccccagcatgcctgctattctcttcccaatcctcccccttgctgtcctgccccaccccaccccccagaatagaatgacacctactcagacaatgcgatgcaatttcctcattttattaggaaaggacagtgggagtggcaccttccagggtcaaggaaggcacgggggaggggcaaacaacagatggctggcaactagaaggcacagtcgaggctgatcagcgagccgccggcgtctagagaattgatcccctcaggcgccaggctttctggtcatgcaccaggttctagggccctcaggcacttccacgtcggcggtcacggtgaagcccagtctctcgtagaagggcaggtttctgggggcgcttgtttccaggaaggcgggcacgccagccctttcagcagcttccaccccaggcagcaccacagcagatcccagtcccttgccctggtggtcaggtgacacgcccacggtggccagaaaccaggcaggctcttttggtctgtggggggccagcaggccttccatctgctgctgggcagccagtctagagccgctcagctcggccattctaggtccgatctcggcgaacacagcgccggcttccacagactcaggggttgtccacacagccacagcggcgccatcatcggccacccacactttgccgatgtccaggcccactctggtcagaaacagttcctgcagctcggtcactctctcgatgtgccggtcggggtccacggtgtgtcttgtggcagggtaatcggcgaaggcagcggccagtgtccgcacagctcttggcacatcgtccctggtggccagccgcactgtgggcttgtactcggtcatggtggcgcgccttttaggggtagttttcacgacacctgaaatggaagaaaaaaactttgaaccactgtctgaggcttgagaatgaaccaagatccaaactcaaaaagggcaaattccaaggagaattacatcaagtgccaagctggcctaacttcagtctccacccactcagtgtggggaaactccatcgcataaaacccctccccccaacctaaagacgacgtactccaaaagctcgagaactaatcgaggtgcctggacggcgcccggtactccgtggagtcacatgaagcgacggctgaggacggaaaggcccttttcctttgtgtgggtgactcacccgcccgctctcccgagcgccgcgtcctccattttgagctccctgcagcagggccgggaagcggccatctttccgctcacgcaactggtgccgaccgggccagccttgccgcccagggcggggcgatacacggcggcgcgaggccaggcaccagagcaggccggccagcttgagactacccccgtccgattctcggtggccgcgctcgcaggccccgcctcgccgaacatgtgcgctgggacgcacgggccccgtcgccgcccgcggccccaaaaaccgaaataccagtgtgcagatcttggcccgcatttacaagactatcttgccagaaaaaaagcgtcgcagcaggtcatcaaaaattttaaatggctagagacttatcgaaagcagcgagacaggcgcgaaggtgccaccagattcgcacgcggcggccccagcgcccaggccaggcctcaactcaagcacgaggcgaaggggctccttaagcgcaaggcctcgaactctcccacccacttccaacccgaagctcgggatcaagaatcacgtactgcagccaggggcgtggaagtaattcaaggcacgcaagggccataacccgtaaagaggccaggcccgcgggaaccacacacggcacttacctgtgttctggcggcaaacccgttgcgaaaaagaacgttcacggcgactactgcacttatatacggttctcccccaccctcgggaaaaaggcggagccagtacacgacatcactttcccagtttaccccgcgccaccttctctaggcaccggttcaattgccgacccctccccccaacttctcggggactgtgggcgatgtgcgctctgcccactgacgggcaccggagccaattcgaatcgcctgcttttctgcctggtactaacttctctcccctctcctcttttctttttctgcagggcggccgcggaagttcctatacttcaaatagaataggaacttccggcgggtcacccgaggatgagaatgctgctctggaagagaagatcgcccagctgaagcagaagaacgccgctctgaaagaagagatccaggctctggaatacggaggcggaggcatgatgctgaagaagatcctgaagatcgaagaactggacgagcgcgagctgatcgacatcgaggtgtccggcaaccacctgttctacgccaacgatatcctgacccacaactcgtcttcgtacccagcttttgttccctttagtgagggttaattgcgcgcttggcgtaatcatggtcatagctgtttcctgtgtgaaattgttatccgctcacaattccacacaacatacgagccggaagcataaagtgtaaagcctggggtgcctaatgagtgagctaactcacattaattgcgttgcgctcactgcccgctttccagtcgggaaacctgtcgtgccagctgcattaatgaatcggccaacgcgcggggagaggcggtttgcgtattgggcgctcttccgcttcctcgctcactgactcgctgcgctcggtcgttcggctgcggcgagcggtatcagctcactcaaaggcggtaatacggttatccacagaatcaggggataacgcaggaaagaacatgtgagcaaaaggccagcaaaaggccaggaaccgtaaaaaggccgcgttgctggcgtttttccataggctccgcccccctgacgagcatcacaaaaatcgacgctcaagtcagaggtggcgaaacccgacaggactataaagataccaggcgtttccccctggaagctccctcgtgcgctctcctgttccgaccctgccgcttaccggatacctgtccgcctttctcccttcgggaagcgtggcgctttctcatagctcacgctgtaggtatctcagttcggtgtaggtcgttcgctccaagctgggctgtgtgcacgaaccccccgttcagcccgaccgctgcgccttatccggtaactatcgtcttgagtccaacccggtaagacacgacttatcgccactggcagcagccactggtaacaggattagcagagcgaggtatgtaggcggtgctacagagttcttgaagtggtggcctaactacggctacactagaaggacagtatttggtatctgcgctctgctgaagccagttaccttcggaaaaagagttggtagctcttgatccggcaaacaaaccaccgctggtagcggtggtttttttgtttgcaagcagcagattacgcgcagaaaaaaaggatctcaagaagatcctttgatcttttctacggggtctgacgctcagtggaacgaaaactcacgttaagggattttggtcatgagattatcaaaaaggatcttcacctagatccttttaaattaaaaatgaagttttaaatcaatctaaagtatatatgagtaaacttggtctgacagttaccaatgcttaatcagtgaggcacctatctcagcgatctgtctatttcgttcatccatagttgcctgactccccgtcgtgtagataactacgatacgggagggcttaccatctggccccagtgctgcaatgataccgcgagacccacgctcaccggctccagatttatcagcaataaaccagccagccggaagggccgagcgcagaagtggtcctgcaactttatccgcctccatccagtctattaattgttgccgggaagctagagtaagtagttcgccagttaatagtttgcgcaacgttgttgccattgctacaggcatcgtggtgtcacgctcgtcgtttggtatggcttcattcagctccggttcccaacgatcaaggcgagttacatgatcccccatgttgtgcaaaaaagcggttagctccttcggtcctccgatcgttgtcagaagtaagttggccgcagtgttatcactcatggttatggcagcactgcataattctcttactgtcatgccatccgtaagatgcttttctgtgactggtgagtactcaaccaagtcattctgagaatagtgtatgcggcgaccgagttgctcttgcccggcgtcaatacgggataataccgcgccacatagcagaactttaaaagtgctcatcattggaaaacgttcttcggggcgaaaactctcaaggatcttaccgctgttgagatccagttcgatgtaacccactcgtgcacccaactgatcttcagcatcttttactttcaccagcgtttctgggtgagcaaaaacaggaaggcaaaatgccgcaaaaaagggaataagggcgacacggaaatgttgaatactcatactcttcctttttcaatattattgaagcatttatcagggttattgtctcatgagcggatacatatttgaatgtatttagaaaaataaacaaataggggttccgcgcacatttccccgaaaagtgccac

SEQ ID NO: 52 - DNA, 6573 bp, Artificial
  Vector comprising split intein - heterologous polynucleotide construct
ctaaattgtaagcgttaatattttgttaaaattcgcgttaaatttttgttaaatcagctcattttttaaccaataggccgaaatcggcaaaatcccttataaatcaaaagaatagaccgagatagggttgagtgttgttccagtttggaacaagagtccactattaaagaacgtggactccaacgtcaaagggcgaaaaaccgtctatcagggcgatggcccactacgtgaaccatcaccctaatcaagttttttggggtcgaggtgccgtaaagcactaaatcggaaccctaaagggagcccccgatttagagcttgacggggaaagccggcgaacgtggcgagaaaggaagggaagaaagcgaaaggagcgggcgctagggcgctggcaagtgtagcggtcacgctgcgcgtaaccaccacacccgccgcgcttaatgcgccgctacagggcgcgtcccattcgccattcaggctgcgcaactgttgggaagggcgatcggtgcgggcctcttcgctattacgccagctggcgaaagggggatgtgctgcaaggcgattaagttgggtaacgccagggttttcccagtcacgacgttgtaaaacgacggccagtgagcgcgcgtaatacgactcactatagggcgaattggagctgaagactctgcctggaccttaagacccaggtgcagaccccccagggcatgaaggaaatcagcaacatccaagtgggcgacctggtgctgagcaacaccggctacaacgaggtgctgaacgtgttccccaagagcaagaagaagtcctacaagatcaccctggaagatggcaaagagatcatctgctccgaggaacacctgttcccaacccagaccggcgagatgaacatctctggcggcctgaaagagggcatgtgcctgtacgtgaaagaaggcggcggaggacctgaggataagctccaggccattaagtacgagctggcccagaacgaggaagaactggctcagatcgaagagaagctggccgccaacaaagaaggcggatccgtgtccaagggcgaagaggacaacatggccagcctgcctgccacccacgagctgcacatcttcggcagcatcaacggcgtggacttcgacatggtgggacagggcaccggcaaccccaacgacggatacgaggaactgaacctgaagtccaccaagggggacctccagttcagcccctggattctggtgccccacatcggctacggcttccaccagtacctgccctaccctgacggcatgagccctttccaggccgctatggtggacggctctggctaccaggtgcacagaaccatgcagttcgaggacggcgccagcctgaccgtgaactacagatacacctacgagggcagccacatcaagggcgaggcccaagtgaagggcacaggcttccctgctgacggccccgtgatgaccaactctctgacagccgccgactggtgcagaagcaagaaaacctaccctaacgacaagaccatcatcagcaccttcaagtggtcctacaccacaggcaacggcaagagatacagaagcaccgccagaaccacctacaccttcgccaagcccatggccgccaactacctgaagaaccagcctatgtacgtgttccgaaagaccgagctgaagcacagcaagacagaactgaacttcaaagagtggcagaaagccttcaccgacgtgatgggcatggacgagctgtacaagggaaccggtttcgccaacgagctgggccccagactgatgggcaaaggctccggaggaagttcctatacttcaaatagaataggaacttcgcaggtaagtatcctttttacagcacaacttaatgagacagatagaaactggtcttgtagaaacagagtaggctagcccccagctggttctttccgcctcagaagccatagagcccaccgcatccccagcatgcctgctattctcttcccaatcctcccccttgctgtcctgccccaccccaccccccagaatagaatgacacctactcagacaatgcgatgcaatttcctcattttattaggaaaggacagtgggagtggcaccttccagggtcaaggaaggcacgggggaggggcaaacaacagatggctggcaactagaaggcacagtcgaggctgatcagcgagccgccggcgtctagagaattgatcccctcaggcgccaggctttctggtcatgcaccaggttctagggccctcaggcacttccacgtcggcggtcacggtgaagcccagtctctcgtagaagggcaggtttctgggggcgcttgtttccaggaaggcgggcacgccagccctttcagcagcttccaccccaggcagcaccacagcagatcccagtcccttgccctggtggtcaggtgacacgcccacggtggccagaaaccaggcaggctcttttggtctgtggggggccagcaggccttccatctgctgctgggcagccagtctagagccgctcagctcggccattctaggtccgatctcggcgaacacagcgccggcttccacagactcaggggttgtccacacagccacagcggcgccatcatcggccacccacactttgccgatgtccaggcccactctggtcagaaacagttcctgcagctcggtcactctctcgatgtgccggtcggggtccacggtgtgtcttgtggcagggtaatcggcgaaggcagcggccagtgtccgcacagctcttggcacatcgtccctggtggccagccgcactgtgggcttgtactcggtcatggtggcgcgccttttaggggtagttttcacgacacctgaaatggaagaaaaaaactttgaaccactgtctgaggcttgagaatgaaccaagatccaaactcaaaaagggcaaattccaaggagaattacatcaagtgccaagctggcctaacttcagtctccacccactcagtgtggggaaactccatcgcataaaacccctccccccaacctaaagacgacgtactccaaaagctcgagaactaatcgaggtgcctggacggcgcccggtactccgtggagtcacatgaagcgacggctgaggacggaaaggcccttttcctttgtgtgggtgactcacccgcccgctctcccgagcgccgcgtcctccattttgagctccctgcagcagggccgggaagcggccatctttccgctcacgcaactggtgccgaccgggccagccttgccgcccagggcggggcgatacacggcggcgcgaggccaggcaccagagcaggccggccagcttgagactacccccgtccgattctcggtggccgcgctcgcaggccccgcctcgccgaacatgtgcgctgggacgcacgggccccgtcgccgcccgcggccccaaaaaccgaaataccagtgtgcagatcttggcccgcatttacaagactatcttgccagaaaaaaagcgtcgcagcaggtcatcaaaaattttaaatggctagagacttatcgaaagcagcgagacaggcgcgaaggtgccaccagattcgcacgcggcggccccagcgcccaggccaggcctcaactcaagcacgaggcgaaggggctccttaagcgcaaggcctcgaactctcccacccacttccaacccgaagctcgggatcaagaatcacgtactgcagccaggggcgtggaagtaattcaaggcacgcaagggccataacccgtaaagaggccaggcccgcgggaaccacacacggcacttacctgtgttctggcggcaaacccgttgcgaaaaagaacgttcacggcgactactgcacttatatacggttctcccccaccctcgggaaaaaggcggagccagtacacgacatcactttcccagtttaccccgcgccaccttctctaggcaccggttcaattgccgacccctccccccaacttctcggggactgtgggcgatgtgcgctctgcccactgacgggcaccggagccaattcgaatcgcctgcttttctgcctggtactaacttctctcccctctcctcttttctttttctgcagggcggccgcggaagttcctatacttcaaatagaataggaacttccggcgggtcacccgaggatgagaatgctgctctggaagagaagatcgcccagctgaagcagaagaacgccgctctgaaagaagagatccaggctctggaatacggaggcggaggcatgatgctgaagaagatcctgaagatcgaagaactggacgagcgcgagctgatcgacatcgaggtgtccggcaaccacctgttctacgccaacgatatcctgacccacaactcgtcttcgtacccagcttttgttccctttagtgagggttaattgcgcgcttggcgtaatcatggtcatagctgtttcctgtgtgaaattgttatccgctcacaattccacacaacatacgagccggaagcataaagtgtaaagcctggggtgcctaatgagtgagctaactcacattaattgcgttgcgctcactgcccgctttccagtcgggaaacctgtcgtgccagctgcattaatgaatcggccaacgcgcggggagaggcggtttgcgtattgggcgctcttccgcttcctcgctcactgactcgctgcgctcggtcgttcggctgcggcgagcggtatcagctcactcaaaggcggtaatacggttatccacagaatcaggggataacgcaggaaagaacatgtgagcaaaaggccagcaaaaggccaggaaccgtaaaaaggccgcgttgctggcgtttttccataggctccgcccccctgacgagcatcacaaaaatcgacgctcaagtcagaggtggcgaaacccgacaggactataaagataccaggcgtttccccctggaagctccctcgtgcgctctcctgttccgaccctgccgcttaccggatacctgtccgcctttctcccttcgggaagcgtggcgctttctcatagctcacgctgtaggtatctcagttcggtgtaggtcgttcgctccaagctgggctgtgtgcacgaaccccccgttcagcccgaccgctgcgccttatccggtaactatcgtcttgagtccaacccggtaagacacgacttatcgccactggcagcagccactggtaacaggattagcagagcgaggtatgtaggcggtgctacagagttcttgaagtggtggcctaactacggctacactagaaggacagtatttggtatctgcgctctgctgaagccagttaccttcggaaaaagagttggtagctcttgatccggcaaacaaaccaccgctggtagcggtggtttttttgtttgcaagcagcagattacgcgcagaaaaaaaggatctcaagaagatcctttgatcttttctacggggtctgacgctcagtggaacgaaaactcacgttaagggattttggtcatgagattatcaaaaaggatcttcacctagatccttttaaattaaaaatgaagttttaaatcaatctaaagtatatatgagtaaacttggtctgacagttaccaatgcttaatcagtgaggcacctatctcagcgatctgtctatttcgttcatccatagttgcctgactccccgtcgtgtagataactacgatacgggagggcttaccatctggccccagtgctgcaatgataccgcgagacccacgctcaccggctccagatttatcagcaataaaccagccagccggaagggccgagcgcagaagtggtcctgcaactttatccgcctccatccagtctattaattgttgccgggaagctagagtaagtagttcgccagttaatagtttgcgcaacgttgttgccattgctacaggcatcgtggtgtcacgctcgtcgtttggtatggcttcattcagctccggttcccaacgatcaaggcgagttacatgatcccccatgttgtgcaaaaaagcggttagctccttcggtcctccgatcgttgtcagaagtaagttggccgcagtgttatcactcatggttatggcagcactgcataattctcttactgtcatgccatccgtaagatgcttttctgtgactggtgagtactcaaccaagtcattctgagaatagtgtatgcggcgaccgagttgctcttgcccggcgtcaatacgggataataccgcgccacatagcagaactttaaaagtgctcatcattggaaaacgttcttcggggcgaaaactctcaaggatcttaccgctgttgagatccagttcgatgtaacccactcgtgcacccaactgatcttcagcatcttttactttcaccagcgtttctgggtgagcaaaaacaggaaggcaaaatgccgcaaaaaagggaataagggcgacacggaaatgttgaatactcatactcttcctttttcaatattattgaagcatttatcagggttattgtctcatgagcggatacatatttgaatgtatttagaaaaataaacaaataggggttccgcgcacatttccccgaaaagtgccac

SEQ ID NO: 53 - DNA, 4052 bp, Artificial
  Vector comprising split intein - heterologous polynucleotide construct
ctaaattgtaagcgttaatattttgttaaaattcgcgttaaatttttgttaaatcagctcattttttaaccaataggccgaaatcggcaaaatcccttataaatcaaaagaatagaccgagatagggttgagtgttgttccagtttggaacaagagtccactattaaagaacgtggactccaacgtcaaagggcgaaaaaccgtctatcagggcgatggcccactacgtgaaccatcaccctaatcaagttttttggggtcgaggtgccgtaaagcactaaatcggaaccctaaagggagcccccgatttagagcttgacggggaaagccggcgaacgtggcgagaaaggaagggaagaaagcgaaaggagcgggcgctagggcgctggcaagtgtagcggtcacgctgcgcgtaaccaccacacccgccgcgcttaatgcgccgctacagggcgcgtcccattcgccattcaggctgcgcaactgttgggaagggcgatcggtgcgggcctcttcgctattacgccagctggcgaaagggggatgtgctgcaaggcgattaagttgggtaacgccagggttttcccagtcacgacgttgtaaaacgacggccagtgagcgcgcgtaatacgactcactatagggcgaattggagctgaagactctgcctggaccttaagacccaggtgcagaccccccagggcatgaaggaaatcagcaacatccaagtgggcgacctggtgctgagcaacaccggctacaacgaggtgctgaacgtgttccccaagagcaagaagaagtcctacaagatcaccctggaagatggcaaagagatcatctgctccgaggaacacctgttcccaacccagaccggcgagatgaacatctctggcggcctgaaagagggcatgtgcctgtacgtgaaagaaggcggcggaggatccggcggaggcggaagcggtggcggtggaagcggaggtggcggatctggacttgtgcctgagctgaacgagaaggacgacgaccaggtccagaaggccctggcctccagagaaaacacccagctgatgaacagagacaacatcgagatcaccgtgcgggacttcaagacactggccccgagaagatggctgaacagcggcatcatcagctttttcatgaagtacatcgagaagtctacccctaacaccgtggccttcaacagcttcttctacaccaacctgagcgagaggggctaccagggcgttagacggtggatgaagagaaagaaaacccagatcgacaagctggacaagatcttcacccctatcaacctgaaccagagccactgggccctgggcatcatcgacctgaagaagaaaacaatcggctacgtggacagcctgagcaacggccctaacgccatgtctttcgccatcctgaccgacctccagaaatacgtgatggaagagagcaagcacaccatcggcgaggacttcgacctgatccacctggactgtccccagcagcctaacggctacgactgtggcatctacgtgtgcatgaacaccctgtacggcagcgccgatgctcccctggacttcgattacaaggacgccatcagaatgaggcggtttatcgcccacctgatcctgacagacgccctgaaaggtggtggtggttctggcaccggtttcgccaacgagctgggccccagactgatgggcaaaggctccggaggcggaggcatgatgctgaagaagatcctgaagatcgaagaactggacgagcgcgagctgatcgacatcgaggtgtccggcaaccacctgttctacgccaacgatatcctgacccacaactcgtcttcgtacccagcttttgttccctttagtgagggttaattgcgcgcttggcgtaatcatggtcatagctgtttcctgtgtgaaattgttatccgctcacaattccacacaacatacgagccggaagcataaagtgtaaagcctggggtgcctaatgagtgagctaactcacattaattgcgttgcgctcactgcccgctttccagtcgggaaacctgtcgtgccagctgcattaatgaatcggccaacgcgcggggagaggcggtttgcgtattgggcgctcttccgcttcctcgctcactgactcgctgcgctcggtcgttcggctgcggcgagcggtatcagctcactcaaaggcggtaatacggttatccacagaatcaggggataacgcaggaaagaacatgtgagcaaaaggccagcaaaaggccaggaaccgtaaaaaggccgcgttgctggcgtttttccataggctccgcccccctgacgagcatcacaaaaatcgacgctcaagtcagaggtggcgaaacccgacaggactataaagataccaggcgtttccccctggaagctccctcgtgcgctctcctgttccgaccctgccgcttaccggatacctgtccgcctttctcccttcgggaagcgtggcgctttctcatagctcacgctgtaggtatctcagttcggtgtaggtcgttcgctccaagctgggctgtgtgcacgaaccccccgttcagcccgaccgctgcgccttatccggtaactatcgtcttgagtccaacccggtaagacacgacttatcgccactggcagcagccactggtaacaggattagcagagcgaggtatgtaggcggtgctacagagttcttgaagtggtggcctaactacggctacactagaaggacagtatttggtatctgcgctctgctgaagccagttaccttcggaaaaagagttggtagctcttgatccggcaaacaaaccaccgctggtagcggtggtttttttgtttgcaagcagcagattacgcgcagaaaaaaaggatctcaagaagatcctttgatcttttctacggggtctgacgctcagtggaacgaaaactcacgttaagggattttggtcatgagattatcaaaaaggatcttcacctagatccttttaaattaaaaatgaagttttaaatcaatctaaagtatatatgagtaaacttggtctgacagttaccaatgcttaatcagtgaggcacctatctcagcgatctgtctatttcgttcatccatagttgcctgactccccgtcgtgtagataactacgatacgggagggcttaccatctggccccagtgctgcaatgataccgcgagacccacgctcaccggctccagatttatcagcaataaaccagccagccggaagggccgagcgcagaagtggtcctgcaactttatccgcctccatccagtctattaattgttgccgggaagctagagtaagtagttcgccagttaatagtttgcgcaacgttgttgccattgctacaggcatcgtggtgtcacgctcgtcgtttggtatggcttcattcagctccggttcccaacgatcaaggcgagttacatgatcccccatgttgtgcaaaaaagcggttagctccttcggtcctccgatcgttgtcagaagtaagttggccgcagtgttatcactcatggttatggcagcactgcataattctcttactgtcatgccatccgtaagatgcttttctgtgactggtgagtactcaaccaagtcattctgagaatagtgtatgcggcgaccgagttgctcttgcccggcgtcaatacgggataataccgcgccacatagcagaactttaaaagtgctcatcattggaaaacgttcttcggggcgaaaactctcaaggatcttaccgctgttgagatccagttcgatgtaacccactcgtgcacccaactgatcttcagcatcttttactttcaccagcgtttctgggtgagcaaaaacaggaaggcaaaatgccgcaaaaaagggaataagggcgacacggaaatgttgaatactcatactcttcctttttcaatattattgaagcatttatcagggttattgtctcatgagcggatacatatttgaatgtatttagaaaaataaacaaataggggttccgcgcacatttccccgaaaagtgccac

SEQ ID NO: 54 - DNA, 6636 bp, Artificial
  Vector comprising split intein - heterologous polynucleotide construct
ctaaattgtaagcgttaatattttgttaaaattcgcgttaaatttttgttaaatcagctcattttttaaccaataggccgaaatcggcaaaatcccttataaatcaaaagaatagaccgagatagggttgagtgttgttccagtttggaacaagagtccactattaaagaacgtggactccaacgtcaaagggcgaaaaaccgtctatcagggcgatggcccactacgtgaaccatcaccctaatcaagttttttggggtcgaggtgccgtaaagcactaaatcggaaccctaaagggagcccccgatttagagcttgacggggaaagccggcgaacgtggcgagaaaggaagggaagaaagcgaaaggagcgggcgctagggcgctggcaagtgtagcggtcacgctgcgcgtaaccaccacacccgccgcgcttaatgcgccgctacagggcgcgtcccattcgccattcaggctgcgcaactgttgggaagggcgatcggtgcgggcctcttcgctattacgccagctggcgaaagggggatgtgctgcaaggcgattaagttgggtaacgccagggttttcccagtcacgacgttgtaaaacgacggccagtgagcgcgcgtaatacgactcactatagggcgaattggagctgaagactctgcctggaccttaagacccaggtgcagaccccccagggcatgaaggaaatcagcaacatccaagtgggcgacctggtgctgagcaacaccggctacaacgaggtgctgaacgtgttccccaagagcaagaagaagtcctacaagatcaccctggaagatggcaaagagatcatctgctccgaggaacacctgttcccaacccagaccggcgagatgaacatctctggcggcctgaaagagggcatgtgcctgtacgtgaaagaaggcggcggaggacctgaggataagctccaggccattaagtacgagctggcccagaacgaggaagaactggctcagatcgaagagaagctggccgccaacaaagaaggcggatccggcggaggcggaagcggtggcggtggaagcggaggtggcggatctggcgaatctctgttcaagggccccagagactacaaccccatcagcagcaccatctgccacctgaccaacgagtctgacggccacaccacaagcctgtacggcatcggcttcggccccttcatcatcaccaacaagcacctgttcagacggaacaacggcaccctggtggtgcagtctctgcacggcgtgttcaaagtgaagaacaccaccacactccagcagcatctgatcgacggcagagacatgatcatcatcagaatgcccaaggacttcccgccttttccacagaagctgaagttcagagagcctcagagagaggaacggatctgcctcgtgaccaccaacttccagaccaagagcatgagcagcatggtgtccgacacaagctgcacattccctagcggcgacggcatcttctggaagcactggattcagaccaaggacggccagtgtggaagccctctggtgtctaccagagatggcttcatcgtgggcatccacagcgccagcaacttcaccaacacaaacaactacttcaccagcgtgccgaagaacttcatggaactgctgaccaatcaagaggcccagcagtgggtttcaggctggcggctgaatgccgattctgtgctgtggggaggccacaaggtgttcatggtcaagcccgaggaacccttccagcctgtgaaagaggccacacagctgatgaatggtggcggaggttctggcaccggtttcgccaacgagctgggccccagactgatgggcaaaggctccggaggaagttcctatacttcaaatagaataggaacttcgcaggtaagtatcctttttacagcacaacttaatgagacagatagaaactggtcttgtagaaacagagtaggctagcccccagctggttctttccgcctcagaagccatagagcccaccgcatccccagcatgcctgctattctcttcccaatcctcccccttgctgtcctgccccaccccaccccccagaatagaatgacacctactcagacaatgcgatgcaatttcctcattttattaggaaaggacagtgggagtggcaccttccagggtcaaggaaggcacgggggaggggcaaacaacagatggctggcaactagaaggcacagtcgaggctgatcagcgagccgccggcgtctagagaattgatcccctcaggcgccaggctttctggtcatgcaccaggttctagggccctcaggcacttccacgtcggcggtcacggtgaagcccagtctctcgtagaagggcaggtttctgggggcgcttgtttccaggaaggcgggcacgccagccctttcagcagcttccaccccaggcagcaccacagcagatcccagtcccttgccctggtggtcaggtgacacgcccacggtggccagaaaccaggcaggctcttttggtctgtggggggccagcaggccttccatctgctgctgggcagccagtctagagccgctcagctcggccattctaggtccgatctcggcgaacacagcgccggcttccacagactcaggggttgtccacacagccacagcggcgccatcatcggccacccacactttgccgatgtccaggcccactctggtcagaaacagttcctgcagctcggtcactctctcgatgtgccggtcggggtccacggtgtgtcttgtggcagggtaatcggcgaaggcagcggccagtgtccgcacagctcttggcacatcgtccctggtggccagccgcactgtgggcttgtactcggtcatggtggcgcgccttttaggggtagttttcacgacacctgaaatggaagaaaaaaactttgaaccactgtctgaggcttgagaatgaaccaagatccaaactcaaaaagggcaaattccaaggagaattacatcaagtgccaagctggcctaacttcagtctccacccactcagtgtggggaaactccatcgcataaaacccctccccccaacctaaagacgacgtactccaaaagctcgagaactaatcgaggtgcctggacggcgcccggtactccgtggagtcacatgaagcgacggctgaggacggaaaggcccttttcctttgtgtgggtgactcacccgcccgctctcccgagcgccgcgtcctccattttgagctccctgcagcagggccgggaagcggccatctttccgctcacgcaactggtgccgaccgggccagccttgccgcccagggcggggcgatacacggcggcgcgaggccaggcaccagagcaggccggccagcttgagactacccccgtccgattctcggtggccgcgctcgcaggccccgcctcgccgaacatgtgcgctgggacgcacgggccccgtcgccgcccgcggccccaaaaaccgaaataccagtgtgcagatcttggcccgcatttacaagactatcttgccagaaaaaaagcgtcgcagcaggtcatcaaaaattttaaatggctagagacttatcgaaagcagcgagacaggcgcgaaggtgccaccagattcgcacgcggcggccccagcgcccaggccaggcctcaactcaagcacgaggcgaaggggctccttaagcgcaaggcctcgaactctcccacccacttccaacccgaagctcgggatcaagaatcacgtactgcagccaggggcgtggaagtaattcaaggcacgcaagggccataacccgtaaagaggccaggcccgcgggaaccacacacggcacttacctgtgttctggcggcaaacccgttgcgaaaaagaacgttcacggcgactactgcacttatatacggttctcccccaccctcgggaaaaaggcggagccagtacacgacatcactttcccagtttaccccgcgccaccttctctaggcaccggttcaattgccgacccctccccccaacttctcggggactgtgggcgatgtgcgctctgcccactgacgggcaccggagccaattcgaatcgcctgcttttctgcctggtactaacttctctcccctctcctcttttctttttctgcagggcggccgcggaagttcctatacttcaaatagaataggaacttccggcgggtcacccgaggatgagaatgctgctctggaagagaagatcgcccagctgaagcagaagaacgccgctctgaaagaagagatccaggctctggaatacggaggcggaggcatgatgctgaagaagatcctgaagatcgaagaactggacgagcgcgagctgatcgacatcgaggtgtccggcaaccacctgttctacgccaacgatatcctgacccacaactcgtcttcgtacccagcttttgttccctttagtgagggttaattgcgcgcttggcgtaatcatggtcatagctgtttcctgtgtgaaattgttatccgctcacaattccacacaacatacgagccggaagcataaagtgtaaagcctggggtgcctaatgagtgagctaactcacattaattgcgttgcgctcactgcccgctttccagtcgggaaacctgtcgtgccagctgcattaatgaatcggccaacgcgcggggagaggcggtttgcgtattgggcgctcttccgcttcctcgctcactgactcgctgcgctcggtcgttcggctgcggcgagcggtatcagctcactcaaaggcggtaatacggttatccacagaatcaggggataacgcaggaaagaacatgtgagcaaaaggccagcaaaaggccaggaaccgtaaaaaggccgcgttgctggcgtttttccataggctccgcccccctgacgagcatcacaaaaatcgacgctcaagtcagaggtggcgaaacccgacaggactataaagataccaggcgtttccccctggaagctccctcgtgcgctctcctgttccgaccctgccgcttaccggatacctgtccgcctttctcccttcgggaagcgtggcgctttctcatagctcacgctgtaggtatctcagttcggtgtaggtcgttcgctccaagctgggctgtgtgcacgaaccccccgttcagcccgaccgctgcgccttatccggtaactatcgtcttgagtccaacccggtaagacacgacttatcgccactggcagcagccactggtaacaggattagcagagcgaggtatgtaggcggtgctacagagttcttgaagtggtggcctaactacggctacactagaaggacagtatttggtatctgcgctctgctgaagccagttaccttcggaaaaagagttggtagctcttgatccggcaaacaaaccaccgctggtagcggtggtttttttgtttgcaagcagcagattacgcgcagaaaaaaaggatctcaagaagatcctttgatcttttctacggggtctgacgctcagtggaacgaaaactcacgttaagggattttggtcatgagattatcaaaaaggatcttcacctagatccttttaaattaaaaatgaagttttaaatcaatctaaagtatatatgagtaaacttggtctgacagttaccaatgcttaatcagtgaggcacctatctcagcgatctgtctatttcgttcatccatagttgcctgactccccgtcgtgtagataactacgatacgggagggcttaccatctggccccagtgctgcaatgataccgcgagacccacgctcaccggctccagatttatcagcaataaaccagccagccggaagggccgagcgcagaagtggtcctgcaactttatccgcctccatccagtctattaattgttgccgggaagctagagtaagtagttcgccagttaatagtttgcgcaacgttgttgccattgctacaggcatcgtggtgtcacgctcgtcgtttggtatggcttcattcagctccggttcccaacgatcaaggcgagttacatgatcccccatgttgtgcaaaaaagcggttagctccttcggtcctccgatcgttgtcagaagtaagttggccgcagtgttatcactcatggttatggcagcactgcataattctcttactgtcatgccatccgtaagatgcttttctgtgactggtgagtactcaaccaagtcattctgagaatagtgtatgcggcgaccgagttgctcttgcccggcgtcaatacgggataataccgcgccacatagcagaactttaaaagtgctcatcattggaaaacgttcttcggggcgaaaactctcaaggatcttaccgctgttgagatccagttcgatgtaacccactcgtgcacccaactgatcttcagcatcttttactttcaccagcgtttctgggtgagcaaaaacaggaaggcaaaatgccgcaaaaaagggaataagggcgacacggaaatgttgaatactcatactcttcctttttcaatattattgaagcatttatcagggttattgtctcatgagcggatacatatttgaatgtatttagaaaaataaacaaataggggttccgcgcacatttccccgaaaagtgccac

SEQ ID NO: 55 - DNA, 4037 bp, Artificial
  Vector comprising split intein - heterologous polynucleotide construct
ctaaattgtaagcgttaatattttgttaaaattcgcgttaaatttttgttaaatcagctcattttttaaccaataggccgaaatcggcaaaatcccttataaatcaaaagaatagaccgagatagggttgagtgttgttccagtttggaacaagagtccactattaaagaacgtggactccaacgtcaaagggcgaaaaaccgtctatcagggcgatggcccactacgtgaaccatcaccctaatcaagttttttggggtcgaggtgccgtaaagcactaaatcggaaccctaaagggagcccccgatttagagcttgacggggaaagccggcgaacgtggcgagaaaggaagggaagaaagcgaaaggagcgggcgctagggcgctggcaagtgtagcggtcacgctgcgcgtaaccaccacacccgccgcgcttaatgcgccgctacagggcgcgtcccattcgccattcaggctgcgcaactgttgggaagggcgatcggtgcgggcctcttcgctattacgccagctggcgaaagggggatgtgctgcaaggcgattaagttgggtaacgccagggttttcccagtcacgacgttgtaaaacgacggccagtgagcgcgcgtaatacgactcactatagggcgaattggagctgaagactctgcctggaccttaagacccaggtgcagaccccccagggcatgaaggaaatcagcaacatccaagtgggcgacctggtgctgagcaacaccggctacaacgaggtgctgaacgtgttccccaagagcaagaagaagtcctacaagatcaccctggaagatggcaaagagatcatctgctccgaggaacacctgttcccaacccagaccggcgagatgaacatctctggcggcctgaaagagggcatgtgcctgtacgtgaaagaaggcggcggaggatccgtgtccaagggcgaagaggacaacatggccagcctgcctgccacccacgagctgcacatcttcggcagcatcaacggcgtggacttcgacatggtgggacagggcaccggcaaccccaacgacggatacgaggaactgaacctgaagtccaccaagggggacctccagttcagcccctggattctggtgccccacatcggctacggcttccaccagtacctgccctaccctgacggcatgagccctttccaggccgctatggtggacggctctggctaccaggtgcacagaaccatgcagttcgaggacggcgccagcctgaccgtgaactacagatacacctacgagggcagccacatcaagggcgaggcccaagtgaagggcacaggcttccctgctgacggccccgtgatgaccaactctctgacagccgccgactggtgcagaagcaagaaaacctaccctaacgacaagaccatcatcagcaccttcaagtggtcctacaccacaggcaacggcaagagatacagaagcaccgccagaaccacctacaccttcgccaagcccatggccgccaactacctgaagaaccagcctatgtacgtgttccgaaagaccgagctgaagcacagcaagacagaactgaacttcaaagagtggcagaaagccttcaccgacgtgatgggcatggacgagctgtacaagggaaccggtttcgccaacgagctgggccccagactgatgggcaaaggctccggaggcggaggcatgatgctgaagaagatcctgaagatcgaagaactggacgagcgcgagctgatcgacatcgaggtgtccggcaaccacctgttctacgccaacgatatcctgacccacaactcgtcttcgtacccagcttttgttccctttagtgagggttaattgcgcgcttggcgtaatcatggtcatagctgtttcctgtgtgaaattgttatccgctcacaattccacacaacatacgagccggaagcataaagtgtaaagcctggggtgcctaatgagtgagctaactcacattaattgcgttgcgctcactgcccgctttccagtcgggaaacctgtcgtgccagctgcattaatgaatcggccaacgcgcggggagaggcggtttgcgtattgggcgctcttccgcttcctcgctcactgactcgctgcgctcggtcgttcggctgcggcgagcggtatcagctcactcaaaggcggtaatacggttatccacagaatcaggggataacgcaggaaagaacatgtgagcaaaaggccagcaaaaggccaggaaccgtaaaaaggccgcgttgctggcgtttttccataggctccgcccccctgacgagcatcacaaaaatcgacgctcaagtcagaggtggcgaaacccgacaggactataaagataccaggcgtttccccctggaagctccctcgtgcgctctcctgttccgaccctgccgcttaccggatacctgtccgcctttctcccttcgggaagcgtggcgctttctcatagctcacgctgtaggtatctcagttcggtgtaggtcgttcgctccaagctgggctgtgtgcacgaaccccccgttcagcccgaccgctgcgccttatccggtaactatcgtcttgagtccaacccggtaagacacgacttatcgccactggcagcagccactggtaacaggattagcagagcgaggtatgtaggcggtgctacagagttcttgaagtggtggcctaactacggctacactagaaggacagtatttggtatctgcgctctgctgaagccagttaccttcggaaaaagagttggtagctcttgatccggcaaacaaaccaccgctggtagcggtggtttttttgtttgcaagcagcagattacgcgcagaaaaaaaggatctcaagaagatcctttgatcttttctacggggtctgacgctcagtggaacgaaaactcacgttaagggattttggtcatgagattatcaaaaaggatcttcacctagatccttttaaattaaaaatgaagttttaaatcaatctaaagtatatatgagtaaacttggtctgacagttaccaatgcttaatcagtgaggcacctatctcagcgatctgtctatttcgttcatccatagttgcctgactccccgtcgtgtagataactacgatacgggagggcttaccatctggccccagtgctgcaatgataccgcgagacccacgctcaccggctccagatttatcagcaataaaccagccagccggaagggccgagcgcagaagtggtcctgcaactttatccgcctccatccagtctattaattgttgccgggaagctagagtaagtagttcgccagttaatagtttgcgcaacgttgttgccattgctacaggcatcgtggtgtcacgctcgtcgtttggtatggcttcattcagctccggttcccaacgatcaaggcgagttacatgatcccccatgttgtgcaaaaaagcggttagctccttcggtcctccgatcgttgtcagaagtaagttggccgcagtgttatcactcatggttatggcagcactgcataattctcttactgtcatgccatccgtaagatgcttttctgtgactggtgagtactcaaccaagtcattctgagaatagtgtatgcggcgaccgagttgctcttgcccggcgtcaatacgggataataccgcgccacatagcagaactttaaaagtgctcatcattggaaaacgttcttcggggcgaaaactctcaaggatcttaccgctgttgagatccagttcgatgtaacccactcgtgcacccaactgatcttcagcatcttttactttcaccagcgtttctgggtgagcaaaaacaggaaggcaaaatgccgcaaaaaagggaataagggcgacacggaaatgttgaatactcatactcttcctttttcaatattattgaagcatttatcagggttattgtctcatgagcggatacatatttgaatgtatttagaaaaataaacaaataggggttccgcgcacatttccccgaaaagtgccac

SEQ ID NO: 56 - DNA, 8644 bp, Artificial
  Vector comprising split intein - heterologous polynucleotide construct
ggcgcgccggattcgacattgattattgactagttattaatagtaatcaattacggggtcattagttcatagcccatatatggagttccgcgttacataacttacggtaaatggcccgcctggctgaccgcccaacgacccccgcccattgacgtcaataatgacgtatgttcccatagtaacgccaatagggactttccattgacgtcaatgggtggagtatttacggtaaactgcccacttggcagtacatcaagtgtatcatatgccaagtacgccccctattgacgtcaatgacggtaaatggcccgcctggcattatgcccagtacatgaccttatgggactttcctacttggcagtacatctacgtattagtcatcgctattaccatggtcgaggtgagccccacgttctgcttcactctccccatctcccccccctccccacccccaattttgtatttatttattttttaattattttgtgcagcgatgggggcggggggggggggggggcgcgcgccaggcggggcggggcggggcgaggggcggggcggggcgaggcggagaggtgcggcggcagccaatcagagcggcgcgctccgaaagtttccttttatggcgaggcggcggcggcggcggccctataaaaagcgaagcgcgcggcgggcgggagtcgctgcgtcgcgccttcgccccgtgccccgctccgccgccgcctcgcgccgcccgccccggctctgactgaccgcgttactcccacaggtgagcgggcgggacggcccttctcctccgggctgtaattagcgcttggtttaatgacggctcgtttcttttctgtggctgcgtgaaagccttaaagggctccgggagggccctttgtgcgggggggagcggctcggggggtgcgtgcgtgtgtgtgtgcgtggggagcgccgcgtgcggcccgcgctgcccggcggctgtgagcgctgcgggcgcggcgcggggctttgtgcgctccgcgtgtgcgcgaggggagcgcggccgggggcggtgccccgcggtgcgggggggctgcgaggggaacaaaggctgcgtgcggggtgtgtgcgtgggggggtgagcagggggtgtgggcgcggcggtcgggctgtaacccccccctgcacccccctccccgagttgctgagcacggcccggcttcgggtgcggggctccgtgcggggcgtggcgcggggctcgccgtgccgggcggggggtggcggcaggtgggggtgccgggcggggcggggccgcctcgggccggggagggctcgggggaggggcgcggcggccccggagcgccggcggctgtcgaggcgcggcgagccgcagccattgccttttatggtaatcgtgcgagagggcgcagggacttcctttgtcccaaatctggcggagccgaaatctgggaggcgccgccgcaccccctctagcgggcgcgggcgaagcggtgcggcgccggcaggaaggaaatgggcggggagggccttcgtgcgtcgccgcgccgccgtccccttctccatctccagcctcggggctgccgcagggggacggctgccttcgggggggacggggcagggcggggttcggcttctggcgtgtgaccggcggctctagagcctctgctaaccatgttcatgccttcttctttttcctacagatccttaattaataatacgactcactataggggccgccaccatgacaccacctaagaagaaacggaaggtcgaggacggcgagggccctgctgctaagagagtgaaactggactccggagtgtccaagggcgaagaggacaacatggccagcctgcctgccacccacgagctgcacatcttcggcagcatcaacggcgtggacttcgacatggtgggacagggcaccggcaaccccaacgacggatacgaggaactgaacctgaagtccaccaagggggacctccagttcagcccctggattctggtgccccacatcggctacggcttccaccagtacctgccctaccctgacggcatgagccctttccaggccgctatggtggacggctgcctggaccttaagacccaggtgcagaccccccagggcatgaaggaaatcagcaacatccaagtgggcgacctggtgctgagcaacaccggctacaacgaggtgctgaacgtgttccccaagagcaagaagaagtcctacaagatcaccctggaagatggcaaagagatcatctgctccgaggaacacctgttcccaacccagaccggcgagatgaacatctctggcggcctgaaagagggcatgtgcctgtacgtgaaagaaggcggcggaggacctgaggataagctccaggccattaagtacgagctggcccagaacgaggaagaactggctcagatcgaagagaagctggccgccaacaaagaaggcggatccggcggaggcggatctggaaccggttttgctaatgagctgggccccagactgatgggcaaaggcagcggaggaggcggaagcggacctcctaggaagagatgttgttgcgctagaagaggcacccagctgatgctcgtgggcctgctgtctacagctatgtgggctggactgctggctctgctgctgctttggcattgggagacggaaggtggtggtggatctggtggcggaggtagcggtggtggcggtagcggaggcggtggatctagaaaacgtacccagcctaccttcggcttcaccgtgaactggaagttcagcgagagcaccaccgtgttcaccggccagtgcttcatcgacagaaacggcaaagaggtgctgaaaaccatgtggctgctgagaagcagcgtgaacgacatcggcgacgactggaaggccaccagagtgggcatcaacatcttcaccagactgaggacccagaaagagggcggctctggcggaagcgccagaaagtgtagcctgaccggcaagtggaccaacgacctgggcagcaacatgaccatcggcgccgtgaacagcagaggcgagttcacaggcacctacatcaccgccgtgaccgccaccagcaacgagatcaaagagagccccctgcacggcacccagaacaccatcaacaagagcggcggcagcacaacagtgtttacaggacagtgttttatcgaccggaatgggaaagaagtgctgaaaacaatgtggctgctgcggtcctccgtgaacgacattggagatgattggaaagctacacgagtggggattaacatttttacccggctgcgcacacagaaagaagggggcagcggcggctccgctagaaagtgttctctgactggaaaatggacaaacgatctggggtccaatatgacaatcggggcagtgaactctaggggcgagtttaccggaacatatattacagccgtgacagctacctctaacgaaatcaaagagtctcctctgcacgggacacagaataccattaacaaaagaacccagcccacattcgggtttacagtgaattggaaattctccgagggcggcagcggaagcggatctggctctggatctggcaggacacagcccacctttggattcactgtgaattggaagttttctgagtctaccacagtgttcactgggcagtgtttcattgatcgcaatggaaaagaggtgctgaaaactatgtggctgctgcgctcaagtgtgaatgacatcggggatgattggaaggcaactcgcgtgggaatcaatatctttacacggctgagaactcagaaagaggggggaagcggaggcagcgcccggaaatgctctctgacagggaagtggactaatgatctgggctctaacatgactattggagctgtgaatagccggggagagttcaccgggacttatatcactgctgtgactgccacctcaaatgagatcaaagaatcccccctgcatggaacacagaacactattaacaagtccggcggctccacaaccgtgttcacagggcagtgctttattgaccggaacggcaaagaggtgctgaaaacaatgtggctgctgcgaagctctgtgaatgatattggggacgactggaaagcaactagagtggggatcaatattttcactcgcctgcggacccagaaagaaggcggaagcggaggatctgccagaaagtgctcactgacaggcaaatggacaaatgacctggggagtaatatgactattggggccgtgaacagtcgcggcgagtttactgggacttacattaccgcagtgacagcaacatccaatgagatcaaagaaagtcctctgcatggcactcagaacacaatcaacaaaaggacccagccaacctttggctttaccgtgaattggaagttctctgaaggcggcggaggatccggcggagggggaagtggcgggggaggcagtgggggcggaggaagcgctcaccactttagcgagcccgagatcaccctgatcatcttcggcgtgatggccctcgtgatcggcaccatcctgctgatctcttacggcatcagacggctgatcaagaagtccccctcaggcggaggcggctctaccggttccggaggcagcggcttctgctacgagaacgaagtcggcagtggcaggtccagattcgtgaagaaggacggccactgcaacgtgcagttcatcaacgtcggaagcggcaagagcagaatcacctctgagggcgagtacatccctctggaccagatcgatattaatgtcggttccggaggaagttcctatacttcaaatagaataggaacttccggcgggtcacccgaggatgagaatgctgctctggaagagaagatcgcccagctgaagcagaagaacgccgctctgaaagaagagatccaggctctggaatacggaggcggaggcatgatgctgaagaagatcctgaagatcgaagaactggacgagcgcgagctgatcgacatcgaggtgtccggcaaccacctgttctacgccaacgatatcctgacccacaactctggctaccaggtgcacagaaccatgcagttcgaggacggcgccagcctgaccgtgaactacagatacacctacgagggcagccacatcaagggcgaggcccaagtgaagggcacaggcttccctgctgacggccccgtgatgaccaactctctgacagccgccgactggtgcagaagcaagaaaacctaccctaacgacaagaccatcatcagcaccttcaagtggtcctacaccacaggcaacggcaagagatacagaagcaccgccagaaccacctacaccttcgccaagcccatggccgccaactacctgaagaaccagcctatgtacgtgttccgaaagaccgagctgaagcacagcaagacagaactgaacttcaaagagtggcagaaagccttcaccgacgtgatgggcatggacgagctgtacaagtccggagctgctccagccgccaagaagaagaagctcgactacaaggacgacgacgataagtgaacgcgtaaatgattgcagatccactagttctagagctcgctgatcagcctcgactgtgccttctagttgccagccatctgttgtttgcccctcccccgtgccttccttgaccctggaaggtgccactcccactgtcctttcctaataaaatgaggaaattgcatcgcattgtctgagtaggtgtcattctattctggggggtggggtggggcaggacagcaagggggaggattgggaagacaatagcaggcatgctggggatgcggtgggctctatggcttctgaggcggaaagaaccagctggggctcgagatccactagttctagcctcgaggctagagcggccgccactggccgtcgttttacaacgtcgtgactgggaaaaccctggcgttacccaacttaatcgccttgcagcacatccccctttcgccagctggcgtaatagcgaagaggcccgcaccgatcgcccttcccaacagttgcgcagcctgaatggcgaatgggacgcgccctgtagcggcgcattaagcgcggcgggtgtggtggttacgcgcagcgtgaccgctacacttgccagcgccctagcgcccgctcctttcgctttcttcccttcctttctcgccacgttcgccggctttccccgtcaagctctaaatcgggggctccctttagggttccgatttagtgctttacggcacctcgaccccaaaaaacttgattagggtgatggttcacgtagtgggccatcgccctgatagacggtttttcgccctttgacgttggagtccacgttctttaatagtggactcttgttccaaactggaacaacactcaaccctatctcggtctattcttttgatttataagggattttgccgatttcggcctattggttaaaaaatgagctgatttaacaaaaatttaacgcgaattttaacaaaatattaacgcttacaatttaggtggcacttttcggggaaatgtgcgcggaacccctatttgtttatttttctaaatacattcaaatatgtatccgctcatgagacaataaccctgataaatgcttcaataatattgaaaaaggaagagtatgagtattcaacatttccgtgtcgcccttattcccttttttgcggcattttgccttcctgtttttgctcacccagaaacgctggtgaaagtaaaagatgctgaagatcagttgggtgcacgagtgggttacatcgaactggatctcaacagcggtaagatccttgagagttttcgccccgaagaacgttttccaatgatgagcacttttaaagttctgctatgtggcgcggtattatcccgtattgacgccgggcaagagcaactcggtcgccgcatacactattctcagaatgacttggttgagtactcaccagtcacagaaaagcatcttacggatggcatgacagtaagagaattatgcagtgctgccataaccatgagtgataacactgcggccaacttacttctgacaacgatcggaggaccgaaggagctaaccgcttttttgcacaacatgggggatcatgtaactcgccttgatcgttgggaaccggagctgaatgaagccataccaaacgacgagcgtgacaccacgatgcctgtagcaatggcaacaacgttgcgcaaactattaactggcgaactacttactctagcttcccggcaacaattaatagactggatggaggcggataaagttgcaggaccacttctgcgctcggcccttccggctggctggtttattgctgataaatctggagccggtgagcgtgggtctcgcggtatcattgcagcactggggccagatggtaagccctcccgtatcgtagttatctacacgacggggagtcaggcaactatggatgaacgaaatagacagatcgctgagataggtgcctcactgattaagcattggtaactgtcagaccaagtttactcatatatactttagattgatttaaaacttcatttttaatttaaaaggatctaggtgaagatcctttttgataatctcatgaccaaaatcccttaacgtgagttttcgttccactgagcgtcagaccccgtagaaaagatcaaaggatcttcttgagatcctttttttctgcgcgtaatctgctgcttgcaaacaaaaaaaccaccgctaccagcggtggtttgtttgccggatcaagagctaccaactctttttccgaaggtaactggcttcagcagagcgcagataccaaatactgtccttctagtgtagccgtagttaggccaccacttcaagaactctgtagcaccgcctacatacctcgctctgctaatcctgttaccagtggctgctgccagtggcgataagtcgtgtcttaccgggttggactcaagacgatagttaccggataaggcgcagcggtcgggctgaacggggggttcgtgcacacagcccagcttggagcgaacgacctacaccgaactgagatacctacagcgtgagctatgagaaagcgccacgcttcccgaagggagaaaggcggacaggtatccggtaagcggcagggtcggaacaggagagcgcacgagggagcttccagggggaaacgcctggtatctttatagtcctgtcgggtttcgccacctctgacttgagcgtcgatttttgtgatgctcgtcaggggggcggagcctatggaaaaacgccagcaacgcggcctttttacggttcctggccttttgctggccttttgctcacatgttctttcctgcgttatcccctgattctgtggataaccgtattaccgcctttgagtgagctgataccgctcgccgcagccgaacgaccgagcgcagcgagtcagtgagcgaggaagcggaagagcgcccaatacgcaaaccgcctctccccgcgcgttggccgattcattaatgcagctggcacgacaggtttcccgactggaaagcgggcagtgagcgcaacgcaattaatgtgagttagctcactcattaggcaccccaggctttacactttatgcttccggctcgtatgttgtgtggaattgtgagcggataacaatttcacacaggaaacagctatgaccatga

SEQ ID NO: 57 - DNA, 7801 bp, Artificial
  Vector comprising split intein - heterologous polynucleotide construct
ggcgcgccggattcgacattgattattgactagttattaatagtaatcaattacggggtcattagttcatagcccatatatggagttccgcgttacataacttacggtaaatggcccgcctggctgaccgcccaacgacccccgcccattgacgtcaataatgacgtatgttcccatagtaacgccaatagggactttccattgacgtcaatgggtggagtatttacggtaaactgcccacttggcagtacatcaagtgtatcatatgccaagtacgccccctattgacgtcaatgacggtaaatggcccgcctggcattatgcccagtacatgaccttatgggactttcctacttggcagtacatctacgtattagtcatcgctattaccatggtcgaggtgagccccacgttctgcttcactctccccatctcccccccctccccacccccaattttgtatttatttattttttaattattttgtgcagcgatgggggcggggggggggggggggcgcgcgccaggcggggcggggcggggcgaggggcggggcggggcgaggcggagaggtgcggcggcagccaatcagagcggcgcgctccgaaagtttccttttatggcgaggcggcggcggcggcggccctataaaaagcgaagcgcgcggcgggcgggagtcgctgcgtcgcgccttcgccccgtgccccgctccgccgccgcctcgcgccgcccgccccggctctgactgaccgcgttactcccacaggtgagcgggcgggacggcccttctcctccgggctgtaattagcgcttggtttaatgacggctcgtttcttttctgtggctgcgtgaaagccttaaagggctccgggagggccctttgtgcgggggggagcggctcggggggtgcgtgcgtgtgtgtgtgcgtggggagcgccgcgtgcggcccgcgctgcccggcggctgtgagcgctgcgggcgcggcgcggggctttgtgcgctccgcgtgtgcgcgaggggagcgcggccgggggcggtgccccgcggtgcgggggggctgcgaggggaacaaaggctgcgtgcggggtgtgtgcgtgggggggtgagcagggggtgtgggcgcggcggtcgggctgtaacccccccctgcacccccctccccgagttgctgagcacggcccggcttcgggtgcggggctccgtgcggggcgtggcgcggggctcgccgtgccgggcggggggtggcggcaggtgggggtgccgggcggggcggggccgcctcgggccggggagggctcgggggaggggcgcggcggccccggagcgccggcggctgtcgaggcgcggcgagccgcagccattgccttttatggtaatcgtgcgagagggcgcagggacttcctttgtcccaaatctggcggagccgaaatctgggaggcgccgccgcaccccctctagcgggcgcgggcgaagcggtgcggcgccggcaggaaggaaatgggcggggagggccttcgtgcgtcgccgcgccgccgtccccttctccatctccagcctcggggctgccgcagggggacggctgccttcgggggggacggggcagggcggggttcggcttctggcgtgtgaccggcggctctagagcctctgctaaccatgttcatgccttcttctttttcctacagatccttaattaataatacgactcactataggggccgccaccatgacaccacctaagaagaaacggaaggtcgaggacggcgagggccctgctgctaagagagtgaaactggactccggagtgtccaagggcgaagaggacaacatggccagcctgcctgccacccacgagctgcacatcttcggcagcatcaacggcgtggacttcgacatggtgggacagggcaccggcaaccccaacgacggatacgaggaactgaacctgaagtccaccaagggggacctccagttcagcccctggattctggtgccccacatcggctacggcttccaccagtacctgccctaccctgacggcatgagccctttccaggccgctatggtggacggctgcctggaccttaagacccaggtgcagaccccccagggcatgaaggaaatcagcaacatccaagtgggcgacctggtgctgagcaacaccggctacaacgaggtgctgaacgtgttccccaagagcaagaagaagtcctacaagatcaccctggaagatggcaaagagatcatctgctccgaggaacacctgttcccaacccagaccggcgagatgaacatctctggcggcctgaaagagggcatgtgcctgtacgtgaaagaaggcggcggaggacctgaggataagctccaggccattaagtacgagctggcccagaacgaggaagaactggctcagatcgaagagaagctggccgccaacaaagaaggcggatccggcggaggcggatctggaaccggttttgctaatgagctgggccccagactgatgggcaaaggcagcggaggaggcggaagcggacctcctaggaagagatgttgttgcgctagaagaggcacccagctgatgctcgtgggcctgctgtctacagctatgtgggctggactgctggctctgctgctgctttggcattgggagacggaaggtggtggtggatctggtggcggaggctctgaaatcggcacaggcttccctttcgaccctcactacgtggaagtgctgggcgagagaatgcactatgtggatgtgggccctagagatggaacccctgtgctgtttctgcacggcaaccctaccagctcttacgtgtggcggaacatcatccctcacgtggcccctacacacagagtgatcgcccctgatctgatcggcatgggcaagagcgacaagcctgacctgggctacttcttcgacgaccacgtgcggttcatggacgccttcatcgaggctctgggactcgaagaggtggtgctggtcatccacgattggggctctgctctgggcttccactgggccaagagaaaccccgaaagagtgaagggaatcgccttcatggagttcatcagacccattcctacctgggacgagtggcccgagttcgccagagagacattccaggccttcagaacaaccgacgtgggcagaaagctgatcatcgaccagaatgtgtttatcgagggcaccctgcctatgggcgtcgtcagacctctgaccgaggtggaaatggaccactacagagagccttttctgaaccccgtggatagagaacctctgtggcggttccctaacgagctgcctattgctggcgagcccgctaacattgtggccctggtcgaagagtacatggactggctgcatcagagccccgtgcctaagctgctgttttggggaactcccggcgtgctgatccctcctgctgaagctgctagactggctaagagcctgcctaacgctaaggccgtggacatcggacctggcctgaatctgctgcaagaggataaccccgacctgatcggctctgagatcgccagatggctgagcacactggaaatttctggcggtggtggcggtagcggtggcggtggaagcgctcaccactttagcgagcccgagatcaccctgatcatcttcggcgtgatggccctcgtgatcggcaccatcctgctgatctcttacggcatcagacggctgatcaagaagtccccctcaggcggaggcggctctaccggttccggaggcagcggcttctgctacgagaacgaagtcggcagtggcaggtccagattcgtgaagaaggacggccactgcaacgtgcagttcatcaacgtcggaagcggcaagagcagaatcacctctgagggcgagtacatccctctggaccagatcgatattaatgtcggttccggaggaagttcctatacttcaaatagaataggaacttccggcgggtcacccgaggatgagaatgctgctctggaagagaagatcgcccagctgaagcagaagaacgccgctctgaaagaagagatccaggctctggaatacggaggcggaggcatgatgctgaagaagatcctgaagatcgaagaactggacgagcgcgagctgatcgacatcgaggtgtccggcaaccacctgttctacgccaacgatatcctgacccacaactctggctaccaggtgcacagaaccatgcagttcgaggacggcgccagcctgaccgtgaactacagatacacctacgagggcagccacatcaagggcgaggcccaagtgaagggcacaggcttccctgctgacggccccgtgatgaccaactctctgacagccgccgactggtgcagaagcaagaaaacctaccctaacgacaagaccatcatcagcaccttcaagtggtcctacaccacaggcaacggcaagagatacagaagcaccgccagaaccacctacaccttcgccaagcccatggccgccaactacctgaagaaccagcctatgtacgtgttccgaaagaccgagctgaagcacagcaagacagaactgaacttcaaagagtggcagaaagccttcaccgacgtgatgggcatggacgagctgtacaagtccggagctgctccagccgccaagaagaagaagctcgactacaaggacgacgacgataagtgaacgcgtaaatgattgcagatccactagttctagagctcgctgatcagcctcgactgtgccttctagttgccagccatctgttgtttgcccctcccccgtgccttccttgaccctggaaggtgccactcccactgtcctttcctaataaaatgaggaaattgcatcgcattgtctgagtaggtgtcattctattctggggggtggggtggggcaggacagcaagggggaggattgggaagacaatagcaggcatgctggggatgcggtgggctctatggcttctgaggcggaaagaaccagctggggctcgagatccactagttctagcctcgaggctagagcggccgccactggccgtcgttttacaacgtcgtgactgggaaaaccctggcgttacccaacttaatcgccttgcagcacatccccctttcgccagctggcgtaatagcgaagaggcccgcaccgatcgcccttcccaacagttgcgcagcctgaatggcgaatgggacgcgccctgtagcggcgcattaagcgcggcgggtgtggtggttacgcgcagcgtgaccgctacacttgccagcgccctagcgcccgctcctttcgctttcttcccttcctttctcgccacgttcgccggctttccccgtcaagctctaaatcgggggctccctttagggttccgatttagtgctttacggcacctcgaccccaaaaaacttgattagggtgatggttcacgtagtgggccatcgccctgatagacggtttttcgccctttgacgttggagtccacgttctttaatagtggactcttgttccaaactggaacaacactcaaccctatctcggtctattcttttgatttataagggattttgccgatttcggcctattggttaaaaaatgagctgatttaacaaaaatttaacgcgaattttaacaaaatattaacgcttacaatttaggtggcacttttcggggaaatgtgcgcggaacccctatttgtttatttttctaaatacattcaaatatgtatccgctcatgagacaataaccctgataaatgcttcaataatattgaaaaaggaagagtatgagtattcaacatttccgtgtcgcccttattcccttttttgcggcattttgccttcctgtttttgctcacccagaaacgctggtgaaagtaaaagatgctgaagatcagttgggtgcacgagtgggttacatcgaactggatctcaacagcggtaagatccttgagagttttcgccccgaagaacgttttccaatgatgagcacttttaaagttctgctatgtggcgcggtattatcccgtattgacgccgggcaagagcaactcggtcgccgcatacactattctcagaatgacttggttgagtactcaccagtcacagaaaagcatcttacggatggcatgacagtaagagaattatgcagtgctgccataaccatgagtgataacactgcggccaacttacttctgacaacgatcggaggaccgaaggagctaaccgcttttttgcacaacatgggggatcatgtaactcgccttgatcgttgggaaccggagctgaatgaagccataccaaacgacgagcgtgacaccacgatgcctgtagcaatggcaacaacgttgcgcaaactattaactggcgaactacttactctagcttcccggcaacaattaatagactggatggaggcggataaagttgcaggaccacttctgcgctcggcccttccggctggctggtttattgctgataaatctggagccggtgagcgtgggtctcgcggtatcattgcagcactggggccagatggtaagccctcccgtatcgtagttatctacacgacggggagtcaggcaactatggatgaacgaaatagacagatcgctgagataggtgcctcactgattaagcattggtaactgtcagaccaagtttactcatatatactttagattgatttaaaacttcatttttaatttaaaaggatctaggtgaagatcctttttgataatctcatgaccaaaatcccttaacgtgagttttcgttccactgagcgtcagaccccgtagaaaagatcaaaggatcttcttgagatcctttttttctgcgcgtaatctgctgcttgcaaacaaaaaaaccaccgctaccagcggtggtttgtttgccggatcaagagctaccaactctttttccgaaggtaactggcttcagcagagcgcagataccaaatactgtccttctagtgtagccgtagttaggccaccacttcaagaactctgtagcaccgcctacatacctcgctctgctaatcctgttaccagtggctgctgccagtggcgataagtcgtgtcttaccgggttggactcaagacgatagttaccggataaggcgcagcggtcgggctgaacggggggttcgtgcacacagcccagcttggagcgaacgacctacaccgaactgagatacctacagcgtgagctatgagaaagcgccacgcttcccgaagggagaaaggcggacaggtatccggtaagcggcagggtcggaacaggagagcgcacgagggagcttccagggggaaacgcctggtatctttatagtcctgtcgggtttcgccacctctgacttgagcgtcgatttttgtgatgctcgtcaggggggcggagcctatggaaaaacgccagcaacgcggcctttttacggttcctggccttttgctggccttttgctcacatgttctttcctgcgttatcccctgattctgtggataaccgtattaccgcctttgagtgagctgataccgctcgccgcagccgaacgaccgagcgcagcgagtcagtgagcgaggaagcggaagagcgcccaatacgcaaaccgcctctccccgcgcgttggccgattcattaatgcagctggcacgacaggtttcccgactggaaagcgggcagtgagcgcaacgcaattaatgtgagttagctcactcattaggcaccccaggctttacactttatgcttccggctcgtatgttgtgtggaattgtgagcggataacaatttcacacaggaaacagctatgaccatga

SEQ ID NO: 58 - DNA, 7444 bp, Artificial
  Vector comprising split intein - heterologous polynucleotide construct
ggcgcgccggattcgacattgattattgactagttattaatagtaatcaattacggggtcattagttcatagcccatatatggagttccgcgttacataacttacggtaaatggcccgcctggctgaccgcccaacgacccccgcccattgacgtcaataatgacgtatgttcccatagtaacgccaatagggactttccattgacgtcaatgggtggagtatttacggtaaactgcccacttggcagtacatcaagtgtatcatatgccaagtacgccccctattgacgtcaatgacggtaaatggcccgcctggcattatgcccagtacatgaccttatgggactttcctacttggcagtacatctacgtattagtcatcgctattaccatggtcgaggtgagccccacgttctgcttcactctccccatctcccccccctccccacccccaattttgtatttatttattttttaattattttgtgcagcgatgggggcggggggggggggggggcgcgcgccaggcggggcggggcggggcgaggggcggggcggggcgaggcggagaggtgcggcggcagccaatcagagcggcgcgctccgaaagtttccttttatggcgaggcggcggcggcggcggccctataaaaagcgaagcgcgcggcgggcgggagtcgctgcgtcgcgccttcgccccgtgccccgctccgccgccgcctcgcgccgcccgccccggctctgactgaccgcgttactcccacaggtgagcgggcgggacggcccttctcctccgggctgtaattagcgcttggtttaatgacggctcgtttcttttctgtggctgcgtgaaagccttaaagggctccgggagggccctttgtgcgggggggagcggctcggggggtgcgtgcgtgtgtgtgtgcgtggggagcgccgcgtgcggcccgcgctgcccggcggctgtgagcgctgcgggcgcggcgcggggctttgtgcgctccgcgtgtgcgcgaggggagcgcggccgggggcggtgccccgcggtgcgggggggctgcgaggggaacaaaggctgcgtgcggggtgtgtgcgtgggggggtgagcagggggtgtgggcgcggcggtcgggctgtaacccccccctgcacccccctccccgagttgctgagcacggcccggcttcgggtgcggggctccgtgcggggcgtggcgcggggctcgccgtgccgggcggggggtggcggcaggtgggggtgccgggcggggcggggccgcctcgggccggggagggctcgggggaggggcgcggcggccccggagcgccggcggctgtcgaggcgcggcgagccgcagccattgccttttatggtaatcgtgcgagagggcgcagggacttcctttgtcccaaatctggcggagccgaaatctgggaggcgccgccgcaccccctctagcgggcgcgggcgaagcggtgcggcgccggcaggaaggaaatgggcggggagggccttcgtgcgtcgccgcgccgccgtccccttctccatctccagcctcggggctgccgcagggggacggctgccttcgggggggacggggcagggcggggttcggcttctggcgtgtgaccggcggctctagagcctctgctaaccatgttcatgccttcttctttttcctacagatccttaattaataatacgactcactataggggccgccaccatgacaccacctaagaagaaacggaaggtcgaggacggcgagggccctgctgctaagagagtgaaactggactccggagtgtccaagggcgaagaggacaacatggccagcctgcctgccacccacgagctgcacatcttcggcagcatcaacggcgtggacttcgacatggtgggacagggcaccggcaaccccaacgacggatacgaggaactgaacctgaagtccaccaagggggacctccagttcagcccctggattctggtgccccacatcggctacggcttccaccagtacctgccctaccctgacggcatgagccctttccaggccgctatggtggacggctgcctggaccttaagacccaggtgcagaccccccagggcatgaaggaaatcagcaacatccaagtgggcgacctggtgctgagcaacaccggctacaacgaggtgctgaacgtgttccccaagagcaagaagaagtcctacaagatcaccctggaagatggcaaagagatcatctgctccgaggaacacctgttcccaacccagaccggcgagatgaacatctctggcggcctgaaagagggcatgtgcctgtacgtgaaagaaggcggcggaggacctgaggataagctccaggccattaagtacgagctggcccagaacgaggaagaactggctcagatcgaagagaagctggccgccaacaaagaaggcggatccggcggaggcggatctggaaccggttttgctaatgagctgggccccagactgatgggcaaaggcagcggaggaggcggaagcggacctcctaggaagagatgttgttgcgctagaagaggcacccagctgatgctcgtgggcctgctgtctacagctatgtgggctggactgctggctctgctgctgctttggcattgggagacggaaggtggtggtggatctggtaccggaagcggagtctttacactggaagatttcgtcggcgactggcggcagacagctggctacaatctggaccaggtgctggaacaaggcggcgtgtcctctctgtttcagaacctgggagtgtctgtgacccctatccagagaatcgtgctgagcggcgagaacggcctgaagatcgacatccacgtgatcatcccttacgagggcctgtccggcgatcagatgggacagatcgagaagatctttaaggtggtgtaccccgtggacgaccaccacttcaaagtgatcctgcactacggcaccctggtcatcgatggcgtgaccccaaacatgatcgactacttcggcagaccctacgagggaatcgccgtgttcgacggcaagaaaatcaccgtgaccggcacactgtggaacggcaacaagatcatcgacgagagactgatcaaccccgacggcagcctgctgttcagagtgacaatcaacggcgtgacaggctggcggctgtgcgaaagaatccttgctggtaccgactacaaggacgacgacgacaaaggaggtggcggtggaagcgctcaccactttagcgagcccgagatcaccctgatcatcttcggcgtgatggccctcgtgatcggcaccatcctgctgatctcttacggcatcagacggctgatcaagaagtccccctcaggcggaggcggctctaccggttccggaggcagcggcttctgctacgagaacgaagtcggcagtggcaggtccagattcgtgaagaaggacggccactgcaacgtgcagttcatcaacgtcggaagcggcaagagcagaatcacctctgagggcgagtacatccctctggaccagatcgatattaatgtcggttccggaggaagttcctatacttcaaatagaataggaacttccggcgggtcacccgaggatgagaatgctgctctggaagagaagatcgcccagctgaagcagaagaacgccgctctgaaagaagagatccaggctctggaatacggaggcggaggcatgatgctgaagaagatcctgaagatcgaagaactggacgagcgcgagctgatcgacatcgaggtgtccggcaaccacctgttctacgccaacgatatcctgacccacaactctggctaccaggtgcacagaaccatgcagttcgaggacggcgccagcctgaccgtgaactacagatacacctacgagggcagccacatcaagggcgaggcccaagtgaagggcacaggcttccctgctgacggccccgtgatgaccaactctctgacagccgccgactggtgcagaagcaagaaaacctaccctaacgacaagaccatcatcagcaccttcaagtggtcctacaccacaggcaacggcaagagatacagaagcaccgccagaaccacctacaccttcgccaagcccatggccgccaactacctgaagaaccagcctatgtacgtgttccgaaagaccgagctgaagcacagcaagacagaactgaacttcaaagagtggcagaaagccttcaccgacgtgatgggcatggacgagctgtacaagtccggagctgctccagccgccaagaagaagaagctcgactacaaggacgacgacgataagtgaacgcgtaaatgattgcagatccactagttctagagctcgctgatcagcctcgactgtgccttctagttgccagccatctgttgtttgcccctcccccgtgccttccttgaccctggaaggtgccactcccactgtcctttcctaataaaatgaggaaattgcatcgcattgtctgagtaggtgtcattctattctggggggtggggtggggcaggacagcaagggggaggattgggaagacaatagcaggcatgctggggatgcggtgggctctatggcttctgaggcggaaagaaccagctggggctcgagatccactagttctagcctcgaggctagagcggccgccactggccgtcgttttacaacgtcgtgactgggaaaaccctggcgttacccaacttaatcgccttgcagcacatccccctttcgccagctggcgtaatagcgaagaggcccgcaccgatcgcccttcccaacagttgcgcagcctgaatggcgaatgggacgcgccctgtagcggcgcattaagcgcggcgggtgtggtggttacgcgcagcgtgaccgctacacttgccagcgccctagcgcccgctcctttcgctttcttcccttcctttctcgccacgttcgccggctttccccgtcaagctctaaatcgggggctccctttagggttccgatttagtgctttacggcacctcgaccccaaaaaacttgattagggtgatggttcacgtagtgggccatcgccctgatagacggtttttcgccctttgacgttggagtccacgttctttaatagtggactcttgttccaaactggaacaacactcaaccctatctcggtctattcttttgatttataagggattttgccgatttcggcctattggttaaaaaatgagctgatttaacaaaaatttaacgcgaattttaacaaaatattaacgcttacaatttaggtggcacttttcggggaaatgtgcgcggaacccctatttgtttatttttctaaatacattcaaatatgtatccgctcatgagacaataaccctgataaatgcttcaataatattgaaaaaggaagagtatgagtattcaacatttccgtgtcgcccttattcccttttttgcggcattttgccttcctgtttttgctcacccagaaacgctggtgaaagtaaaagatgctgaagatcagttgggtgcacgagtgggttacatcgaactggatctcaacagcggtaagatccttgagagttttcgccccgaagaacgttttccaatgatgagcacttttaaagttctgctatgtggcgcggtattatcccgtattgacgccgggcaagagcaactcggtcgccgcatacactattctcagaatgacttggttgagtactcaccagtcacagaaaagcatcttacggatggcatgacagtaagagaattatgcagtgctgccataaccatgagtgataacactgcggccaacttacttctgacaacgatcggaggaccgaaggagctaaccgcttttttgcacaacatgggggatcatgtaactcgccttgatcgttgggaaccggagctgaatgaagccataccaaacgacgagcgtgacaccacgatgcctgtagcaatggcaacaacgttgcgcaaactattaactggcgaactacttactctagcttcccggcaacaattaatagactggatggaggcggataaagttgcaggaccacttctgcgctcggcccttccggctggctggtttattgctgataaatctggagccggtgagcgtgggtctcgcggtatcattgcagcactggggccagatggtaagccctcccgtatcgtagttatctacacgacggggagtcaggcaactatggatgaacgaaatagacagatcgctgagataggtgcctcactgattaagcattggtaactgtcagaccaagtttactcatatatactttagattgatttaaaacttcatttttaatttaaaaggatctaggtgaagatcctttttgataatctcatgaccaaaatcccttaacgtgagttttcgttccactgagcgtcagaccccgtagaaaagatcaaaggatcttcttgagatcctttttttctgcgcgtaatctgctgcttgcaaacaaaaaaaccaccgctaccagcggtggtttgtttgccggatcaagagctaccaactctttttccgaaggtaactggcttcagcagagcgcagataccaaatactgtccttctagtgtagccgtagttaggccaccacttcaagaactctgtagcaccgcctacatacctcgctctgctaatcctgttaccagtggctgctgccagtggcgataagtcgtgtcttaccgggttggactcaagacgatagttaccggataaggcgcagcggtcgggctgaacggggggttcgtgcacacagcccagcttggagcgaacgacctacaccgaactgagatacctacagcgtgagctatgagaaagcgccacgcttcccgaagggagaaaggcggacaggtatccggtaagcggcagggtcggaacaggagagcgcacgagggagcttccagggggaaacgcctggtatctttatagtcctgtcgggtttcgccacctctgacttgagcgtcgatttttgtgatgctcgtcaggggggcggagcctatggaaaaacgccagcaacgcggcctttttacggttcctggccttttgctggccttttgctcacatgttctttcctgcgttatcccctgattctgtggataaccgtattaccgcctttgagtgagctgataccgctcgccgcagccgaacgaccgagcgcagcgagtcagtgagcgaggaagcggaagagcgcccaatacgcaaaccgcctctccccgcgcgttggccgattcattaatgcagctggcacgacaggtttcccgactggaaagcgggcagtgagcgcaacgcaattaatgtgagttagctcactcattaggcaccccaggctttacactttatgcttccggctcgtatgttgtgtggaattgtgagcggataacaatttcacacaggaaacagctatgaccatga

SEQ ID NO: 59 - DNA, 7504 bp, Artificial
  Vector comprising split intein - heterologous polynucleotide construct
ggcgcgccggattcgacattgattattgactagttattaatagtaatcaattacggggtcattagttcatagcccatatatggagttccgcgttacataacttacggtaaatggcccgcctggctgaccgcccaacgacccccgcccattgacgtcaataatgacgtatgttcccatagtaacgccaatagggactttccattgacgtcaatgggtggagtatttacggtaaactgcccacttggcagtacatcaagtgtatcatatgccaagtacgccccctattgacgtcaatgacggtaaatggcccgcctggcattatgcccagtacatgaccttatgggactttcctacttggcagtacatctacgtattagtcatcgctattaccatggtcgaggtgagccccacgttctgcttcactctccccatctcccccccctccccacccccaattttgtatttatttattttttaattattttgtgcagcgatgggggcggggggggggggggggcgcgcgccaggcggggcggggcggggcgaggggcggggcggggcgaggcggagaggtgcggcggcagccaatcagagcggcgcgctccgaaagtttccttttatggcgaggcggcggcggcggcggccctataaaaagcgaagcgcgcggcgggcgggagtcgctgcgtcgcgccttcgccccgtgccccgctccgccgccgcctcgcgccgcccgccccggctctgactgaccgcgttactcccacaggtgagcgggcgggacggcccttctcctccgggctgtaattagcgcttggtttaatgacggctcgtttcttttctgtggctgcgtgaaagccttaaagggctccgggagggccctttgtgcgggggggagcggctcggggggtgcgtgcgtgtgtgtgtgcgtggggagcgccgcgtgcggcccgcgctgcccggcggctgtgagcgctgcgggcgcggcgcggggctttgtgcgctccgcgtgtgcgcgaggggagcgcggccgggggcggtgccccgcggtgcgggggggctgcgaggggaacaaaggctgcgtgcggggtgtgtgcgtgggggggtgagcagggggtgtgggcgcggcggtcgggctgtaacccccccctgcacccccctccccgagttgctgagcacggcccggcttcgggtgcggggctccgtgcggggcgtggcgcggggctcgccgtgccgggcggggggtggcggcaggtgggggtgccgggcggggcggggccgcctcgggccggggagggctcgggggaggggcgcggcggccccggagcgccggcggctgtcgaggcgcggcgagccgcagccattgccttttatggtaatcgtgcgagagggcgcagggacttcctttgtcccaaatctggcggagccgaaatctgggaggcgccgccgcaccccctctagcgggcgcgggcgaagcggtgcggcgccggcaggaaggaaatgggcggggagggccttcgtgcgtcgccgcgccgccgtccccttctccatctccagcctcggggctgccgcagggggacggctgccttcgggggggacggggcagggcggggttcggcttctggcgtgtgaccggcggctctagagcctctgctaaccatgttcatgccttcttctttttcctacagatccttaattaataatacgactcactataggggccgccaccatgacaccacctaagaagaaacggaaggtcgaggacggcgagggccctgctgctaagagagtgaaactggactccggagtgtccaagggcgaagaggacaacatggccagcctgcctgccacccacgagctgcacatcttcggcagcatcaacggcgtggacttcgacatggtgggacagggcaccggcaaccccaacgacggatacgaggaactgaacctgaagtccaccaagggggacctccagttcagcccctggattctggtgccccacatcggctacggcttccaccagtacctgccctaccctgacggcatgagccctttccaggccgctatggtggacggctgcctggaccttaagacccaggtgcagaccccccagggcatgaaggaaatcagcaacatccaagtgggcgacctggtgctgagcaacaccggctacaacgaggtgctgaacgtgttccccaagagcaagaagaagtcctacaagatcaccctggaagatggcaaagagatcatctgctccgaggaacacctgttcccaacccagaccggcgagatgaacatctctggcggcctgaaagagggcatgtgcctgtacgtgaaagaaggcggcggaggacctgaggataagctccaggccattaagtacgagctggcccagaacgaggaagaactggctcagatcgaagagaagctggccgccaacaaagaaggcggatccggcggaggcggatctggaaccggttttgctaatgagctgggccccagactgatgggcaaaggcagcggaggaggcggaagcggacctcctaggaagagatgttgttgcgctagaagaggcacccagctgatgctcgtgggcctgctgtctacagctatgtgggctggactgctggctctgctgctgctttggcattgggagacggaaggtggtggtggatctcgccgcagaagaagaaagagaagcgccagaggtaccggaagcggagtctttacactggaagatttcgtcggcgactggcggcagacagctggctacaatctggaccaggtgctggaacaaggcggcgtgtcctctctgtttcagaacctgggagtgtctgtgacccctatccagagaatcgtgctgagcggcgagaacggcctgaagatcgacatccacgtgatcatcccttacgagggcctgtccggcgatcagatgggacagatcgagaagatctttaaggtggtgtaccccgtggacgaccaccacttcaaagtgatcctgcactacggcaccctggtcatcgatggcgtgaccccaaacatgatcgactacttcggcagaccctacgagggaatcgccgtgttcgacggcaagaaaatcaccgtgaccggcacactgtggaacggcaacaagatcatcgacgagagactgatcaaccccgacggcagcctgctgttcagagtgacaatcaacggcgtgacaggctggcggctgtgcgaaagaatccttgctggtaccgactacaaggacgacgacgacaaaggacgcaggcggagaagaaaaagatccgctcgcggtggcggtggaagcgctcaccactttagcgagcccgagatcaccctgatcatcttcggcgtgatggccctcgtgatcggcaccatcctgctgatctcttacggcatcagacggctgatcaagaagtccccctcaggcggaggcggctctaccggttccggaggcagcggcttctgctacgagaacgaagtcggcagtggcaggtccagattcgtgaagaaggacggccactgcaacgtgcagttcatcaacgtcggaagcggcaagagcagaatcacctctgagggcgagtacatccctctggaccagatcgatattaatgtcggttccggaggaagttcctatacttcaaatagaataggaacttccggcgggtcacccgaggatgagaatgctgctctggaagagaagatcgcccagctgaagcagaagaacgccgctctgaaagaagagatccaggctctggaatacggaggcggaggcatgatgctgaagaagatcctgaagatcgaagaactggacgagcgcgagctgatcgacatcgaggtgtccggcaaccacctgttctacgccaacgatatcctgacccacaactctggctaccaggtgcacagaaccatgcagttcgaggacggcgccagcctgaccgtgaactacagatacacctacgagggcagccacatcaagggcgaggcccaagtgaagggcacaggcttccctgctgacggccccgtgatgaccaactctctgacagccgccgactggtgcagaagcaagaaaacctaccctaacgacaagaccatcatcagcaccttcaagtggtcctacaccacaggcaacggcaagagatacagaagcaccgccagaaccacctacaccttcgccaagcccatggccgccaactacctgaagaaccagcctatgtacgtgttccgaaagaccgagctgaagcacagcaagacagaactgaacttcaaagagtggcagaaagccttcaccgacgtgatgggcatggacgagctgtacaagtccggagctgctccagccgccaagaagaagaagctcgactacaaggacgacgacgataagtgaacgcgtaaatgattgcagatccactagttctagagctcgctgatcagcctcgactgtgccttctagttgccagccatctgttgtttgcccctcccccgtgccttccttgaccctggaaggtgccactcccactgtcctttcctaataaaatgaggaaattgcatcgcattgtctgagtaggtgtcattctattctggggggtggggtggggcaggacagcaagggggaggattgggaagacaatagcaggcatgctggggatgcggtgggctctatggcttctgaggcggaaagaaccagctggggctcgagatccactagttctagcctcgaggctagagcggccgccactggccgtcgttttacaacgtcgtgactgggaaaaccctggcgttacccaacttaatcgccttgcagcacatccccctttcgccagctggcgtaatagcgaagaggcccgcaccgatcgcccttcccaacagttgcgcagcctgaatggcgaatgggacgcgccctgtagcggcgcattaagcgcggcgggtgtggtggttacgcgcagcgtgaccgctacacttgccagcgccctagcgcccgctcctttcgctttcttcccttcctttctcgccacgttcgccggctttccccgtcaagctctaaatcgggggctccctttagggttccgatttagtgctttacggcacctcgaccccaaaaaacttgattagggtgatggttcacgtagtgggccatcgccctgatagacggtttttcgccctttgacgttggagtccacgttctttaatagtggactcttgttccaaactggaacaacactcaaccctatctcggtctattcttttgatttataagggattttgccgatttcggcctattggttaaaaaatgagctgatttaacaaaaatttaacgcgaattttaacaaaatattaacgcttacaatttaggtggcacttttcggggaaatgtgcgcggaacccctatttgtttatttttctaaatacattcaaatatgtatccgctcatgagacaataaccctgataaatgcttcaataatattgaaaaaggaagagtatgagtattcaacatttccgtgtcgcccttattcccttttttgcggcattttgccttcctgtttttgctcacccagaaacgctggtgaaagtaaaagatgctgaagatcagttgggtgcacgagtgggttacatcgaactggatctcaacagcggtaagatccttgagagttttcgccccgaagaacgttttccaatgatgagcacttttaaagttctgctatgtggcgcggtattatcccgtattgacgccgggcaagagcaactcggtcgccgcatacactattctcagaatgacttggttgagtactcaccagtcacagaaaagcatcttacggatggcatgacagtaagagaattatgcagtgctgccataaccatgagtgataacactgcggccaacttacttctgacaacgatcggaggaccgaaggagctaaccgcttttttgcacaacatgggggatcatgtaactcgccttgatcgttgggaaccggagctgaatgaagccataccaaacgacgagcgtgacaccacgatgcctgtagcaatggcaacaacgttgcgcaaactattaactggcgaactacttactctagcttcccggcaacaattaatagactggatggaggcggataaagttgcaggaccacttctgcgctcggcccttccggctggctggtttattgctgataaatctggagccggtgagcgtgggtctcgcggtatcattgcagcactggggccagatggtaagccctcccgtatcgtagttatctacacgacggggagtcaggcaactatggatgaacgaaatagacagatcgctgagataggtgcctcactgattaagcattggtaactgtcagaccaagtttactcatatatactttagattgatttaaaacttcatttttaatttaaaaggatctaggtgaagatcctttttgataatctcatgaccaaaatcccttaacgtgagttttcgttccactgagcgtcagaccccgtagaaaagatcaaaggatcttcttgagatcctttttttctgcgcgtaatctgctgcttgcaaacaaaaaaaccaccgctaccagcggtggtttgtttgccggatcaagagctaccaactctttttccgaaggtaactggcttcagcagagcgcagataccaaatactgtccttctagtgtagccgtagttaggccaccacttcaagaactctgtagcaccgcctacatacctcgctctgctaatcctgttaccagtggctgctgccagtggcgataagtcgtgtcttaccgggttggactcaagacgatagttaccggataaggcgcagcggtcgggctgaacggggggttcgtgcacacagcccagcttggagcgaacgacctacaccgaactgagatacctacagcgtgagctatgagaaagcgccacgcttcccgaagggagaaaggcggacaggtatccggtaagcggcagggtcggaacaggagagcgcacgagggagcttccagggggaaacgcctggtatctttatagtcctgtcgggtttcgccacctctgacttgagcgtcgatttttgtgatgctcgtcaggggggcggagcctatggaaaaacgccagcaacgcggcctttttacggttcctggccttttgctggccttttgctcacatgttctttcctgcgttatcccctgattctgtggataaccgtattaccgcctttgagtgagctgataccgctcgccgcagccgaacgaccgagcgcagcgagtcagtgagcgaggaagcggaagagcgcccaatacgcaaaccgcctctccccgcgcgttggccgattcattaatgcagctggcacgacaggtttcccgactggaaagcgggcagtgagcgcaacgcaattaatgtgagttagctcactcattaggcaccccaggctttacactttatgcttccggctcgtatgttgtgtggaattgtgagcggataacaatttcacacaggaaacagctatgaccatga

SEQ ID NO: 60 - DNA, 6748 bp, Artificial
  Vector comprising split intein - heterologous polynucleotide construct
ggcgcgccggattcgacattgattattgactagttattaatagtaatcaattacggggtcattagttcatagcccatatatggagttccgcgttacataacttacggtaaatggcccgcctggctgaccgcccaacgacccccgcccattgacgtcaataatgacgtatgttcccatagtaacgccaatagggactttccattgacgtcaatgggtggagtatttacggtaaactgcccacttggcagtacatcaagtgtatcatatgccaagtacgccccctattgacgtcaatgacggtaaatggcccgcctggcattatgcccagtacatgaccttatgggactttcctacttggcagtacatctacgtattagtcatcgctattaccatggtcgaggtgagccccacgttctgcttcactctccccatctcccccccctccccacccccaattttgtatttatttattttttaattattttgtgcagcgatgggggcggggggggggggggggcgcgcgccaggcggggcggggcggggcgaggggcggggcggggcgaggcggagaggtgcggcggcagccaatcagagcggcgcgctccgaaagtttccttttatggcgaggcggcggcggcggcggccctataaaaagcgaagcgcgcggcgggcgggagtcgctgcgtcgcgccttcgccccgtgccccgctccgccgccgcctcgcgccgcccgccccggctctgactgaccgcgttactcccacaggtgagcgggcgggacggcccttctcctccgggctgtaattagcgcttggtttaatgacggctcgtttcttttctgtggctgcgtgaaagccttaaagggctccgggagggccctttgtgcgggggggagcggctcggggggtgcgtgcgtgtgtgtgtgcgtggggagcgccgcgtgcggcccgcgctgcccggcggctgtgagcgctgcgggcgcggcgcggggctttgtgcgctccgcgtgtgcgcgaggggagcgcggccgggggcggtgccccgcggtgcgggggggctgcgaggggaacaaaggctgcgtgcggggtgtgtgcgtgggggggtgagcagggggtgtgggcgcggcggtcgggctgtaacccccccctgcacccccctccccgagttgctgagcacggcccggcttcgggtgcggggctccgtgcggggcgtggcgcggggctcgccgtgccgggcggggggtggcggcaggtgggggtgccgggcggggcggggccgcctcgggccggggagggctcgggggaggggcgcggcggccccggagcgccggcggctgtcgaggcgcggcgagccgcagccattgccttttatggtaatcgtgcgagagggcgcagggacttcctttgtcccaaatctggcggagccgaaatctgggaggcgccgccgcaccccctctagcgggcgcgggcgaagcggtgcggcgccggcaggaaggaaatgggcggggagggccttcgtgcgtcgccgcgccgccgtccccttctccatctccagcctcggggctgccgcagggggacggctgccttcgggggggacggggcagggcggggttcggcttctggcgtgtgaccggcggctctagagcctctgctaaccatgttcatgccttcttctttttcctacagatccttaattaataatacgactcactataggggccgccaccatgacaccacctaagaagaaacggaaggtcgaggacggcgagggccctgctgctaagagagtgaaactggactccggagtgtccaagggcgaagaggacaacatggccagcctgcctgccacccacgagctgcacatcttcggcagcatcaacggcgtggacttcgacatggtgggacagggcaccggcaaccccaacgacggatacgaggaactgaacctgaagtccaccaagggggacctccagttcagcccctggattctggtgccccacatcggctacggcttccaccagtacctgccctaccctgacggcatgagccctttccaggccgctatggtggacggctgcctggaccttaagacccaggtgcagaccccccagggcatgaaggaaatcagcaacatccaagtgggcgacctggtgctgagcaacaccggctacaacgaggtgctgaacgtgttccccaagagcaagaagaagtcctacaagatcaccctggaagatggcaaagagatcatctgctccgaggaacacctgttcccaacccagaccggcgagatgaacatctctggcggcctgaaagagggcatgtgcctgtacgtgaaagaaggcggcggaggaggcggatccggcggaggcggatctggaaccggttttgctaatgagctgggccccagactgatgggcaaaggcagcggaggaggcggaagcggagtctttacactggaagatttcgtcggcgactggcggcagacagctggctacaatctggaccaggtgctggaacaaggcggcgtgtcctctctgtttcagaacctgggagtgtctgtgacccctatccagagaatcgtgctgagcggcgagaacggcctgaagatcgacatccacgtgatcatcccttacgagggcctgtccggcgatcagatgggacagatcgagaagatctttaaggtggtgtaccccgtggacgaccaccacttcaaagtgatcctgcactacggcaccctggtcatcgatggcgtgaccccaaacatgatcgactacttcggcagaccctacgagggaatcgccgtgttcgacggcaagaaaatcaccgtgaccggcacactgtggaacggcaacaagatcatcgacgagagactgatcaaccccgacggcagcctgctgttcagagtgacaatcaacggcgtgacaggctggcggctgtgcgaaagaatccttgctggttccggaggaagttcctatacttcaaatagaataggaacttccggcgggtcaggaggcggaggcatgatgctgaagaagatcctgaagatcgaagaactggacgagcgcgagctgatcgacatcgaggtgtccggcaaccacctgttctacgccaacgatatcctgacccacaactctggctaccaggtgcacagaaccatgcagttcgaggacggcgccagcctgaccgtgaactacagatacacctacgagggcagccacatcaagggcgaggcccaagtgaagggcacaggcttccctgctgacggccccgtgatgaccaactctctgacagccgccgactggtgcagaagcaagaaaacctaccctaacgacaagaccatcatcagcaccttcaagtggtcctacaccacaggcaacggcaagagatacagaagcaccgccagaaccacctacaccttcgccaagcccatggccgccaactacctgaagaaccagcctatgtacgtgttccgaaagaccgagctgaagcacagcaagacagaactgaacttcaaagagtggcagaaagccttcaccgacgtgatgggcatggacgagctgtacaagtccggagctgctccagccgccaagaagaagaagctcgactacaaggacgacgacgataagtgaacgcgtaaatgattgcagatccactagttctagagctcgctgatcagcctcgactgtgccttctagttgccagccatctgttgtttgcccctcccccgtgccttccttgaccctggaaggtgccactcccactgtcctttcctaataaaatgaggaaattgcatcgcattgtctgagtaggtgtcattctattctggggggtggggtggggcaggacagcaagggggaggattgggaagacaatagcaggcatgctggggatgcggtgggctctatggcttctgaggcggaaagaaccagctggggctcgagatccactagttctagcctcgaggctagagcggccgccactggccgtcgttttacaacgtcgtgactgggaaaaccctggcgttacccaacttaatcgccttgcagcacatccccctttcgccagctggcgtaatagcgaagaggcccgcaccgatcgcccttcccaacagttgcgcagcctgaatggcgaatgggacgcgccctgtagcggcgcattaagcgcggcgggtgtggtggttacgcgcagcgtgaccgctacacttgccagcgccctagcgcccgctcctttcgctttcttcccttcctttctcgccacgttcgccggctttccccgtcaagctctaaatcgggggctccctttagggttccgatttagtgctttacggcacctcgaccccaaaaaacttgattagggtgatggttcacgtagtgggccatcgccctgatagacggtttttcgccctttgacgttggagtccacgttctttaatagtggactcttgttccaaactggaacaacactcaaccctatctcggtctattcttttgatttataagggattttgccgatttcggcctattggttaaaaaatgagctgatttaacaaaaatttaacgcgaattttaacaaaatattaacgcttacaatttaggtggcacttttcggggaaatgtgcgcggaacccctatttgtttatttttctaaatacattcaaatatgtatccgctcatgagacaataaccctgataaatgcttcaataatattgaaaaaggaagagtatgagtattcaacatttccgtgtcgcccttattcccttttttgcggcattttgccttcctgtttttgctcacccagaaacgctggtgaaagtaaaagatgctgaagatcagttgggtgcacgagtgggttacatcgaactggatctcaacagcggtaagatccttgagagttttcgccccgaagaacgttttccaatgatgagcacttttaaagttctgctatgtggcgcggtattatcccgtattgacgccgggcaagagcaactcggtcgccgcatacactattctcagaatgacttggttgagtactcaccagtcacagaaaagcatcttacggatggcatgacagtaagagaattatgcagtgctgccataaccatgagtgataacactgcggccaacttacttctgacaacgatcggaggaccgaaggagctaaccgcttttttgcacaacatgggggatcatgtaactcgccttgatcgttgggaaccggagctgaatgaagccataccaaacgacgagcgtgacaccacgatgcctgtagcaatggcaacaacgttgcgcaaactattaactggcgaactacttactctagcttcccggcaacaattaatagactggatggaggcggataaagttgcaggaccacttctgcgctcggcccttccggctggctggtttattgctgataaatctggagccggtgagcgtgggtctcgcggtatcattgcagcactggggccagatggtaagccctcccgtatcgtagttatctacacgacggggagtcaggcaactatggatgaacgaaatagacagatcgctgagataggtgcctcactgattaagcattggtaactgtcagaccaagtttactcatatatactttagattgatttaaaacttcatttttaatttaaaaggatctaggtgaagatcctttttgataatctcatgaccaaaatcccttaacgtgagttttcgttccactgagcgtcagaccccgtagaaaagatcaaaggatcttcttgagatcctttttttctgcgcgtaatctgctgcttgcaaacaaaaaaaccaccgctaccagcggtggtttgtttgccggatcaagagctaccaactctttttccgaaggtaactggcttcagcagagcgcagataccaaatactgtccttctagtgtagccgtagttaggccaccacttcaagaactctgtagcaccgcctacatacctcgctctgctaatcctgttaccagtggctgctgccagtggcgataagtcgtgtcttaccgggttggactcaagacgatagttaccggataaggcgcagcggtcgggctgaacggggggttcgtgcacacagcccagcttggagcgaacgacctacaccgaactgagatacctacagcgtgagctatgagaaagcgccacgcttcccgaagggagaaaggcggacaggtatccggtaagcggcagggtcggaacaggagagcgcacgagggagcttccagggggaaacgcctggtatctttatagtcctgtcgggtttcgccacctctgacttgagcgtcgatttttgtgatgctcgtcaggggggcggagcctatggaaaaacgccagcaacgcggcctttttacggttcctggccttttgctggccttttgctcacatgttctttcctgcgttatcccctgattctgtggataaccgtattaccgcctttgagtgagctgataccgctcgccgcagccgaacgaccgagcgcagcgagtcagtgagcgaggaagcggaagagcgcccaatacgcaaaccgcctctccccgcgcgttggccgattcattaatgcagctggcacgacaggtttcccgactggaaagcgggcagtgagcgcaacgcaattaatgtgagttagctcactcattaggcaccccaggctttacactttatgcttccggctcgtatgttgtgtggaattgtgagcggataacaatttcacacaggaaacagctatgaccatga

SEQ ID NO: 61 - DNA, 6934 bp, Artificial
  Vector comprising split intein - heterologous polynucleotide construct
ggcgcgccggattcgacattgattattgactagttattaatagtaatcaattacggggtcattagttcatagcccatatatggagttccgcgttacataacttacggtaaatggcccgcctggctgaccgcccaacgacccccgcccattgacgtcaataatgacgtatgttcccatagtaacgccaatagggactttccattgacgtcaatgggtggagtatttacggtaaactgcccacttggcagtacatcaagtgtatcatatgccaagtacgccccctattgacgtcaatgacggtaaatggcccgcctggcattatgcccagtacatgaccttatgggactttcctacttggcagtacatctacgtattagtcatcgctattaccatggtcgaggtgagccccacgttctgcttcactctccccatctcccccccctccccacccccaattttgtatttatttattttttaattattttgtgcagcgatgggggcggggggggggggggggcgcgcgccaggcggggcggggcggggcgaggggcggggcggggcgaggcggagaggtgcggcggcagccaatcagagcggcgcgctccgaaagtttccttttatggcgaggcggcggcggcggcggccctataaaaagcgaagcgcgcggcgggcgggagtcgctgcgtcgcgccttcgccccgtgccccgctccgccgccgcctcgcgccgcccgccccggctctgactgaccgcgttactcccacaggtgagcgggcgggacggcccttctcctccgggctgtaattagcgcttggtttaatgacggctcgtttcttttctgtggctgcgtgaaagccttaaagggctccgggagggccctttgtgcgggggggagcggctcggggggtgcgtgcgtgtgtgtgtgcgtggggagcgccgcgtgcggcccgcgctgcccggcggctgtgagcgctgcgggcgcggcgcggggctttgtgcgctccgcgtgtgcgcgaggggagcgcggccgggggcggtgccccgcggtgcgggggggctgcgaggggaacaaaggctgcgtgcggggtgtgtgcgtgggggggtgagcagggggtgtgggcgcggcggtcgggctgtaacccccccctgcacccccctccccgagttgctgagcacggcccggcttcgggtgcggggctccgtgcggggcgtggcgcggggctcgccgtgccgggcggggggtggcggcaggtgggggtgccgggcggggcggggccgcctcgggccggggagggctcgggggaggggcgcggcggccccggagcgccggcggctgtcgaggcgcggcgagccgcagccattgccttttatggtaatcgtgcgagagggcgcagggacttcctttgtcccaaatctggcggagccgaaatctgggaggcgccgccgcaccccctctagcgggcgcgggcgaagcggtgcggcgccggcaggaaggaaatgggcggggagggccttcgtgcgtcgccgcgccgccgtccccttctccatctccagcctcggggctgccgcagggggacggctgccttcgggggggacggggcagggcggggttcggcttctggcgtgtgaccggcggctctagagcctctgctaaccatgttcatgccttcttctttttcctacagatccttaattaataatacgactcactataggggccgccaccatgacaccacctaagaagaaacggaaggtcgaggacggcgagggccctgctgctaagagagtgaaactggactccggagtgtccaagggcgaagaggacaacatggccagcctgcctgccacccacgagctgcacatcttcggcagcatcaacggcgtggacttcgacatggtgggacagggcaccggcaaccccaacgacggatacgaggaactgaacctgaagtccaccaagggggacctccagttcagcccctggattctggtgccccacatcggctacggcttccaccagtacctgccctaccctgacggcatgagccctttccaggccgctatggtggacggctgcctggaccttaagacccaggtgcagaccccccagggcatgaaggaaatcagcaacatccaagtgggcgacctggtgctgagcaacaccggctacaacgaggtgctgaacgtgttccccaagagcaagaagaagtcctacaagatcaccctggaagatggcaaagagatcatctgctccgaggaacacctgttcccaacccagaccggcgagatgaacatctctggcggcctgaaagagggcatgtgcctgtacgtgaaagaaggcggcggaggacctgaggataagctccaggccattaagtacgagctggcccagaacgaggaagaactggctcagatcgaagagaagctggccgccaacaaagaaggcggatccggcggaggcggatctggaaccggttttgctaatgagctgggccccagactgatgggcaaaggcagcggaggaggcggaagcggagtctttacactggaagatttcgtcggcgactggcggcagacagctggctacaatctggaccaggtgctggaacaaggcggcgtgtcctctctgtttcagaacctgggagtgtctgtgacccctatccagagaatcgtgctgagcggcgagaacggcctgaagatcgacatccacgtgatcatcccttacgagggcctgtccggcgatcagatgggacagatcgagaagatctttaaggtggtgtaccccgtggacgaccaccacttcaaagtgatcctgcactacggcaccctggtcatcgatggcgtgaccccaaacatgatcgactacttcggcagaccctacgagggaatcgccgtgttcgacggcaagaaaatcaccgtgaccggcacactgtggaacggcaacaagatcatcgacgagagactgatcaaccccgacggcagcctgctgttcagagtgacaatcaacggcgtgacaggctggcggctgtgcgaaagaatccttgctggttccggaggaagttcctatacttcaaatagaataggaacttccggcgggtcacccgaggatgagaatgctgctctggaagagaagatcgcccagctgaagcagaagaacgccgctctgaaagaagagatccaggctctggaatacggaggcggaggcatgatgctgaagaagatcctgaagatcgaagaactggacgagcgcgagctgatcgacatcgaggtgtccggcaaccacctgttctacgccaacgatatcctgacccacaactctggctaccaggtgcacagaaccatgcagttcgaggacggcgccagcctgaccgtgaactacagatacacctacgagggcagccacatcaagggcgaggcccaagtgaagggcacaggcttccctgctgacggccccgtgatgaccaactctctgacagccgccgactggtgcagaagcaagaaaacctaccctaacgacaagaccatcatcagcaccttcaagtggtcctacaccacaggcaacggcaagagatacagaagcaccgccagaaccacctacaccttcgccaagcccatggccgccaactacctgaagaaccagcctatgtacgtgttccgaaagaccgagctgaagcacagcaagacagaactgaacttcaaagagtggcagaaagccttcaccgacgtgatgggcatggacgagctgtacaagtccggagctgctccagccgccaagaagaagaagctcgactacaaggacgacgacgataagtgaacgcgtaaatgattgcagatccactagttctagagctcgctgatcagcctcgactgtgccttctagttgccagccatctgttgtttgcccctcccccgtgccttccttgaccctggaaggtgccactcccactgtcctttcctaataaaatgaggaaattgcatcgcattgtctgagtaggtgtcattctattctggggggtggggtggggcaggacagcaagggggaggattgggaagacaatagcaggcatgctggggatgcggtgggctctatggcttctgaggcggaaagaaccagctggggctcgagatccactagttctagcctcgaggctagagcggccgccactggccgtcgttttacaacgtcgtgactgggaaaaccctggcgttacccaacttaatcgccttgcagcacatccccctttcgccagctggcgtaatagcgaagaggcccgcaccgatcgcccttcccaacagttgcgcagcctgaatggcgaatgggacgcgccctgtagcggcgcattaagcgcggcgggtgtggtggttacgcgcagcgtgaccgctacacttgccagcgccctagcgcccgctcctttcgctttcttcccttcctttctcgccacgttcgccggctttccccgtcaagctctaaatcgggggctccctttagggttccgatttagtgctttacggcacctcgaccccaaaaaacttgattagggtgatggttcacgtagtgggccatcgccctgatagacggtttttcgccctttgacgttggagtccacgttctttaatagtggactcttgttccaaactggaacaacactcaaccctatctcggtctattcttttgatttataagggattttgccgatttcggcctattggttaaaaaatgagctgatttaacaaaaatttaacgcgaattttaacaaaatattaacgcttacaatttaggtggcacttttcggggaaatgtgcgcggaacccctatttgtttatttttctaaatacattcaaatatgtatccgctcatgagacaataaccctgataaatgcttcaataatattgaaaaaggaagagtatgagtattcaacatttccgtgtcgcccttattcccttttttgcggcattttgccttcctgtttttgctcacccagaaacgctggtgaaagtaaaagatgctgaagatcagttgggtgcacgagtgggttacatcgaactggatctcaacagcggtaagatccttgagagttttcgccccgaagaacgttttccaatgatgagcacttttaaagttctgctatgtggcgcggtattatcccgtattgacgccgggcaagagcaactcggtcgccgcatacactattctcagaatgacttggttgagtactcaccagtcacagaaaagcatcttacggatggcatgacagtaagagaattatgcagtgctgccataaccatgagtgataacactgcggccaacttacttctgacaacgatcggaggaccgaaggagctaaccgcttttttgcacaacatgggggatcatgtaactcgccttgatcgttgggaaccggagctgaatgaagccataccaaacgacgagcgtgacaccacgatgcctgtagcaatggcaacaacgttgcgcaaactattaactggcgaactacttactctagcttcccggcaacaattaatagactggatggaggcggataaagttgcaggaccacttctgcgctcggcccttccggctggctggtttattgctgataaatctggagccggtgagcgtgggtctcgcggtatcattgcagcactggggccagatggtaagccctcccgtatcgtagttatctacacgacggggagtcaggcaactatggatgaacgaaatagacagatcgctgagataggtgcctcactgattaagcattggtaactgtcagaccaagtttactcatatatactttagattgatttaaaacttcatttttaatttaaaaggatctaggtgaagatcctttttgataatctcatgaccaaaatcccttaacgtgagttttcgttccactgagcgtcagaccccgtagaaaagatcaaaggatcttcttgagatcctttttttctgcgcgtaatctgctgcttgcaaacaaaaaaaccaccgctaccagcggtggtttgtttgccggatcaagagctaccaactctttttccgaaggtaactggcttcagcagagcgcagataccaaatactgtccttctagtgtagccgtagttaggccaccacttcaagaactctgtagcaccgcctacatacctcgctctgctaatcctgttaccagtggctgctgccagtggcgataagtcgtgtcttaccgggttggactcaagacgatagttaccggataaggcgcagcggtcgggctgaacggggggttcgtgcacacagcccagcttggagcgaacgacctacaccgaactgagatacctacagcgtgagctatgagaaagcgccacgcttcccgaagggagaaaggcggacaggtatccggtaagcggcagggtcggaacaggagagcgcacgagggagcttccagggggaaacgcctggtatctttatagtcctgtcgggtttcgccacctctgacttgagcgtcgatttttgtgatgctcgtcaggggggcggagcctatggaaaaacgccagcaacgcggcctttttacggttcctggccttttgctggccttttgctcacatgttctttcctgcgttatcccctgattctgtggataaccgtattaccgcctttgagtgagctgataccgctcgccgcagccgaacgaccgagcgcagcgagtcagtgagcgaggaagcggaagagcgcccaatacgcaaaccgcctctccccgcgcgttggccgattcattaatgcagctggcacgacaggtttcccgactggaaagcgggcagtgagcgcaacgcaattaatgtgagttagctcactcattaggcaccccaggctttacactttatgcttccggctcgtatgttgtgtggaattgtgagcggataacaatttcacacaggaaacagctatgaccatga

SEQ ID NO: 62 - protein, 388 aa, Homo sapiens
MAVSVTPIRDTKWLTLEVCREFQRGTCSRPDTECKFAHPSKSCQVENGRVIACFDSLKGRCSRENCKYLHPPPHLKTQLEINGRNNLIQQKNMAMLAQQMQLANAMMPGAPLQPVPMFSVAPSLATNASAAAFNPYLGPVSPSLVPAEILPTAPMLVTGNPGVPVPAAAAAAAQKLMRTDRLEVCREYQRGNCNRGENDCRFAHPADSTMIDTNDNTVTVCMDYIKGRCSREKCKYFHPPAHLQAKIKAAQYQVNQAAAAQAAATAAAMTQSAVKSLKRPLEATFDLGIPQAVLPPLPKRPALEKTNGATAVFNTGIFQYQQALANMQLQQHTAFLPPVPMVHGATPATVSAATTSATSVPFAATATANQIPIISAEHLTSHKYVTQM

SEQ ID NO: 63 - protein, 373 aa, Homo sapiens
MALNVAPVRDTKWLTLEVCRQFQRGTCSRSDEECKFAHPPKSCQVENGRVIACFDSLKGRCSRENCKYLHPPTHLKTQLEINGRNNLIQQKTAAAMLAQQMQFMFPGTPLHPVPTFPVGPAIGTNTAISFAPYLAPVTPGVGLVPTEILPTTPVIVPGSPPVTVPGSTATQKLLRTDKLEVCREFQRGNCARGETDCRFAHPADSTMIDTSDNTVTVCMDYIKGRCMREKCKYFHPPAHLQAKIKAAQHQANQAAVAAQAAAAAATVMAFPPGALHPLPKRQALEKSNGTSAVFNPSVLHYQQALTSAQLQQHAAFIPTGSVLCMTPATSIDNSEIISRNGMECQESALRITKHCYCTYYPVSSSIELPQTAC

SEQ ID NO: 64 - protein, 782 aa, Homo sapiens
MSGEDGPAAGPGAAAAAARERRREQLRQWGARAGAEPGPGERRARTVRFERAAEFLAACAGGDLDEARLMLRAADPGPGAELDPAAPPPARAVLDSTNADGISALHQACIDENLEVVRFLVEQGATVNQADNEGWTPLHVAASCGYLDIARYLLSHGANIAAVNSDGDLPLDLAESDAMEGLLKAEIARRGVDVEAAKRAEEELLLHDTRCWLNGGAMPEARHPRTGASALHVAAAKGYIEVMRLLLQAGYDPELRDGDGWTPLHAAAHWGVEDACRLLAEHGGGMDSLTHAGQRPCDLADEEVLSLLEELARKQEDLRNQKEASQSRGQEPQAPSSSKHRRSSVCRLSSREKISLQDLSKERRPGGAGGPPIQDEDEGEEGPTEPPPAEPRTLNGVSSPPHPSPKSPVQLEEAPFSRRFGLLKTGSSGALGPPERRTAEGAPGAGLQRSASSSWLEGTSTQAKELRLARITPTPSPKLPEPSVLSEVTKPPPCLENSSPPSRIPEPESPAKPNVPTASTAPPADSRDRRRSYQMPVRDEESESQRKARSRLMRQSRRSTQGVTLTDLKEAEKAAGKAPESEKPAQSLDPSRRPRVPGVENSDSPAQRAEAPDGQGPGPQAAREHRKVGKEWRGPAEGEEAEPADRSQESSTLEGGPSARRQRWQRDLNPEPEPESEEPDGGFRTLYAELRRENERLREALTETTLRLAQLKVELERATQRQERFAERPALLELERFERRALERKAAELEEELKALSDLRADNQRLKDENAALIRVISKLSK

SEQ ID NO: 65 - DNA, 4104 bp, Artificial sequence
  mammalian codon-optimized nuclease-defect S. pyogenes Cas9 (D10A, H840A)
atggacaagaagtacagcatcggcctggccatcggcaccaactctgtgggctgggccgtgatcaccgacgagtacaaggtgcccagcaagaaattcaaggtgctgggcaacaccgaccggcacagcatcaagaagaacctgatcggagccctgctgttcgacagcggcgaaacagccgaggccacccggctgaagagaaccgccagaagaagatacaccagacggaagaaccggatctgctatctgcaagagatcttcagcaacgagatggccaaggtggacgacagcttcttccacagactggaagagtccttcctggtggaagaggataagaagcacgagcggcaccccatcttcggcaacatcgtggacgaggtggcctaccacgagaagtaccccaccatctaccacctgagaaagaaactggtggacagcaccgacaaggccgacctgcggctgatctatctggccctggcccacatgatcaagttccggggccacttcctgatcgagggcgacctgaaccccgacaacagcgacgtggacaagctgttcatccagctggtgcagacctacaaccagctgttcgaggaaaaccccatcaacgccagcggcgtggacgccaaggccatcctgtctgccagactgagcaagagcagacggctggaaaatctgatcgcccagctgcccggcgagaagaagaatggcctgttcggcaacctgattgccctgagcctgggcctgacccccaacttcaagagcaacttcgacctggccgaggatgccaaactgcagctgagcaaggacacctacgacgacgacctggacaacctgctggcccagatcggcgaccagtacgccgacctgtttctggccgccaagaacctgtccgacgccatcctgctgagcgacatcctgagagtgaacaccgagatcaccaaggcccccctgagcgcctctatgatcaagagatacgacgagcaccaccaggacctgaccctgctgaaagctctcgtgcggcagcagctgcctgagaagtacaaagagattttcttcgaccagagcaagaacggctacgccggctacattgacggcggagccagccaggaagagttctacaagttcatcaagcccatcctggaaaagatggacggcaccgaggaactgctcgtgaagctgaacagagaggacctgctgcggaagcagcggaccttcgacaacggcagcatcccccaccagatccacctgggagagctgcacgccattctgcggcggcaggaagatttttacccattcctgaaggacaaccgggaaaagatcgagaagatcctgaccttccgcatcccctactacgtgggccctctggccaggggaaacagcagattcgcctggatgaccagaaagagcgaggaaaccatcaccccctggaacttcgaggaagtggtggacaagggcgcttccgcccagagcttcatcgagcggatgaccaacttcgataagaacctgcccaacgagaaggtgctgcccaagcacagcctgctgtacgagtacttcaccgtgtataacgagctgaccaaagtgaaatacgtgaccgagggaatgagaaagcccgccttcctgagcggcgagcagaaaaaggccatcgtggacctgctgttcaagaccaaccggaaagtgaccgtgaagcagctgaaagaggactacttcaagaaaatcgagtgcttcgactccgtggaaatctccggcgtggaagatcggttcaacgcctccctgggcacataccacgatctgctgaaaattatcaaggacaaggacttcctggacaatgaggaaaacgaggacattctggaagatatcgtgctgaccctgacactgtttgaggacagagagatgatcgaggaacggctgaaaacctatgcccacctgttcgacgacaaagtgatgaagcagctgaagcggcggagatacaccggctggggcaggctgagccggaagctgatcaacggcatccgggacaagcagtccggcaagacaatcctggatttcctgaagtccgacggcttcgccaacagaaacttcatgcagctgatccacgacgacagcctgacctttaaagaggacatccagaaagcccaggtgtccggccagggcgatagcctgcacgagcacattgccaatctggccggcagccccgccattaagaagggcatcctgcagacagtgaaggtggtggacgagctcgtgaaagtgatgggccggcacaagcccgagaacatcgtgatcgaaatggccagagagaaccagaccacccagaagggacagaagaacagccgcgagagaatgaagcggatcgaagagggcatcaaagagctgggcagccagatcctgaaagaacaccccgtggaaaacacccagctgcagaacgagaagctgtacctgtactacctgcagaatgggcgggatatgtacgtggaccaggaactggacatcaaccggctgtccgactacgatgtggacgccatcgtgcctcagagctttctgaaggacgactccatcgacaacaaggtgctgaccagaagcgacaagaaccggggcaagagcgacaacgtgccctccgaagaggtcgtgaagaagatgaagaactactggcggcagctgctgaacgccaagctgattacccagagaaagttcgacaatctgaccaaggccgagagaggcggcctgagcgaactggataaggccggcttcatcaagagacagctggtggaaacccggcagatcacaaagcacgtggcacagatcctggactcccggatgaacactaagtacgacgagaatgacaagctgatccgggaagtgaaagtgatcaccctgaagtccaagctggtgtccgatttccggaaggatttccagttttacaaagtgcgcgagatcaacaactaccaccacgcccacgacgcctacctgaacgccgtcgtgggaaccgccctgatcaaaaagtaccctaagctggaaagcgagttcgtgtacggcgactacaaggtgtacgacgtgcggaagatgatcgccaagagcgagcaggaaatcggcaaggctaccgccaagtacttcttctacagcaacatcatgaactttttcaagaccgagattaccctggccaacggcgagatccggaagcggcctctgatcgagacaaacggcgaaaccggggagatcgtgtgggataagggccgggattttgccaccgtgcggaaagtgctgagcatgccccaagtgaatatcgtgaaaaagaccgaggtgcagacaggcggcttcagcaaagagtctatcctgcccaagaggaacagcgataagctgatcgccagaaagaaggactgggaccctaagaagtacggcggcttcgacagccccaccgtggcctattctgtgctggtggtggccaaagtggaaaagggcaagtccaagaaactgaagagtgtgaaagagctgctggggatcaccatcatggaaagaagcagcttcgagaagaatcccatcgactttctggaagccaagggctacaaagaagtgaaaaaggacctgatcatcaagctgcctaagtactccctgttcgagctggaaaacggccggaagagaatgctggcctctgccggcgaactgcagaagggaaacgaactggccctgccctccaaatatgtgaacttcctgtacctggccagccactatgagaagctgaagggctcccccgaggataatgagcagaaacagctgtttgtggaacagcacaagcactacctggacgagatcatcgagcagatcagcgagttctccaagagagtgatcctggccgacgctaatctggacaaagtgctgtccgcctacaacaagcaccgggataagcccatcagagagcaggccgagaatatcatccacctgtttaccctgaccaatctgggagcccctgccgccttcaagtactttgacaccaccatcgaccggaagaggtacaccagcaccaaagaggtgctggacgccaccctgatccaccagagcatcaccggcctgtacgagacacggatcgacctgtctcagctgggaggcgac